European Patent Application EP 4 361 270 A1, published May 1, 2024. Title: non naturally ocurring 5'-untranslated region and 3'- untranslated region and use thereof. Applicant: HANMI PHARM. CO., LTD. The sequence listing filed with the application follows.

SEQUENCE LISTING (115 sequences)

SEQ ID NO: 1 - RNA, 61 nt, Artificial
  5'-UTR sequence
aguccuccccauccucucccucugucccucugucccucugacccugcacugucccagcacc

SEQ ID NO: 2 - RNA, 61 nt, Artificial
  5'-UTR sequence
aguccucccccgucccucugaauccucucccucugucccucuccugcacugucccagcacc

SEQ ID NO: 3 - RNA, 61 nt, Artificial
  5'-UTR sequence
aguccuccccauccucucccucuuucccucugucccucuuacccuucacuuucccagcacc

SEQ ID NO: 4 - RNA, 61 nt, Artificial
  5'-UTR sequence
aguccuccccauuuuuuuuuucugucccucugucccucugacccugcacugucccagcacc

SEQ ID NO: 5 - RNA, 61 nt, Artificial
  5'-UTR sequence
aguccuccccauccaacuaaacugucccucugucccucugacccugcacugucccagcacc

SEQ ID NO: 6 - RNA, 61 nt, Artificial
  5'-UTR sequence
aguccuccccauccaacuaaacugucccucugucccaacuaaacugcacugucccagcacc

SEQ ID NO: 7 - RNA, 61 nt, Artificial
  5'-UTR sequence
aguccuccccauaacuaaacucugucccucugucccaacuaaacugcacugucccagcacc

SEQ ID NO: 8 - RNA, 61 nt, Artificial
  5'-UTR sequence
aguccuccccauaacuaaaaacugucccucugucccaacuaaacugcacugucccagcacc

SEQ ID NO: 9 - RNA, 61 nt, Artificial
  31
aguccuccccauccaacuaaacugucccucuaucccaacuaaacugcacuguuccagcacc

SEQ ID NO: 10 - RNA, 61 nt, Artificial
  5'-UTR sequence
agugcuccccauccaacuaaacugucccucuguccgaacuaaacugcacugucccagcacc

SEQ ID NO: 11 - RNA, 61 nt, Artificial
  5'-UTR sequence
aguccuacccauccaacuaaacuguccuucugucccaacuaaacugcacugucccagcacc

SEQ ID NO: 12 - RNA, 62 nt, Artificial
  5'-UTR sequence
gaguccuccccauccaacuaaacugucccucuaucccaacuaaacugcacuguuccagcacc

SEQ ID NO: 13 - RNA, 10 nt, Artificial
  hairpin sequence
gucccucuga

SEQ ID NO: 14 - RNA, 169 nt, Artificial
  3'-UTR sequence
ccacacccccauucccccacuccagauaaagcuucaguuauaucucacgugucuggaguucuuugccaagagggagaggcugaaauccccagccgccucaccugcagcucagcuccauccccucaccuguucccaccgcauuuucuccuggcguucgccugcuagugug

SEQ ID NO: 15 - RNA, 186 nt, Artificial
  3'-UTR sequence
ccacacccccauucccccacuccagauaaagcuucaguuauaucucacgugucuggaguucuuugccaagagggagaggcugaaauccccagccgccucaccugcagcucagcuccauccuccacccccccaucuccccucaccuguucccaccgcauuuucuccuggcguucgccugcuagugug

SEQ ID NO: 16 - RNA, 176 nt, Artificial
  3'-UTR sequence
ccacacccccauucccccacuccagauaaagcuucaguuauaucucacgugucuggaguucuuugccaagagggagaggcugaaauccccagccgccucaccugcagcucagcuccauccuugguuuccucaccuguucccaccgcauuuucuccuggcguucgccugcuagugug

SEQ ID NO: 17 - RNA, 150 nt, Artificial
  3'-UTR sequence
gugugacccugaaccccccgcuuucaaacaaguuuucaaauuguuugaggucaggauuucucaaacugauuccuuucuuugcauaugaguauuugaaaauaaauauuuucccagaauauaaauaaaucaucacaugauuauuuuaacuau

SEQ ID NO: 18 - RNA, 167 nt, Artificial
  3'-UTR sequence
guguguccacccccccaucuccacccugaaccccccgcuuucaaacaaguuuucaaauuguuugaggucaggauuucucaaacugauuccuuucuuugcauaugaguauuugaaaauaaauauuuucccagaauauaaauaaaucaucacaugauuauuuuaacuau

SEQ ID NO: 19 - RNA, 157 nt, Artificial
  3'-UTR sequence
guguguugguuuacccugaaccccccgcuuucaaacaaguuuucaaauuguuugaggucaggauuucucaaacugauuccuuucuuugcauaugaguauuugaaaauaaauauuuucccagaauauaaauaaaucaucacaugauuauuuuaacuau

SEQ ID NO: 20 - RNA, 158 nt, Artificial
  3'-UTR sequence
guguguggaggacacccugaaccccccgcuuucaaacaaguuuucaaauuguuugaggucaggauuucucaaacugauuccuuucuuugcauaugaguauuugaaaauaaauauuuucccagaauauaaauaaaucaucacaugauuauuuuaacuau

SEQ ID NO: 21 - RNA, 17 nt, Artificial
  CU-rich element
uccacccccccaucucc

SEQ ID NO: 22 - DNA, 61 bp, Artificial
  nucleotide sequence encoding 5'-UTR sequence
agtcctccccatcctctccctctgtccctctgtccctctgaccctgcactgtcccagcacc

SEQ ID NO: 23 - DNA, 61 bp, Artificial
  nucleotide sequence encoding 5'-UTR sequence
agtcctcccccgtccctctgaatcctctccctctgtccctctcctgcactgtcccagcacc

SEQ ID NO: 24 - DNA, 61 bp, Artificial
  nucleotide sequence encoding 5'-UTR sequence
agtcctccccatcctctccctctttccctctgtccctcttacccttcactttcccagcacc

SEQ ID NO: 25 - DNA, 61 bp, Artificial
  nucleotide sequence encoding 5'-UTR sequence
agtcctccccattttttttttctgtccctctgtccctctgaccctgcactgtcccagcacc

SEQ ID NO: 26 - DNA, 61 bp, Artificial
  nucleotide sequence encoding 5'-UTR sequence
agtcctccccatccaactaaactgtccctctgtccctctgaccctgcactgtcccagcacc

SEQ ID NO: 27 - DNA, 61 bp, Artificial
  nucleotide sequence encoding 5'-UTR sequence
agtcctccccatccaactaaactgtccctctgtcccaactaaactgcactgtcccagcacc

SEQ ID NO: 28 - DNA, 61 bp, Artificial
  nucleotide sequence encoding 5'-UTR sequence
agtcctccccataactaaactctgtccctctgtcccaactaaactgcactgtcccagcacc

SEQ ID NO: 29 - DNA, 61 bp, Artificial
  nucleotide sequence encoding 5'-UTR sequence
agtcctccccataactaaaaactgtccctctgtcccaactaaactgcactgtcccagcacc

SEQ ID NO: 30 - DNA, 61 bp, Artificial
  nucleotide sequence encoding 5'-UTR sequence
agtcctccccatccaactaaactgtccctctatcccaactaaactgcactgttccagcacc

SEQ ID NO: 31 - DNA, 61 bp, Artificial
  nucleotide sequence encoding 5'-UTR sequence
agtgctccccatccaactaaactgtccctctgtccgaactaaactgcactgtcccagcacc

SEQ ID NO: 32 - DNA, 61 bp, Artificial
  nucleotide sequence encoding 5'-UTR sequence
agtcctacccatccaactaaactgtccttctgtcccaactaaactgcactgtcccagcacc

SEQ ID NO: 33 - DNA, 62 bp, Artificial
  nucleotide sequence encoding 5'-UTR sequence
gagtcctccccatccaactaaactgtccctctatcccaactaaactgcactgttccagcacc

SEQ ID NO: 34 - DNA, 169 bp, Artificial
  nucleotide sequence encoding 3'-UTR
ccacacccccattcccccactccagataaagcttcagttatatctcacgtgtctggagttctttgccaagagggagaggctgaaatccccagccgcctcacctgcagctcagctccatcccctcacctgttcccaccgcattttctcctggcgttcgcctgctagtgtg

SEQ ID NO: 35 - DNA, 186 bp, Artificial
  nucleotide sequence encoding 3'-UTR
ccacacccccattcccccactccagataaagcttcagttatatctcacgtgtctggagttctttgccaagagggagaggctgaaatccccagccgcctcacctgcagctcagctccatcctccacccccccatctcccctcacctgttcccaccgcattttctcctggcgttcgcctgctagtgtg

SEQ ID NO: 36 - DNA, 176 bp, Artificial
  nucleotide sequence encoding 3'-UTR
ccacacccccattcccccactccagataaagcttcagttatatctcacgtgtctggagttctttgccaagagggagaggctgaaatccccagccgcctcacctgcagctcagctccatccttggtttcctcacctgttcccaccgcattttctcctggcgttcgcctgctagtgtg

SEQ ID NO: 37 - DNA, 150 bp, Artificial
  nucleotide sequence encoding 3'-UTR
gtgtgaccctgaaccccccgctttcaaacaagttttcaaattgtttgaggtcaggatttctcaaactgattcctttctttgcatatgagtatttgaaaataaatattttcccagaatataaataaatcatcacatgattattttaactat

SEQ ID NO: 38 - DNA, 167 bp, Artificial
  nucleotide sequence encoding 3'-UTR
gtgtgtccacccccccatctccaccctgaaccccccgctttcaaacaagttttcaaattgtttgaggtcaggatttctcaaactgattcctttctttgcatatgagtatttgaaaataaatattttcccagaatataaataaatcatcacatgattattttaactat

SEQ ID NO: 39 - DNA, 157 bp, Artificial
  nucleotide sequence encoding 3'-UTR
gtgtgttggtttaccctgaaccccccgctttcaaacaagttttcaaattgtttgaggtcaggatttctcaaactgattcctttctttgcatatgagtatttgaaaataaatattttcccagaatataaataaatcatcacatgattattttaactat

SEQ ID NO: 40 - DNA, 158 bp, Artificial
  nucleotide sequence encoding 3'-UTR
gtgtgtggaggacaccctgaaccccccgctttcaaacaagttttcaaattgtttgaggtcaggatttctcaaactgattcctttctttgcatatgagtatttgaaaataaatattttcccagaatataaataaatcatcacatgattattttaactat

SEQ ID NO: 41 - DNA, 100 bp, Artificial
  polyA DNA
aaaaaaaaaaaaaaaaaaaaaaaaaaaaaaaaaaaaaaaaaaaaaaaaaaaaaaaaaaaaaaaaaaaaaaaaaaaaaaaaaaaaaaaaaaaaaaaaaaaa

SEQ ID NO: 42 - protein, 1273 aa, SARS-CoV-2
MFVFLVLLPLVSSQCVNLTTRTQLPPAYTNSFTRGVYYPDKVFRSSVLHSTQDLFLPFFSNVTWFHAIHVSGTNGTKRFDNPVLPFNDGVYFASTEKSNIIRGWIFGTTLDSKTQSLLIVNNATNVVIKVCEFQFCNDPFLGVYYHKNNKSWMESEFRVYSSANNCTFEYVSQPFLMDLEGKQGNFKNLREFVFKNIDGYFKIYSKHTPINLVRDLPQGFSALEPLVDLPIGINITRFQTLLALHRSYLTPGDSSSGWTAGAAAYYVGYLQPRTFLLKYNENGTITDAVDCALDPLSETKCTLKSFTVEKGIYQTSNFRVQPTESIVRFPNITNLCPFGEVFNATRFASVYAWNRKRISNCVADYSVLYNSASFSTFKCYGVSPTKLNDLCFTNVYADSFVIRGDEVRQIAPGQTGKIADYNYKLPDDFTGCVIAWNSNNLDSKVGGNYNYLYRLFRKSNLKPFERDISTEIYQAGSTPCNGVEGFNCYFPLQSYGFQPTNGVGYQPYRVVVLSFELLHAPATVCGPKKSTNLVKNKCVNFNFNGLTGTGVLTESNKKFLPFQQFGRDIADTTDAVRDPQTLEILDITPCSFGGVSVITPGTNTSNQVAVLYQDVNCTEVPVAIHADQLTPTWRVYSTGSNVFQTRAGCLIGAEHVNNSYECDIPIGAGICASYQTQTNSPRRARSVASQSIIAYTMSLGAENSVAYSNNSIAIPTNFTISVTTEILPVSMTKTSVDCTMYICGDSTECSNLLLQYGSFCTQLNRALTGIAVEQDKNTQEVFAQVKQIYKTPPIKDFGGFNFSQILPDPSKPSKRSFIEDLLFNKVTLADAGFIKQYGDCLGDIAARDLICAQKFNGLTVLPPLLTDEMIAQYTSALLAGTITSGWTFGAGAALQIPFAMQMAYRFNGIGVTQNVLYENQKLIANQFNSAIGKIQDSLSSTASALGKLQDVVNQNAQALNTLVKQLSSNFGAISSVLNDILSRLDPPEAEVQIDRLITGRLQSLQTYVTQQLIRAAEIRASANLAATKMSECVLGQSKRVDFCGKGYHLMSFPQSAPHGVVFLHVTYVPAQEKNFTTAPAICHDGKAHFPREGVFVSNGTHWFVTQRNFYEPQIITTDNTFVSGNCDVVIGIVNNTVYDPLQPELDSFKEELDKYFKNHTSPDVDLGDISGINASVVNIQKEIDRLNEVAKNLNESLIDLQELGKYEQYIKWPWYIWLGFIAGLIAIVMVTIMLCCMTSCCSCLKGCCSCGSCCKFDEDDSEPVLKGVKLHYT

SEQ ID NO: 43 - protein, 1270 aa, SARS-CoV-2
MFVFLVLLPLVSSQCVNLTTRTQLPPAYTNSFTRGVYYPDKVFRSSVLHSTQDLFLPFFSNVTWFHAISGTNGTKRFDNPVLPFNDGVYFASTEKSNIIRGWIFGTTLDSKTQSLLIVNNATNVVIKVCEFQFCNDPFLGVYHKNNKSWMESEFRVYSSANNCTFEYVSQPFLMDLEGKQGNFKNLREFVFKNIDGYFKIYSKHTPINLVRDLPQGFSALEPLVDLPIGINITRFQTLLALHRSYLTPGDSSSGWTAGAAAYYVGYLQPRTFLLKYNENGTITDAVDCALDPLSETKCTLKSFTVEKGIYQTSNFRVQPTESIVRFPNITNLCPFGEVFNATRFASVYAWNRKRISNCVADYSVLYNSASFSTFKCYGVSPTKLNDLCFTNVYADSFVIRGDEVRQIAPGQTGKIADYNYKLPDDFTGCVIAWNSNNLDSKVGGNYNYLYRLFRKSNLKPFERDISTEIYQAGSTPCNGVEGFNCYFPLQSYGFQPTYGVGYQPYRVVVLSFELLHAPATVCGPKKSTNLVKNKCVNFNFNGLTGTGVLTESNKKFLPFQQFGRDIDDTTDAVRDPQTLEILDITPCSFGGVSVITPGTNTSNQVAVLYQGVNCTEVPVAIHADQLTPTWRVYSTGSNVFQTRAGCLIGAEHVNNSYECDIPIGAGICASYQTQTNSHRRARSVASQSIIAYTMSLGAENSVAYSNNSIAIPINFTISVTTEILPVSMTKTSVDCTMYICGDSTECSNLLLQYGSFCTQLNRALTGIAVEQDKNTQEVFAQVKQIYKTPPIKDFGGFNFSQILPDPSKPSKRSFIEDLLFNKVTLADAGFIKQYGDCLGDIAARDLICAQKFNGLTVLPPLLTDEMIAQYTSALLAGTITSGWTFGAGAALQIPFAMQMAYRFNGIGVTQNVLYENQKLIANQFNSAIGKIQDSLSSTASALGKLQDVVNQNAQALNTLVKQLSSNFGAISSVLNDILARLDPPEAEVQIDRLITGRLQSLQTYVTQQLIRAAEIRASANLAATKMSECVLGQSKRVDFCGKGYHLMSFPQSAPHGVVFLHVTYVPAQEKNFTTAPAICHDGKAHFPREGVFVSNGTHWFVTQRNFYEPQIITTHNTFVSGNCDVVIGIVNNTVYDPLQPELDSFKEELDKYFKNHTSPDVDLGDISGINASVVNIQKEIDRLNEVAKNLNESLIDLQELGKYEQYIKWPWYIWLGFIAGLIAIVMVTIMLCCMTSCCSCLKGCCSCGSCCKFDEDDSEPVLKGVKLHYT

SEQ ID NO: 44 - protein, 1270 aa, SARS-CoV-2
MFVFLVLLPLVSSQCVNFTTRTQLPPAYTNSFTRGVYYPDKVFRSSVLHSTQDLFLPFFSNVTWFHAIHVSGTNGTKRFANPVLPFNDGVYFASTEKSNIIRGWIFGTTLDSKTQSLLIVNNATNVVIKVCEFQFCNDPFLGVYYHKNNKSWMESEFRVYSSANNCTFEYVSQPFLMDLEGKQGNFKNLREFVFKNIDGYFKIYSKHTPINLVRGLPQGFSALEPLVDLPIGINITRFQTLHRSYLTPGDSSSGWTAGAAAYYVGYLQPRTFLLKYNENGTITDAVDCALDPLSETKCTLKSFTVEKGIYQTSNFRVQPTESIVRFPNITNLCPFGEVFNATRFASVYAWNRKRISNCVADYSVLYNSASFSTFKCYGVSPTKLNDLCFTNVYADSFVIRGDEVRQIAPGQTGNIADYNYKLPDDFTGCVIAWNSNNLDSKVGGNYNYLYRLFRKSNLKPFERDISTEIYQAGSTPCNGVKGFNCYFPLQSYGFQPTYGVGYQPYRVVVLSFELLHAPATVCGPKKSTNLVKNKCVNFNFNGLTGTGVLTESNKKFLPFQQFGRDIADTTDAVRDPQTLEILDITPCSFGGVSVITPGTNTSNQVAVLYQGVNCTEVPVAIHADQLTPTWRVYSTGSNVFQTRAGCLIGAEHVNNSYECDIPIGAGICASYQTQTNSPRRARSVASQSIIAYTMSLGVENSVAYSNNSIAIPTNFTISVTTEILPVSMTKTSVDCTMYICGDSTECSNLLLQYGSFCTQLNRALTGIAVEQDKNTQEVFAQVKQIYKTPPIKDFGGFNFSQILPDPSKPSKRSFIEDLLFNKVTLADAGFIKQYGDCLGDIAARDLICAQKFNGLTVLPPLLTDEMIAQYTSALLAGTITSGWTFGAGAALQIPFAMQMAYRFNGIGVTQNVLYENQKLIANQFNSAIGKIQDSLSSTASALGKLQDVVNQNAQALNTLVKQLSSNFGAISSVLNDILSRLDPPEAEVQIDRLITGRLQSLQTYVTQQLIRAAEIRASANLAATKMSECVLGQSKRVDFCGKGYHLMSFPQSAPHGVVFLHVTYVPAQEKNFTTAPAICHDGKAHFPREGVFVSNGTHWFVTQRNFYEPQIITTDNTFVSGNCDVVIGIVNNTVYDPLQPELDSFKEELDKYFKNHTSPDVDLGDISGINASVVNIQKEIDRLNEVAKNLNESLIDLQELGKYEQYIKWPWYIWLGFIAGLIAIVMVTIMLCCMTSCCSCLKGCCSCGSCCKFDEDDSEPVLKGVKLHYT

SEQ ID NO: 45 - protein, 1273 aa, SARS-CoV-2
MFVFLVLLPLVSSQCVNFTNRTQLPSAYTNSFTRGVYYPDKVFRSSVLHSTQDLFLPFFSNVTWFHAIHVSGTNGTKRFDNPVLPFNDGVYFASTEKSNIIRGWIFGTTLDSKTQSLLIVNNATNVVIKVCEFQFCNYPFLGVYYHKNNKSWMESEFRVYSSANNCTFEYVSQPFLMDLEGKQGNFKNLSEFVFKNIDGYFKIYSKHTPINLVRDLPQGFSALEPLVDLPIGINITRFQTLLALHRSYLTPGDSSSGWTAGAAAYYVGYLQPRTFLLKYNENGTITDAVDCALDPLSETKCTLKSFTVEKGIYQTSNFRVQPTESIVRFPNITNLCPFGEVFNATRFASVYAWNRKRISNCVADYSVLYNSASFSTFKCYGVSPTKLNDLCFTNVYADSFVIRGDEVRQIAPGQTGTIADYNYKLPDDFTGCVIAWNSNNLDSKVGGNYNYLYRLFRKSNLKPFERDISTEIYQAGSTPCNGVKGFNCYFPLQSYGFQPTYGVGYQPYRVVVLSFELLHAPATVCGPKKSTNLVKNKCVNFNFNGLTGTGVLTESNKKFLPFQQFGRDIADTTDAVRDPQTLEILDITPCSFGGVSVITPGTNTSNQVAVLYQGVNCTEVPVAIHADQLTPTWRVYSTGSNVFQTRAGCLIGAEYVNNSYECDIPIGAGICASYQTQTNSPRRARSVASQSIIAYTMSLGAENSVAYSNNSIAIPTNFTISVTTEILPVSMTKTSVDCTMYICGDSTECSNLLLQYGSFCTQLNRALTGIAVEQDKNTQEVFAQVKQIYKTPPIKDFGGFNFSQILPDPSKPSKRSFIEDLLFNKVTLADAGFIKQYGDCLGDIAARDLICAQKFNGLTVLPPLLTDEMIAQYTSALLAGTITSGWTFGAGAALQIPFAMQMAYRFNGIGVTQNVLYENQKLIANQFNSAIGKIQDSLSSTASALGKLQDVVNQNAQALNTLVKQLSSNFGAISSVLNDILSRLDPPEAEVQIDRLITGRLQSLQTYVTQQLIRAAEIRASANLAAIKMSECVLGQSKRVDFCGKGYHLMSFPQSAPHGVVFLHVTYVPAQEKNFTTAPAICHDGKAHFPREGVFVSNGTHWFVTQRNFYEPQIITTDNTFVSGNCDVVIGIVNNTVYDPLQPELDSFKEELDKYFKNHTSPDVDLGDISGINASFVNIQKEIDRLNEVAKNLNESLIDLQELGKYEQYIKWPWYIWLGFIAGLIAIVMVTIMLCCMTSCCSCLKGCCSCGSCCKFDEDDSEPVLKGVKLHYT

SEQ ID NO: 46 - protein, 1271 aa, SARS-CoV-2
MFVFLVLLPLVSSQCVNLRTRTQLPPAYTNSFTRGVYYPDKVFRSSVLHSTQDLFLPFFSNVTWFHAIHVSGTNGTKRFDNPVLPFNDGVYFASTEKSNIIRGWIFGTTLDSKTQSLLIVNNATNVVIKVCEFQFCNDPFLDVYYHKNNKSWMESGVYSSANNCTFEYVSQPFLMDLEGKQGNFKNLREFVFKNIDGYFKIYSKHTPINLVRDLPQGFSALEPLVDLPIGINITRFQTLLALHRSYLTPGDSSSGWTAGAAAYYVGYLQPRTFLLKYNENGTITDAVDCALDPLSETKCTLKSFTVEKGIYQTSNFRVQPTESIVRFPNITNLCPFGEVFNATRFASVYAWNRKRISNCVADYSVLYNSASFSTFKCYGVSPTKLNDLCFTNVYADSFVIRGDEVRQIAPGQTGKIADYNYKLPDDFTGCVIAWNSNNLDSKVGGNYNYRYRLFRKSNLKPFERDISTEIYQAGSKPCNGVEGFNCYFPLQSYGFQPTNGVGYQPYRVVVLSFELLHAPATVCGPKKSTNLVKNKCVNFNFNGLTGTGVLTESNKKFLPFQQFGRDIADTTDAVRDPQTLEILDITPCSFGGVSVITPGTNTSNQVAVLYQGVNCTEVPVAIHADQLTPTWRVYSTGSNVFQTRAGCLIGAEHVNNSYECDIPIGAGICASYQTQTNSRRRARSVASQSIIAYTMSLGAENSVAYSNNSIAIPTNFTISVTTEILPVSMTKTSVDCTMYICGDSTECSNLLLQYGSFCTQLNRALTGIAVEQDKNTQEVFAQVKQIYKTPPIKDFGGFNFSQILPDPSKPSKRSFIEDLLFNKVTLADAGFIKQYGDCLGDIAARDLICAQKFNGLTVLPPLLTDEMIAQYTSALLAGTITSGWTFGAGAALQIPFAMQMAYRFNGIGVTQNVLYENQKLIANQFNSAIGKIQDSLSSTASALGKLQNVVNQNAQALNTLVKQLSSNFGAISSVLNDILSRLDPPEAEVQIDRLITGRLQSLQTYVTQQLIRAAEIRASANLAATKMSECVLGQSKRVDFCGKGYHLMSFPQSAPHGVVFLHVTYVPAQEKNFTTAPAICHDGKAHFPREGVFVSNGTHWFVTQRNFYEPQIITTDNTFVSGNCDVVIGIVNNTVYDPLQPELDSFKEELDKYFKNHTSPDVDLGDISGINASVVNIQKEIDRLNEVAKNLNESLIDLQELGKYEQYIKWPWYIWLGFIAGLIAIVMVTIMLCCMTSCCSCLKGCCSCGSCCKFDEDDSEPVLKGVKLHYT

SEQ ID NO: 47 - protein, 1273 aa, SARS-CoV-2
MFVFLVLLPLVSIQCVNLTTRTQLPPAYTNSFTRGVYYPDKVFRSSVLHSTQDLFLPFFSNVTWFHAIHVSGTNGTKRFDNPVLPFNDGVYFASTEKSNIIRGWIFGTTLDSKTQSLLIVNNATNVVIKVCEFQFCNDPFLGVYYHKNNKSCMESEFRVYSSANNCTFEYVSQPFLMDLEGKQGNFKNLREFVFKNIDGYFKIYSKHTPINLVRDLPQGFSALEPLVDLPIGINITRFQTLLALHRSYLTPGDSSSGWTAGAAAYYVGYLQPRTFLLKYNENGTITDAVDCALDPLSETKCTLKSFTVEKGIYQTSNFRVQPTESIVRFPNITNLCPFGEVFNATRFASVYAWNRKRISNCVADYSVLYNSASFSTFKCYGVSPTKLNDLCFTNVYADSFVIRGDEVRQIAPGQTGKIADYNYKLPDDFTGCVIAWNSNNLDSKVGGNYNYRYRLFRKSNLKPFERDISTEIYQAGSTPCNGVEGFNCYFPLQSYGFQPTNGVGYQPYRVVVLSFELLHAPATVCGPKKSTNLVKNKCVNFNFNGLTGTGVLTESNKKFLPFQQFGRDIADTTDAVRDPQTLEILDITPCSFGGVSVITPGTNTSNQVAVLYQGVNCTEVPVAIHADQLTPTWRVYSTGSNVFQTRAGCLIGAEHVNNSYECDIPIGAGICASYQTQTNSPRRARSVASQSIIAYTMSLGAENSVAYSNNSIAIPTNFTISVTTEILPVSMTKTSVDCTMYICGDSTECSNLLLQYGSFCTQLNRALTGIAVEQDKNTQEVFAQVKQIYKTPPIKDFGGFNFSQILPDPSKPSKRSFIEDLLFNKVTLADAGFIKQYGDCLGDIAARDLICAQKFNGLTVLPPLLTDEMIAQYTSALLAGTITSGWTFGAGAALQIPFAMQMAYRFNGIGVTQNVLYENQKLIANQFNSAIGKIQDSLSSTASALGKLQDVVNQNAQALNTLVKQLSSNFGAISSVLNDILSRLDPPEAEVQIDRLITGRLQSLQTYVTQQLIRAAEIRASANLAATKMSECVLGQSKRVDFCGKGYHLMSFPQSAPHGVVFLHVTYVPAQEKNFTTAPAICHDGKAHFPREGVFVSNGTHWFVTQRNFYEPQIITTDNTFVSGNCDVVIGIVNNTVYDPLQPELDSFKEELDKYFKNHTSPDVDLGDISGINASVVNIQKEIDRLNEVAKNLNESLIDLQELGKYEQYIKWPWYIWLGFIAGLIAIVMVTIMLCCMTSCCSCLKGCCSCGSCCKFDEDDSEPVLKGVKLHYT

SEQ ID NO: 48 - protein, 1270 aa, SARS-CoV-2
MFVFLVLLPLVSSQCVNLTTRTQLPPAYTNSFTRGVYYPDKVFRSSVLHSTQDLFLPFFSNVTWFHVISGTNGTKRFDNPVLPFNDGVYFASIEKSNIIRGWIFGTTLDSKTQSLLIVNNATNVVIKVCEFQFCNDPFLDHKNNKSWMESEFRVYSSANNCTFEYVSQPFLMDLEGKQGNFKNLREFVFKNIDGYFKIYSKHTPIIVREPEDLPQGFSALEPLVDLPIGINITRFQTLLALHRSYLTPGDSSSGWTAGAAAYYVGYLQPRTFLLKYNENGTITDAVDCALDPLSETKCTLKSFTVEKGIYQTSNFRVQPTESIVRFPNITNLCPFDEVFNATRFASVYAWNRKRISNCVADYSVLYNLAPFFTFKCYGVSPTKLNDLCFTNVYADSFVIRGDEVRQIAPGQTGNIADYNYKLPDDFTGCVIAWNSNKLDSKVSGNYNYLYRLFRKSNLKPFERDISTEIYQAGNKPCNGVAGFNCYFPLRSYSFRPTYGVGHQPYRVVVLSFELLHAPATVCGPKKSTNLVKNKCVNFNFNGLKGTGVLTESNKKFLPFQQFGRDIADTTDAVRDPQTLEILDITPCSFGGVSVITPGTNTSNQVAVLYQGVNCTEVPVAIHADQLTPTWRVYSTGSNVFQTRAGCLIGAEYVNNSYECDIPIGAGICASYQTQTKSHRRARSVASQSIIAYTMSLGAENSVAYSNNSIAIPTNFTISVTTEILPVSMTKTSVDCTMYICGDSTECSNLLLQYGSFCTQLKRALTGIAVEQDKNTQEVFAQVKQIYKTPPIKYFGGFNFSQILPDPSKPSKRSFIEDLLFNKVTLADAGFIKQYGDCLGDIAARDLICAQKFKGLTVLPPLLTDEMIAQYTSALLAGTITSGWTFGAGAALQIPFAMQMAYRFNGIGVTQNVLYENQKLIANQFNSAIGKIQDSLSSTASALGKLQDVVNHNAQALNTLVKQLSSKFGAISSVLNDIFSRLDPPEAEVQIDRLITGRLQSLQTYVTQQLIRAAEIRASANLAATKMSECVLGQSKRVDFCGKGYHLMSFPQSAPHGVVFLHVTYVPAQEKNFTTAPAICHDGKAHFPREGVFVSNGTHWFVTQRNFYEPQIITTDNTFVSGNCDVVIGIVNNTVYDPLQPELDSFKEELDKYFKNHTSPDVDLGDISGINASVVNIQKEIDRLNEVAKNLNESLIDLQELGKYEQYIKWPWYIWLGFIAGLIAIVMVTIMLCCMTSCCSCLKGCCSCGSCCKFDEDDSEPVLKGVKLHYT

SEQ ID NO: 49 - DNA, 3825 bp, SARS-CoV-2
atgttcgtgttcctggtgctgctgcctctggtgtccagccagtgtgtgaacctgaccaccagaacacagctgcctccagcctacaccaacagctttaccagaggcgtgtactaccccgacaaggtgttcagatccagcgtgctgcactctacccaggacctgttcctgcctttcttcagcaacgtgacctggttccacgccatccacgtgtccggcaccaatggcaccaagagattcgacaaccccgtgctgcccttcaacgacggggtgtactttgccagcaccgagaagtccaacatcatcagaggctggatcttcggcaccacactggacagcaagacccagagcctgctgatcgtgaacaacgccaccaacgtggtcatcaaagtgtgcgagttccagttctgcaacgaccccttcctgggcgtctactaccacaagaacaacaagagctggatggaaagcgagttccgggtgtacagcagcgccaacaactgcaccttcgagtacgtgtcccagcctttcctgatggacctggaaggcaagcagggcaacttcaagaacctgcgcgagttcgtgtttaagaacatcgacggctacttcaagatctacagcaagcacacccctatcaacctcgtgcgggatctgcctcagggcttctctgctctggaacccctggtggatctgcccatcggcatcaacatcacccggtttcagacactgctggccctgcacagaagctacctgacacctggcgatagcagcagcggatggacagctggtgccgccgcttactatgtgggctacctgcagcctagaaccttcctgctgaagtacaacgagaacggcaccatcaccgacgccgtggattgtgctctggatcctctgagcgagacaaagtgcaccctgaagtccttcaccgtggaaaagggcatctaccagaccagcaacttccgggtgcagcccaccgaatccatcgtgcggttccccaatatcaccaatctgtgccccttcggcgaggtgttcaatgccaccagattcgcctctgtgtacgcctggaaccggaagcggatcagcaattgcgtggccgactactccgtgctgtacaactccgccagcttcagcaccttcaagtgctacggcgtgtcccctaccaagctgaacgacctgtgcttcacaaacgtgtacgccgacagcttcgtgatccggggagatgaagtgcggcagattgcccctggacagacaggcaagatcgccgactacaactacaagctgcccgacgacttcaccggctgtgtgattgcctggaacagcaacaacctggactccaaagtcggcggcaactacaattacctgtaccggctgttccggaagtccaatctgaagcccttcgagcgggacatctccaccgagatctatcaggccggcagcaccccttgtaacggcgtggaaggcttcaactgctacttcccactgcagtcctacggctttcagcccacaaatggcgtgggctatcagccctacagagtggtggtgctgagcttcgaactgctgcatgcccctgccacagtgtgcggccctaagaaaagcaccaatctcgtgaagaacaaatgcgtgaacttcaacttcaacggcctgaccggcaccggcgtgctgacagagagcaacaagaagttcctgccattccagcagtttggccgggatatcgccgataccacagacgccgttagagatccccagacactggaaatcctggacatcaccccttgcagcttcggcggagtgtctgtgatcacccctggcaccaacaccagcaatcaggtggcagtgctgtaccaggacgtgaactgtaccgaagtgcccgtggccattcacgccgatcagctgacacctacatggcgggtgtactccaccggcagcaatgtgtttcagaccagagccggctgtctgatcggagccgagcacgtgaacaatagctacgagtgcgacatccccatcggcgctggaatctgcgccagctaccagacacagacaaacagccctcggagagccagaagcgtggccagccagagcatcattgcctacacaatgtctctgggcgccgagaacagcgtggcctactccaacaactctatcgctatccccaccaacttcaccatcagcgtgaccacagagatcctgcctgtgtccatgaccaagaccagcgtggactgcaccatgtacatctgcggcgattccaccgagtgctccaacctgctgctgcagtacggcagcttctgcacccagctgaatagagccctgacagggatcgccgtggaacaggacaagaacacccaagaggtgttcgcccaagtgaagcagatctacaagacccctcctatcaaggacttcggcggcttcaatttcagccagattctgcccgatcctagcaagcccagcaagcggagcttcatcgaggacctgctgttcaacaaagtgacactggccgacgccggcttcatcaagcagtatggcgattgtctgggcgacattgccgccagggatctgatttgcgcccagaagtttaacggactgacagtgctgcctcctctgctgaccgatgagatgatcgcccagtacacatctgccctgctggccggcacaatcacaagcggctggacatttggagcaggcgccgctctgcagatcccctttgctatgcagatggcctaccggttcaacggcatcggagtgacccagaatgtgctgtacgagaaccagaagctgatcgccaaccagttcaacagcgccatcggcaagatccaggacagcctgagcagcacagcaagcgccctgggaaagctgcaggacgtggtcaaccagaatgcccaggcactgaacaccctggtcaagcagctgtcctccaacttcggcgccatcagctctgtgctgaacgatatcctgagcagactggaccctcctgaggccgaggtgcagatcgacagactgatcacaggcagactgcagagcctccagacatacgtgacccagcagctgatcagagccgccgagattagagcctctgccaatctggccgccaccaagatgtctgagtgtgtgctgggccagagcaagagagtggacttttgcggcaagggctaccacctgatgagcttccctcagtctgcccctcacggcgtggtgtttctgcacgtgacatatgtgcccgctcaagagaagaatttcaccaccgctccagccatctgccacgacggcaaagcccactttcctagagaaggcgtgttcgtgtccaacggcacccattggttcgtgacacagcggaacttctacgagccccagatcatcaccaccgacaacaccttcgtgtctggcaactgcgacgtcgtgatcggcattgtgaacaataccgtgtacgaccctctgcagcccgagctggacagcttcaaagaggaactggacaagtactttaagaaccacacaagccccgacgtggacctgggcgatatcagcggaatcaatgccagcgtcgtgaacatccagaaagagatcgaccggctgaacgaggtggccaagaatctgaacgagagcctgatcgacctgcaagaactggggaagtacgagcagtacatcaagtggccctggtacatctggctgggctttatcgccggactgattgccatcgtgatggtcacaatcatgctgtgttgcatgaccagctgctgtagctgcctgaagggctgttgtagctgtggcagctgctgcaagttcgacgaggacgattctgagcccgtgctgaagggcgtgaaactgcactacacatgatga

SEQ ID NO: 50 - DNA, 3816 bp, SARS-CoV-2
atgttcgtgttcctggtgctgctgcctctggtgtccagccagtgtgtgaacctgaccaccagaacacagctgcctccagcctacaccaacagctttaccagaggcgtgtactaccccgacaaggtgttcagatccagcgtgctgcactctacccaggacctgttcctgcctttcttcagcaacgtgacctggttccacgccatctccggcaccaatggcaccaagagattcgacaaccccgtgctgcccttcaacgacggggtgtactttgccagcaccgagaagtccaacatcatcagaggctggatcttcggcaccacactggacagcaagacccagagcctgctgatcgtgaacaacgccaccaacgtggtcatcaaagtgtgcgagttccagttctgcaacgaccccttcctgggcgtctaccacaagaacaacaagagctggatggaaagcgagttccgggtgtacagcagcgccaacaactgcaccttcgagtacgtgtcccagcctttcctgatggacctggaaggcaagcagggcaacttcaagaacctgcgcgagttcgtgtttaagaacatcgacggctacttcaagatctacagcaagcacacccctatcaacctcgtgcgggatctgcctcagggcttctctgctctggaacccctggtggatctgcccatcggcatcaacatcacccggtttcagacactgctggccctgcacagaagctacctgacacctggcgatagcagcagcggatggacagctggtgccgccgcttactatgtgggctacctgcagcctagaaccttcctgctgaagtacaacgagaacggcaccatcaccgacgccgtggattgtgctctggatcctctgagcgagacaaagtgcaccctgaagtccttcaccgtggaaaagggcatctaccagaccagcaacttccgggtgcagcccaccgaatccatcgtgcggttccccaatatcaccaatctgtgccccttcggcgaggtgttcaatgccaccagattcgcctctgtgtacgcctggaaccggaagcggatcagcaattgcgtggccgactactccgtgctgtacaactccgccagcttcagcaccttcaagtgctacggcgtgtcccctaccaagctgaacgacctgtgcttcacaaacgtgtacgccgacagcttcgtgatccggggagatgaagtgcggcagattgcccctggacagacaggcaagatcgccgactacaactacaagctgcccgacgacttcaccggctgtgtgattgcctggaacagcaacaacctggactccaaagtcggcggcaactacaattacctgtaccggctgttccggaagtccaatctgaagcccttcgagcgggacatctccaccgagatctatcaggccggcagcaccccttgtaacggcgtggaaggcttcaactgctacttcccactgcagtcctacggctttcagcccacatacggcgtgggctatcagccctacagagtggtggtgctgagcttcgaactgctgcatgcccctgccacagtgtgcggccctaagaaaagcaccaatctcgtgaagaacaaatgcgtgaacttcaacttcaacggcctgaccggcaccggcgtgctgacagagagcaacaagaagttcctgccattccagcagtttggccgggatatcgacgataccacagacgccgttagagatccccagacactggaaatcctggacatcaccccttgcagcttcggcggagtgtctgtgatcacccctggcaccaacaccagcaatcaggtggcagtgctgtaccagggcgtgaactgtaccgaagtgcccgtggccattcacgccgatcagctgacacctacatggcgggtgtactccaccggcagcaatgtgtttcagaccagagccggctgtctgatcggagccgagcacgtgaacaatagctacgagtgcgacatccccatcggcgctggaatctgcgccagctaccagacacagacaaacagccaccggagagccagaagcgtggccagccagagcatcattgcctacacaatgtctctgggcgccgagaacagcgtggcctactccaacaactctatcgctatccccatcaacttcaccatcagcgtgaccacagagatcctgcctgtgtccatgaccaagaccagcgtggactgcaccatgtacatctgcggcgattccaccgagtgctccaacctgctgctgcagtacggcagcttctgcacccagctgaatagagccctgacagggatcgccgtggaacaggacaagaacacccaagaggtgttcgcccaagtgaagcagatctacaagacccctcctatcaaggacttcggcggcttcaatttcagccagattctgcccgatcctagcaagcccagcaagcggagcttcatcgaggacctgctgttcaacaaagtgacactggccgacgccggcttcatcaagcagtatggcgattgtctgggcgacattgccgccagggatctgatttgcgcccagaagtttaacggactgacagtgctgcctcctctgctgaccgatgagatgatcgcccagtacacatctgccctgctggccggcacaatcacaagcggctggacatttggagcaggcgccgctctgcagatcccctttgctatgcagatggcctaccggttcaacggcatcggagtgacccagaatgtgctgtacgagaaccagaagctgatcgccaaccagttcaacagcgccatcggcaagatccaggacagcctgagcagcacagcaagcgccctgggaaagctgcaggacgtggtcaaccagaatgcccaggcactgaacaccctggtcaagcagctgtcctccaacttcggcgccatcagctctgtgctgaacgatatcctggcaagactggaccctcctgaggccgaggtgcagatcgacagactgatcacaggcagactgcagagcctccagacatacgtgacccagcagctgatcagagccgccgagattagagcctctgccaatctggccgccaccaagatgtctgagtgtgtgctgggccagagcaagagagtggacttttgcggcaagggctaccacctgatgagcttccctcagtctgcccctcacggcgtggtgtttctgcacgtgacatatgtgcccgctcaagagaagaatttcaccaccgctccagccatctgccacgacggcaaagcccactttcctagagaaggcgtgttcgtgtccaacggcacccattggttcgtgacacagcggaacttctacgagccccagatcatcaccacccacaacaccttcgtgtctggcaactgcgacgtcgtgatcggcattgtgaacaataccgtgtacgaccctctgcagcccgagctggacagcttcaaagaggaactggacaagtactttaagaaccacacaagccccgacgtggacctgggcgatatcagcggaatcaatgccagcgtcgtgaacatccagaaagagatcgaccggctgaacgaggtggccaagaatctgaacgagagcctgatcgacctgcaagaactggggaagtacgagcagtacatcaagtggccctggtacatctggctgggctttatcgccggactgattgccatcgtgatggtcacaatcatgctgtgttgcatgaccagctgctgtagctgcctgaagggctgttgtagctgtggcagctgctgcaagttcgacgaggacgattctgagcccgtgctgaagggcgtgaaactgcactacacatgatga

SEQ ID NO: 51 - DNA, 3816 bp, SARS-CoV-2
atgttcgtgttcctggtgctgctgcctctggtgtccagccagtgtgtgaacttcaccaccagaacacagctgcctccagcctacaccaacagctttaccagaggcgtgtactaccccgacaaggtgttcagatccagcgtgctgcactctacccaggacctgttcctgcctttcttcagcaacgtgacctggttccacgccatccacgtgtccggcaccaatggcaccaagagattcgccaaccccgtgctgcccttcaacgacggggtgtactttgccagcaccgagaagtccaacatcatcagaggctggatcttcggcaccacactggacagcaagacccagagcctgctgatcgtgaacaacgccaccaacgtggtcatcaaagtgtgcgagttccagttctgcaacgaccccttcctgggcgtctactaccacaagaacaacaagagctggatggaaagcgagttccgggtgtacagcagcgccaacaactgcaccttcgagtacgtgtcccagcctttcctgatggacctggaaggcaagcagggcaacttcaagaacctgcgcgagttcgtgtttaagaacatcgacggctacttcaagatctacagcaagcacacccctatcaacctcgtgcggggtctgcctcagggcttctctgctctggaacccctggtggatctgcccatcggcatcaacatcacccggtttcagacactgcacagaagctacctgacacctggcgatagcagcagcggatggacagctggtgccgccgcttactatgtgggctacctgcagcctagaaccttcctgctgaagtacaacgagaacggcaccatcaccgacgccgtggattgtgctctggatcctctgagcgagacaaagtgcaccctgaagtccttcaccgtggaaaagggcatctaccagaccagcaacttccgggtgcagcccaccgaatccatcgtgcggttccccaatatcaccaatctgtgccccttcggcgaggtgttcaatgccaccagattcgcctctgtgtacgcctggaaccggaagcggatcagcaattgcgtggccgactactccgtgctgtacaactccgccagcttcagcaccttcaagtgctacggcgtgtcccctaccaagctgaacgacctgtgcttcacaaacgtgtacgccgacagcttcgtgatccggggagatgaagtgcggcagattgcccctggacagacaggcaatatcgccgactacaactacaagctgcccgacgacttcaccggctgtgtgattgcctggaacagcaacaacctggactccaaagtcggcggcaactacaattacctgtaccggctgttccggaagtccaatctgaagcccttcgagcgggacatctccaccgagatctatcaggccggcagcaccccttgtaacggcgtgaaaggcttcaactgctacttcccactgcagtcctacggctttcagcccacatacggcgtgggctatcagccctacagagtggtggtgctgagcttcgaactgctgcatgcccctgccacagtgtgcggccctaagaaaagcaccaatctcgtgaagaacaaatgcgtgaacttcaacttcaacggcctgaccggcaccggcgtgctgacagagagcaacaagaagttcctgccattccagcagtttggccgggatatcgccgataccacagacgccgttagagatccccagacactggaaatcctggacatcaccccttgcagcttcggcggagtgtctgtgatcacccctggcaccaacaccagcaatcaggtggcagtgctgtaccagggcgtgaactgtaccgaagtgcccgtggccattcacgccgatcagctgacacctacatggcgggtgtactccaccggcagcaatgtgtttcagaccagagccggctgtctgatcggagccgagcacgtgaacaatagctacgagtgcgacatccccatcggcgctggaatctgcgccagctaccagacacagacaaacagccctcggagagccagaagcgtggccagccagagcatcattgcctacacaatgtctctgggcgtggagaacagcgtggcctactccaacaactctatcgctatccccaccaacttcaccatcagcgtgaccacagagatcctgcctgtgtccatgaccaagaccagcgtggactgcaccatgtacatctgcggcgattccaccgagtgctccaacctgctgctgcagtacggcagcttctgcacccagctgaatagagccctgacagggatcgccgtggaacaggacaagaacacccaagaggtgttcgcccaagtgaagcagatctacaagacccctcctatcaaggacttcggcggcttcaatttcagccagattctgcccgatcctagcaagcccagcaagcggagcttcatcgaggacctgctgttcaacaaagtgacactggccgacgccggcttcatcaagcagtatggcgattgtctgggcgacattgccgccagggatctgatttgcgcccagaagtttaacggactgacagtgctgcctcctctgctgaccgatgagatgatcgcccagtacacatctgccctgctggccggcacaatcacaagcggctggacatttggagcaggcgccgctctgcagatcccctttgctatgcagatggcctaccggttcaacggcatcggagtgacccagaatgtgctgtacgagaaccagaagctgatcgccaaccagttcaacagcgccatcggcaagatccaggacagcctgagcagcacagcaagcgccctgggaaagctgcaggacgtggtcaaccagaatgcccaggcactgaacaccctggtcaagcagctgtcctccaacttcggcgccatcagctctgtgctgaacgatatcctgagcagactggaccctcctgaggccgaggtgcagatcgacagactgatcacaggcagactgcagagcctccagacatacgtgacccagcagctgatcagagccgccgagattagagcctctgccaatctggccgccaccaagatgtctgagtgtgtgctgggccagagcaagagagtggacttttgcggcaagggctaccacctgatgagcttccctcagtctgcccctcacggcgtggtgtttctgcacgtgacatatgtgcccgctcaagagaagaatttcaccaccgctccagccatctgccacgacggcaaagcccactttcctagagaaggcgtgttcgtgtccaacggcacccattggttcgtgacacagcggaacttctacgagccccagatcatcaccaccgacaacaccttcgtgtctggcaactgcgacgtcgtgatcggcattgtgaacaataccgtgtacgaccctctgcagcccgagctggacagcttcaaagaggaactggacaagtactttaagaaccacacaagccccgacgtggacctgggcgatatcagcggaatcaatgccagcgtcgtgaacatccagaaagagatcgaccggctgaacgaggtggccaagaatctgaacgagagcctgatcgacctgcaagaactggggaagtacgagcagtacatcaagtggccctggtacatctggctgggctttatcgccggactgattgccatcgtgatggtcacaatcatgctgtgttgcatgaccagctgctgtagctgcctgaagggctgttgtagctgtggcagctgctgcaagttcgacgaggacgattctgagcccgtgctgaagggcgtgaaactgcactacacatgatga

SEQ ID NO: 52 - DNA, 3825 bp, SARS-CoV-2
atgttcgtgttcctggtgctgctgcccctggtgagctcccagtgcgtgaactttacaaacagaacacagctgccctccgcctacacaaacagcttcaccaggggcgtgtactaccccgataaggtctttcggtccagcgtgctgcacagcacccaggatctgttcctgcctttcttcagcaacgtgacatggtttcacgccatccacgtgagcgggacaaacggcaccaagcggttcgataacccagtgctgccctttaacgatggggtgtacttcgccagcacagagaagtccaacatcatcaggggctggattttcggcaccaccctcgattccaagacacagtccctgctgatcgtgaacaacgccacaaacgtggtcattaaggtgtgcgagttccagttttgcaactacccattcctgggcgtgtactaccacaagaacaacaagtcctggatggagagcgagttcagggtctactcctccgccaacaactgcaccttcgagtacgtgagccagcccttcctgatggatctggagggcaagcaggggaacttcaagaacctgagcgagttcgtgttcaagaacattgacggctactttaagatctacagtaagcacacacctatcaacctggtgcgggacctgcctcagggcttctccgccctcgagccactggtggatctgccaatcggcattaacatcaccaggttccagacactgctggccctgcacaggagctacctgactccaggcgatagctccagcgggtggacagccggggccgccgcctactacgtgggctacctgcagcccagaacctttctgctgaagtacaacgagaacgggaccatcaccgatgccgtggattgcgccctggaccccctgagcgagaccaagtgcactctcaagtccttcaccgtggagaagggcatctaccagaccagcaacttccgggtccagcccacagagtccatcgtgaggttccccaacatcaccaacctctgccccttcggcgaggtgttcaacgccaccaggtttgccagcgtgtacgcctggaacaggaagaggatctccaactgcgtggccgattacagcgtgctgtacaactccgcctccttcagcaccttcaagtgctacggcgtgagccctaccaagcttaacgatctgtgctttacaaacgtgtacgccgatagctttgtgatccggggggacgaggtgaggcagattgcccccggccagacagggaccatcgccgattacaactacaagctgcccgatgacttcaccgggtgcgtgattgcctggaacagcaacaacctcgatagcaaggtcggggggaactacaactacctgtacaggctgtttagaaagtccaacctcaagcctttcgagcgggatattagcactgagatctaccaggccgggagcacaccctgcaacggggtgaagggcttcaactgctactttcccctgcagagctacggcttccagccaacatacggcgtggggtaccagccctaccgggtggtggtgctgagcttcgagctgctgcacgcccctgccaccgtgtgcggccccaagaaaagcactaacctggtgaagaacaagtgcgtcaacttcaactttaacggcctgaccggcacaggggtgctgaccgagtccaacaagaagttcctgcccttccagcagttcggccgggacatcgccgataccactgacgccgtgagggacccccagaccctggagatcctggacattacaccctgtagcttcggcggggtcagcgtgatcacacccggcaccaacacatccaaccaggtggccgtgctgtaccagggcgtgaactgcaccgaggtgcccgtcgccatccacgccgaccagctgacacccacatggagggtgtacagcacagggagcaacgtgttccagaccagggccgggtgcctgatcggcgccgagtacgtgaacaactcctacgagtgcgacatccccatcggggccggcatttgcgcctcctaccagacccagaccaacagcccccggcgggccaggagcgtggccagccagagcatcattgcctacacaatgtctctgggcgccgagaacagcgtggcctactccaacaactctatcgctatccccaccaacttcaccatcagcgtgaccacagagatcctgcctgtgtccatgaccaagaccagcgtggactgcaccatgtacatctgcggcgattccaccgagtgctccaacctgctgctgcagtacggcagcttctgcacccagctgaatagagccctgacagggatcgccgtggaacaggacaagaacacccaagaggtgttcgcccaagtgaagcagatctacaagacccctcctatcaaggacttcggcggcttcaatttcagccagattctgcccgatcctagcaagcccagcaagcggagcttcatcgaggacctgctgttcaacaaagtgacactggccgacgccggcttcatcaagcagtatggcgattgtctgggcgacattgccgccagggatctgatttgcgcccagaagtttaacggactgacagtgctgcctcctctgctgaccgatgagatgatcgcccagtacacatctgccctgctggccggcacaatcacaagcggctggacatttggagcaggcgccgctctgcagatcccctttgctatgcagatggcctaccggttcaacggcatcggagtgacccagaatgtgctgtacgagaaccagaagctgatcgccaaccagttcaacagcgccatcggcaagatccaggacagcctgagcagcacagcaagcgccctgggaaagctgcaggacgtggtcaaccagaatgcccaggcactgaacaccctggtcaagcagctgtcctccaacttcggcgccatcagctctgtgctgaacgatatcctgagcagactggaccctcctgaggccgaggtgcagatcgacagactgatcacaggcagactgcagagcctccagacatacgtgacccagcagctgatcagagccgccgagattagagcctctgccaatctggccgccatcaagatgtctgagtgtgtgctgggccagagcaagagagtggacttttgcggcaagggctaccacctgatgagcttccctcagtctgcccctcacggcgtggtgtttctgcacgtgacatatgtgcccgctcaagagaagaatttcaccaccgctccagccatctgccacgacggcaaagcccactttcctagagaaggcgtgttcgtgtccaacggcacccattggttcgtgacacagcggaacttctacgagccccagatcatcaccaccgacaacaccttcgtgtctggcaactgcgacgtcgtgatcggcattgtgaacaataccgtgtacgaccctctgcagcccgagctggacagcttcaaagaggaactggacaagtactttaagaaccacacaagccccgacgtggacctgggcgatatcagcggaatcaatgccagcttcgtgaacatccagaaagagatcgaccggctgaacgaggtggccaagaatctgaacgagagcctgatcgacctgcaagaactggggaagtacgagcagtacatcaagtggccctggtacatctggctgggctttatcgccggactgattgccatcgtgatggtcacaatcatgctgtgttgcatgaccagctgctgtagctgcctgaagggctgttgtagctgtggcagctgctgcaagttcgacgaggacgattctgagcccgtgctgaagggcgtgaaactgcactacacatgatga

SEQ ID NO: 53 - DNA, 3819 bp, SARS-CoV-2
atgttcgtgttcctggtgctgctgcctctggtgtccagccagtgtgtgaacctgagaaccagaacacagctgcctccagcctacaccaacagctttaccagaggcgtgtactaccccgacaaggtgttcagatccagcgtgctgcactctacccaggacctgttcctgcctttcttcagcaacgtgacctggttccacgccatccacgtgtccggcaccaatggcaccaagagattcgacaaccccgtgctgcccttcaacgacggggtgtactttgccagcaccgagaagtccaacatcatcagaggctggatcttcggcaccacactggacagcaagacccagagcctgctgatcgtgaacaacgccaccaacgtggtcatcaaagtgtgcgagttccagttctgcaacgaccccttcctggacgtctactaccacaagaacaacaagagctggatggaaagcggcgtgtacagcagcgccaacaactgcaccttcgagtacgtgtcccagcctttcctgatggacctggaaggcaagcagggcaacttcaagaacctgcgcgagttcgtgtttaagaacatcgacggctacttcaagatctacagcaagcacacccctatcaacctcgtgcgggatctgcctcagggcttctctgctctggaacccctggtggatctgcccatcggcatcaacatcacccggtttcagacactgctggccctgcacagaagctacctgacacctggcgatagcagcagcggatggacagctggtgccgccgcttactatgtgggctacctgcagcctagaaccttcctgctgaagtacaacgagaacggcaccatcaccgacgccgtggattgtgctctggatcctctgagcgagacaaagtgcaccctgaagtccttcaccgtggaaaagggcatctaccagaccagcaacttccgggtgcagcccaccgaatccatcgtgcggttccccaatatcaccaatctgtgccccttcggcgaggtgttcaatgccaccagattcgcctctgtgtacgcctggaaccggaagcggatcagcaattgcgtggccgactactccgtgctgtacaactccgccagcttcagcaccttcaagtgctacggcgtgtcccctaccaagctgaacgacctgtgcttcacaaacgtgtacgccgacagcttcgtgatccggggagatgaagtgcggcagattgcccctggacagacaggcaagatcgccgactacaactacaagctgcccgacgacttcaccggctgtgtgattgcctggaacagcaacaacctggactccaaagtcggcggcaactacaattaccggtaccggctgttccggaagtccaatctgaagcccttcgagcgggacatctccaccgagatctatcaggccggcagcaagccttgtaacggcgtggaaggcttcaactgctacttcccactgcagtcctacggctttcagcccacaaatggcgtgggctatcagccctacagagtggtggtgctgagcttcgaactgctgcatgcccctgccacagtgtgcggccctaagaaaagcaccaatctcgtgaagaacaaatgcgtgaacttcaacttcaacggcctgaccggcaccggcgtgctgacagagagcaacaagaagttcctgccattccagcagtttggccgggatatcgccgataccacagacgccgttagagatccccagacactggaaatcctggacatcaccccttgcagcttcggcggagtgtctgtgatcacccctggcaccaacaccagcaatcaggtggcagtgctgtaccagggcgtgaactgtaccgaagtgcccgtggccattcacgccgatcagctgacacctacatggcgggtgtactccaccggcagcaatgtgtttcagaccagagccggctgtctgatcggagccgagcacgtgaacaatagctacgagtgcgacatccccatcggcgctggaatctgcgccagctaccagacacagacaaacagccggcggagagccagaagcgtggccagccagagcatcattgcctacacaatgtctctgggcgccgagaacagcgtggcctactccaacaactctatcgctatccccaccaacttcaccatcagcgtgaccacagagatcctgcctgtgtccatgaccaagaccagcgtggactgcaccatgtacatctgcggcgattccaccgagtgctccaacctgctgctgcagtacggcagcttctgcacccagctgaatagagccctgacagggatcgccgtggaacaggacaagaacacccaagaggtgttcgcccaagtgaagcagatctacaagacccctcctatcaaggacttcggcggcttcaatttcagccagattctgcccgatcctagcaagcccagcaagcggagcttcatcgaggacctgctgttcaacaaagtgacactggccgacgccggcttcatcaagcagtatggcgattgtctgggcgacattgccgccagggatctgatttgcgcccagaagtttaacggactgacagtgctgcctcctctgctgaccgatgagatgatcgcccagtacacatctgccctgctggccggcacaatcacaagcggctggacatttggagcaggcgccgctctgcagatcccctttgctatgcagatggcctaccggttcaacggcatcggagtgacccagaatgtgctgtacgagaaccagaagctgatcgccaaccagttcaacagcgccatcggcaagatccaggacagcctgagcagcacagcaagcgccctgggaaagctgcagaacgtggtcaaccagaatgcccaggcactgaacaccctggtcaagcagctgtcctccaacttcggcgccatcagctctgtgctgaacgatatcctgagcagactggaccctcctgaggccgaggtgcagatcgacagactgatcacaggcagactgcagagcctccagacatacgtgacccagcagctgatcagagccgccgagattagagcctctgccaatctggccgccaccaagatgtctgagtgtgtgctgggccagagcaagagagtggacttttgcggcaagggctaccacctgatgagcttccctcagtctgcccctcacggcgtggtgtttctgcacgtgacatatgtgcccgctcaagagaagaatttcaccaccgctccagccatctgccacgacggcaaagcccactttcctagagaaggcgtgttcgtgtccaacggcacccattggttcgtgacacagcggaacttctacgagccccagatcatcaccaccgacaacaccttcgtgtctggcaactgcgacgtcgtgatcggcattgtgaacaataccgtgtacgaccctctgcagcccgagctggacagcttcaaagaggaactggacaagtactttaagaaccacacaagccccgacgtggacctgggcgatatcagcggaatcaatgccagcgtcgtgaacatccagaaagagatcgaccggctgaacgaggtggccaagaatctgaacgagagcctgatcgacctgcaagaactggggaagtacgagcagtacatcaagtggccctggtacatctggctgggctttatcgccggactgattgccatcgtgatggtcacaatcatgctgtgttgcatgaccagctgctgtagctgcctgaagggctgttgtagctgtggcagctgctgcaagttcgacgaggacgattctgagcccgtgctgaagggcgtgaaactgcactacacatgatga

SEQ ID NO: 54 - DNA, 3825 bp, SARS-CoV-2
atgttcgtgttcctggtgctgctgcctctggtgtccatccagtgtgtgaacctgaccaccagaacacagctgcctccagcctacaccaacagctttaccagaggcgtgtactaccccgacaaggtgttcagatccagcgtgctgcactctacccaggacctgttcctgcctttcttcagcaacgtgacctggttccacgccatccacgtgtccggcaccaatggcaccaagagattcgacaaccccgtgctgcccttcaacgacggggtgtactttgccagcaccgagaagtccaacatcatcagaggctggatcttcggcaccacactggacagcaagacccagagcctgctgatcgtgaacaacgccaccaacgtggtcatcaaagtgtgcgagttccagttctgcaacgaccccttcctgggcgtctactaccacaagaacaacaagagctgcatggaaagcgagttccgggtgtacagcagcgccaacaactgcaccttcgagtacgtgtcccagcctttcctgatggacctggaaggcaagcagggcaacttcaagaacctgcgcgagttcgtgtttaagaacatcgacggctacttcaagatctacagcaagcacacccctatcaacctcgtgcgggatctgcctcagggcttctctgctctggaacccctggtggatctgcccatcggcatcaacatcacccggtttcagacactgctggccctgcacagaagctacctgacacctggcgatagcagcagcggatggacagctggtgccgccgcttactatgtgggctacctgcagcctagaaccttcctgctgaagtacaacgagaacggcaccatcaccgacgccgtggattgtgctctggatcctctgagcgagacaaagtgcaccctgaagtccttcaccgtggaaaagggcatctaccagaccagcaacttccgggtgcagcccaccgaatccatcgtgcggttccccaatatcaccaatctgtgccccttcggcgaggtgttcaatgccaccagattcgcctctgtgtacgcctggaaccggaagcggatcagcaattgcgtggccgactactccgtgctgtacaactccgccagcttcagcaccttcaagtgctacggcgtgtcccctaccaagctgaacgacctgtgcttcacaaacgtgtacgccgacagcttcgtgatccggggagatgaagtgcggcagattgcccctggacagacaggcaagatcgccgactacaactacaagctgcccgacgacttcaccggctgtgtgattgcctggaacagcaacaacctggactccaaagtcggcggcaactacaattaccgctaccggctgttccggaagtccaatctgaagcccttcgagcgggacatctccaccgagatctatcaggccggcagcaccccttgtaacggcgtggaaggcttcaactgctacttcccactgcagtcctacggctttcagcccacaaatggcgtgggctatcagccctacagagtggtggtgctgagcttcgaactgctgcatgcccctgccacagtgtgcggccctaagaaaagcaccaatctcgtgaagaacaaatgcgtgaacttcaacttcaacggcctgaccggcaccggcgtgctgacagagagcaacaagaagttcctgccattccagcagtttggccgggatatcgccgataccacagacgccgttagagatccccagacactggaaatcctggacatcaccccttgcagcttcggcggagtgtctgtgatcacccctggcaccaacaccagcaatcaggtggcagtgctgtaccagggcgtgaactgtaccgaagtgcccgtggccattcacgccgatcagctgacacctacatggcgggtgtactccaccggcagcaatgtgtttcagaccagagccggctgtctgatcggagccgagcacgtgaacaatagctacgagtgcgacatccccatcggcgctggaatctgcgccagctaccagacacagacaaacagccctcggagagccagaagcgtggccagccagagcatcattgcctacacaatgtctctgggcgccgagaacagcgtggcctactccaacaactctatcgctatccccaccaacttcaccatcagcgtgaccacagagatcctgcctgtgtccatgaccaagaccagcgtggactgcaccatgtacatctgcggcgattccaccgagtgctccaacctgctgctgcagtacggcagcttctgcacccagctgaatagagccctgacagggatcgccgtggaacaggacaagaacacccaagaggtgttcgcccaagtgaagcagatctacaagacccctcctatcaaggacttcggcggcttcaatttcagccagattctgcccgatcctagcaagcccagcaagcggagcttcatcgaggacctgctgttcaacaaagtgacactggccgacgccggcttcatcaagcagtatggcgattgtctgggcgacattgccgccagggatctgatttgcgcccagaagtttaacggactgacagtgctgcctcctctgctgaccgatgagatgatcgcccagtacacatctgccctgctggccggcacaatcacaagcggctggacatttggagcaggcgccgctctgcagatcccctttgctatgcagatggcctaccggttcaacggcatcggagtgacccagaatgtgctgtacgagaaccagaagctgatcgccaaccagttcaacagcgccatcggcaagatccaggacagcctgagcagcacagcaagcgccctgggaaagctgcaggacgtggtcaaccagaatgcccaggcactgaacaccctggtcaagcagctgtcctccaacttcggcgccatcagctctgtgctgaacgatatcctgagcagactggaccctcctgaggccgaggtgcagatcgacagactgatcacaggcagactgcagagcctccagacatacgtgacccagcagctgatcagagccgccgagattagagcctctgccaatctggccgccaccaagatgtctgagtgtgtgctgggccagagcaagagagtggacttttgcggcaagggctaccacctgatgagcttccctcagtctgcccctcacggcgtggtgtttctgcacgtgacatatgtgcccgctcaagagaagaatttcaccaccgctccagccatctgccacgacggcaaagcccactttcctagagaaggcgtgttcgtgtccaacggcacccattggttcgtgacacagcggaacttctacgagccccagatcatcaccaccgacaacaccttcgtgtctggcaactgcgacgtcgtgatcggcattgtgaacaataccgtgtacgaccctctgcagcccgagctggacagcttcaaagaggaactggacaagtactttaagaaccacacaagccccgacgtggacctgggcgatatcagcggaatcaatgccagcgtcgtgaacatccagaaagagatcgaccggctgaacgaggtggccaagaatctgaacgagagcctgatcgacctgcaagaactggggaagtacgagcagtacatcaagtggccctggtacatctggctgggctttatcgccggactgattgccatcgtgatggtcacaatcatgctgtgttgcatgaccagctgctgtagctgcctgaagggctgttgtagctgtggcagctgctgcaagttcgacgaggacgattctgagcccgtgctgaagggcgtgaaactgcactacacatgatga

SEQ ID NO: 55 - DNA, 3816 bp, SARS-CoV-2
atgttcgtgttcctggtgctgctgcctctggtgtccagccagtgtgtgaacctgaccaccagaacacagctgcctccagcctacaccaacagctttaccagaggcgtgtactaccccgacaaggtgttcagatccagcgtgctgcactctacccaggacctgttcctgcctttcttcagcaacgtgacctggttccacgtgatctccggcaccaatggcaccaagagattcgacaaccccgtgctgcccttcaacgacggggtgtactttgccagcatcgagaagtccaacatcatcagaggctggatcttcggcaccacactggacagcaagacccagagcctgctgatcgtgaacaacgccaccaacgtggtcatcaaagtgtgcgagttccagttctgcaacgaccccttcctggaccacaagaacaacaagagctggatggaaagcgagttccgggtgtacagcagcgccaacaactgcaccttcgagtacgtgtcccagcctttcctgatggacctggaaggcaagcagggcaacttcaagaacctgcgcgagttcgtgtttaagaacatcgacggctacttcaagatctacagcaagcacacccctatcatcgtgcgggaacctgaagatctgcctcagggcttctctgctctggaacccctggtggatctgcccatcggcatcaacatcacccggtttcagacactgctggccctgcacagaagctacctgacacctggcgatagcagcagcggatggacagctggtgccgccgcttactatgtgggctacctgcagcctagaaccttcctgctgaagtacaacgagaacggcaccatcaccgacgccgtggattgtgctctggatcctctgagcgagacaaagtgcaccctgaagtccttcaccgtggaaaagggcatctaccagaccagcaacttccgggtgcagcccaccgaatccatcgtgcggttccccaatatcaccaatctgtgccccttcgacgaggtgttcaatgccaccagattcgcctctgtgtacgcctggaaccggaagcggatcagcaattgcgtggccgactactccgtgctgtacaacctggcccccttcttcaccttcaagtgctacggcgtgtcccctaccaagctgaacgacctgtgcttcacaaacgtgtacgccgacagcttcgtgatccggggagatgaagtgcggcagattgcccctggacagacaggcaacatcgccgactacaactacaagctgcccgacgacttcaccggctgtgtgattgcctggaacagcaacaagctggactccaaagtctccggcaactacaattacctgtaccggctgttccggaagtccaatctgaagcccttcgagcgggacatctccaccgagatctatcaggccggcaacaagccttgtaacggcgtggccggcttcaactgctacttcccactgcggtcctactcctttcggcccacatatggcgtgggccatcagccctacagagtggtggtgctgagcttcgaactgctgcatgcccctgccacagtgtgcggccctaagaaaagcaccaatctcgtgaagaacaaatgcgtgaacttcaacttcaacggcctgaagggcaccggcgtgctgacagagagcaacaagaagttcctgccattccagcagtttggccgggatatcgccgataccacagacgccgttagagatccccagacactggaaatcctggacatcaccccttgcagcttcggcggagtgtctgtgatcacccctggcaccaacaccagcaatcaggtggcagtgctgtaccagggcgtgaactgtaccgaagtgcccgtggccattcacgccgatcagctgacacctacatggcgggtgtactccaccggcagcaatgtgtttcagaccagagccggctgtctgatcggagccgagtacgtgaacaatagctacgagtgcgacatccccatcggcgctggaatctgcgccagctaccagacacagacaaagagccatcggagagccagaagcgtggccagccagagcatcattgcctacacaatgtctctgggcgccgagaacagcgtggcctactccaacaactctatcgctatccccaccaacttcaccatcagcgtgaccacagagatcctgcctgtgtccatgaccaagaccagcgtggactgcaccatgtacatctgcggcgattccaccgagtgctccaacctgctgctgcagtacggcagcttctgcacccagctgaagagagccctgacagggatcgccgtggaacaggacaagaacacccaagaggtgttcgcccaagtgaagcagatctacaagacccctcctatcaagtacttcggcggcttcaatttcagccagattctgcccgatcctagcaagcccagcaagcggagcttcatcgaggacctgctgttcaacaaagtgacactggccgacgccggcttcatcaagcagtatggcgattgtctgggcgacattgccgccagggatctgatttgcgcccagaagtttaagggactgacagtgctgcctcctctgctgaccgatgagatgatcgcccagtacacatctgccctgctggccggcacaatcacaagcggctggacatttggagcaggcgccgctctgcagatcccctttgctatgcagatggcctaccggttcaacggcatcggagtgacccagaatgtgctgtacgagaaccagaagctgatcgccaaccagttcaacagcgccatcggcaagatccaggacagcctgagcagcacagcaagcgccctgggaaagctgcaggacgtggtcaaccacaatgcccaggcactgaacaccctggtcaagcagctgtcctccaagttcggcgccatcagctctgtgctgaacgatatcttcagcagactggaccctcctgaggccgaggtgcagatcgacagactgatcacaggcagactgcagagcctccagacatacgtgacccagcagctgatcagagccgccgagattagagcctctgccaatctggccgccaccaagatgtctgagtgtgtgctgggccagagcaagagagtggacttttgcggcaagggctaccacctgatgagcttccctcagtctgcccctcacggcgtggtgtttctgcacgtgacatatgtgcccgctcaagagaagaatttcaccaccgctccagccatctgccacgacggcaaagcccactttcctagagaaggcgtgttcgtgtccaacggcacccattggttcgtgacacagcggaacttctacgagccccagatcatcaccaccgacaacaccttcgtgtctggcaactgcgacgtcgtgatcggcattgtgaacaataccgtgtacgaccctctgcagcccgagctggacagcttcaaagaggaactggacaagtactttaagaaccacacaagccccgacgtggacctgggcgatatcagcggaatcaatgccagcgtcgtgaacatccagaaagagatcgaccggctgaacgaggtggccaagaatctgaacgagagcctgatcgacctgcaagaactggggaagtacgagcagtacatcaagtggccctggtacatctggctgggctttatcgccggactgattgccatcgtgatggtcacaatcatgctgtgttgcatgaccagctgctgtagctgcctgaagggctgttgtagctgtggcagctgctgcaagttcgacgaggacgattctgagcccgtgctgaagggcgtgaaactgcactacacatgatga

SEQ ID NO: 56 - RNA, 3825 nt, SARS-CoV-2
auguucguguuccuggugcugcugccucugguguccagccagugugugaaccugaccaccagaacacagcugccuccagccuacaccaacagcuuuaccagaggcguguacuaccccgacaagguguucagauccagcgugcugcacucuacccaggaccuguuccugccuuucuucagcaacgugaccugguuccacgccauccacguguccggcaccaauggcaccaagagauucgacaaccccgugcugcccuucaacgacgggguguacuuugccagcaccgagaaguccaacaucaucagaggcuggaucuucggcaccacacuggacagcaagacccagagccugcugaucgugaacaacgccaccaacguggucaucaaagugugcgaguuccaguucugcaacgaccccuuccugggcgucuacuaccacaagaacaacaagagcuggauggaaagcgaguuccggguguacagcagcgccaacaacugcaccuucgaguacgugucccagccuuuccugauggaccuggaaggcaagcagggcaacuucaagaaccugcgcgaguucguguuuaagaacaucgacggcuacuucaagaucuacagcaagcacaccccuaucaaccucgugcgggaucugccucagggcuucucugcucuggaaccccugguggaucugcccaucggcaucaacaucacccgguuucagacacugcuggcccugcacagaagcuaccugacaccuggcgauagcagcagcggauggacagcuggugccgccgcuuacuaugugggcuaccugcagccuagaaccuuccugcugaaguacaacgagaacggcaccaucaccgacgccguggauugugcucuggauccucugagcgagacaaagugcacccugaaguccuucaccguggaaaagggcaucuaccagaccagcaacuuccgggugcagcccaccgaauccaucgugcgguuccccaauaucaccaaucugugccccuucggcgagguguucaaugccaccagauucgccucuguguacgccuggaaccggaagcggaucagcaauugcguggccgacuacuccgugcuguacaacuccgccagcuucagcaccuucaagugcuacggcguguccccuaccaagcugaacgaccugugcuucacaaacguguacgccgacagcuucgugauccggggagaugaagugcggcagauugccccuggacagacaggcaagaucgccgacuacaacuacaagcugcccgacgacuucaccggcugugugauugccuggaacagcaacaaccuggacuccaaagucggcggcaacuacaauuaccuguaccggcuguuccggaaguccaaucugaagcccuucgagcgggacaucuccaccgagaucuaucaggccggcagcaccccuuguaacggcguggaaggcuucaacugcuacuucccacugcaguccuacggcuuucagcccacaaauggcgugggcuaucagcccuacagagugguggugcugagcuucgaacugcugcaugccccugccacagugugcggcccuaagaaaagcaccaaucucgugaagaacaaaugcgugaacuucaacuucaacggccugaccggcaccggcgugcugacagagagcaacaagaaguuccugccauuccagcaguuuggccgggauaucgccgauaccacagacgccguuagagauccccagacacuggaaauccuggacaucaccccuugcagcuucggcggagugucugugaucaccccuggcaccaacaccagcaaucagguggcagugcuguaccaggacgugaacuguaccgaagugcccguggccauucacgccgaucagcugacaccuacauggcggguguacuccaccggcagcaauguguuucagaccagagccggcugucugaucggagccgagcacgugaacaauagcuacgagugcgacauccccaucggcgcuggaaucugcgccagcuaccagacacagacaaacagcccucggagagccagaagcguggccagccagagcaucauugccuacacaaugucucugggcgccgagaacagcguggccuacuccaacaacucuaucgcuauccccaccaacuucaccaucagcgugaccacagagauccugccuguguccaugaccaagaccagcguggacugcaccauguacaucugcggcgauuccaccgagugcuccaaccugcugcugcaguacggcagcuucugcacccagcugaauagagcccugacagggaucgccguggaacaggacaagaacacccaagagguguucgcccaagugaagcagaucuacaagaccccuccuaucaaggacuucggcggcuucaauuucagccagauucugcccgauccuagcaagcccagcaagcggagcuucaucgaggaccugcuguucaacaaagugacacuggccgacgccggcuucaucaagcaguauggcgauugucugggcgacauugccgccagggaucugauuugcgcccagaaguuuaacggacugacagugcugccuccucugcugaccgaugagaugaucgcccaguacacaucugcccugcuggccggcacaaucacaagcggcuggacauuuggagcaggcgccgcucugcagauccccuuugcuaugcagauggccuaccgguucaacggcaucggagugacccagaaugugcuguacgagaaccagaagcugaucgccaaccaguucaacagcgccaucggcaagauccaggacagccugagcagcacagcaagcgcccugggaaagcugcaggacguggucaaccagaaugcccaggcacugaacacccuggucaagcagcuguccuccaacuucggcgccaucagcucugugcugaacgauauccugagcagacuggacccuccugaggccgaggugcagaucgacagacugaucacaggcagacugcagagccuccagacauacgugacccagcagcugaucagagccgccgagauuagagccucugccaaucuggccgccaccaagaugucugagugugugcugggccagagcaagagaguggacuuuugcggcaagggcuaccaccugaugagcuucccucagucugccccucacggcgugguguuucugcacgugacauaugugcccgcucaagagaagaauuucaccaccgcuccagccaucugccacgacggcaaagcccacuuuccuagagaaggcguguucguguccaacggcacccauugguucgugacacagcggaacuucuacgagccccagaucaucaccaccgacaacaccuucgugucuggcaacugcgacgucgugaucggcauugugaacaauaccguguacgacccucugcagcccgagcuggacagcuucaaagaggaacuggacaaguacuuuaagaaccacacaagccccgacguggaccugggcgauaucagcggaaucaaugccagcgucgugaacauccagaaagagaucgaccggcugaacgagguggccaagaaucugaacgagagccugaucgaccugcaagaacuggggaaguacgagcaguacaucaaguggcccugguacaucuggcugggcuuuaucgccggacugauugccaucgugauggucacaaucaugcuguguugcaugaccagcugcuguagcugccugaagggcuguuguagcuguggcagcugcugcaaguucgacgaggacgauucugagcccgugcugaagggcgugaaacugcacuacacaugauga

SEQ ID NO: 57 - RNA, 3816 nt, SARS-CoV-2
auguucguguuccuggugcugcugccucugguguccagccagugugugaaccugaccaccagaacacagcugccuccagccuacaccaacagcuuuaccagaggcguguacuaccccgacaagguguucagauccagcgugcugcacucuacccaggaccuguuccugccuuucuucagcaacgugaccugguuccacgccaucuccggcaccaauggcaccaagagauucgacaaccccgugcugcccuucaacgacgggguguacuuugccagcaccgagaaguccaacaucaucagaggcuggaucuucggcaccacacuggacagcaagacccagagccugcugaucgugaacaacgccaccaacguggucaucaaagugugcgaguuccaguucugcaacgaccccuuccugggcgucuaccacaagaacaacaagagcuggauggaaagcgaguuccggguguacagcagcgccaacaacugcaccuucgaguacgugucccagccuuuccugauggaccuggaaggcaagcagggcaacuucaagaaccugcgcgaguucguguuuaagaacaucgacggcuacuucaagaucuacagcaagcacaccccuaucaaccucgugcgggaucugccucagggcuucucugcucuggaaccccugguggaucugcccaucggcaucaacaucacccgguuucagacacugcuggcccugcacagaagcuaccugacaccuggcgauagcagcagcggauggacagcuggugccgccgcuuacuaugugggcuaccugcagccuagaaccuuccugcugaaguacaacgagaacggcaccaucaccgacgccguggauugugcucuggauccucugagcgagacaaagugcacccugaaguccuucaccguggaaaagggcaucuaccagaccagcaacuuccgggugcagcccaccgaauccaucgugcgguuccccaauaucaccaaucugugccccuucggcgagguguucaaugccaccagauucgccucuguguacgccuggaaccggaagcggaucagcaauugcguggccgacuacuccgugcuguacaacuccgccagcuucagcaccuucaagugcuacggcguguccccuaccaagcugaacgaccugugcuucacaaacguguacgccgacagcuucgugauccggggagaugaagugcggcagauugccccuggacagacaggcaagaucgccgacuacaacuacaagcugcccgacgacuucaccggcugugugauugccuggaacagcaacaaccuggacuccaaagucggcggcaacuacaauuaccuguaccggcuguuccggaaguccaaucugaagcccuucgagcgggacaucuccaccgagaucuaucaggccggcagcaccccuuguaacggcguggaaggcuucaacugcuacuucccacugcaguccuacggcuuucagcccacauacggcgugggcuaucagcccuacagagugguggugcugagcuucgaacugcugcaugccccugccacagugugcggcccuaagaaaagcaccaaucucgugaagaacaaaugcgugaacuucaacuucaacggccugaccggcaccggcgugcugacagagagcaacaagaaguuccugccauuccagcaguuuggccgggauaucgacgauaccacagacgccguuagagauccccagacacuggaaauccuggacaucaccccuugcagcuucggcggagugucugugaucaccccuggcaccaacaccagcaaucagguggcagugcuguaccagggcgugaacuguaccgaagugcccguggccauucacgccgaucagcugacaccuacauggcggguguacuccaccggcagcaauguguuucagaccagagccggcugucugaucggagccgagcacgugaacaauagcuacgagugcgacauccccaucggcgcuggaaucugcgccagcuaccagacacagacaaacagccaccggagagccagaagcguggccagccagagcaucauugccuacacaaugucucugggcgccgagaacagcguggccuacuccaacaacucuaucgcuauccccaucaacuucaccaucagcgugaccacagagauccugccuguguccaugaccaagaccagcguggacugcaccauguacaucugcggcgauuccaccgagugcuccaaccugcugcugcaguacggcagcuucugcacccagcugaauagagcccugacagggaucgccguggaacaggacaagaacacccaagagguguucgcccaagugaagcagaucuacaagaccccuccuaucaaggacuucggcggcuucaauuucagccagauucugcccgauccuagcaagcccagcaagcggagcuucaucgaggaccugcuguucaacaaagugacacuggccgacgccggcuucaucaagcaguauggcgauugucugggcgacauugccgccagggaucugauuugcgcccagaaguuuaacggacugacagugcugccuccucugcugaccgaugagaugaucgcccaguacacaucugcccugcuggccggcacaaucacaagcggcuggacauuuggagcaggcgccgcucugcagauccccuuugcuaugcagauggccuaccgguucaacggcaucggagugacccagaaugugcuguacgagaaccagaagcugaucgccaaccaguucaacagcgccaucggcaagauccaggacagccugagcagcacagcaagcgcccugggaaagcugcaggacguggucaaccagaaugcccaggcacugaacacccuggucaagcagcuguccuccaacuucggcgccaucagcucugugcugaacgauauccuggcaagacuggacccuccugaggccgaggugcagaucgacagacugaucacaggcagacugcagagccuccagacauacgugacccagcagcugaucagagccgccgagauuagagccucugccaaucuggccgccaccaagaugucugagugugugcugggccagagcaagagaguggacuuuugcggcaagggcuaccaccugaugagcuucccucagucugccccucacggcgugguguuucugcacgugacauaugugcccgcucaagagaagaauuucaccaccgcuccagccaucugccacgacggcaaagcccacuuuccuagagaaggcguguucguguccaacggcacccauugguucgugacacagcggaacuucuacgagccccagaucaucaccacccacaacaccuucgugucuggcaacugcgacgucgugaucggcauugugaacaauaccguguacgacccucugcagcccgagcuggacagcuucaaagaggaacuggacaaguacuuuaagaaccacacaagccccgacguggaccugggcgauaucagcggaaucaaugccagcgucgugaacauccagaaagagaucgaccggcugaacgagguggccaagaaucugaacgagagccugaucgaccugcaagaacuggggaaguacgagcaguacaucaaguggcccugguacaucuggcugggcuuuaucgccggacugauugccaucgugauggucacaaucaugcuguguugcaugaccagcugcuguagcugccugaagggcuguuguagcuguggcagcugcugcaaguucgacgaggacgauucugagcccgugcugaagggcgugaaacugcacuacacaugauga

SEQ ID NO: 58 - RNA, 3816 nt, SARS-CoV-2
auguucguguuccuggugcugcugccucugguguccagccagugugugaacuucaccaccagaacacagcugccuccagccuacaccaacagcuuuaccagaggcguguacuaccccgacaagguguucagauccagcgugcugcacucuacccaggaccuguuccugccuuucuucagcaacgugaccugguuccacgccauccacguguccggcaccaauggcaccaagagauucgccaaccccgugcugcccuucaacgacgggguguacuuugccagcaccgagaaguccaacaucaucagaggcuggaucuucggcaccacacuggacagcaagacccagagccugcugaucgugaacaacgccaccaacguggucaucaaagugugcgaguuccaguucugcaacgaccccuuccugggcgucuacuaccacaagaacaacaagagcuggauggaaagcgaguuccggguguacagcagcgccaacaacugcaccuucgaguacgugucccagccuuuccugauggaccuggaaggcaagcagggcaacuucaagaaccugcgcgaguucguguuuaagaacaucgacggcuacuucaagaucuacagcaagcacaccccuaucaaccucgugcggggucugccucagggcuucucugcucuggaaccccugguggaucugcccaucggcaucaacaucacccgguuucagacacugcacagaagcuaccugacaccuggcgauagcagcagcggauggacagcuggugccgccgcuuacuaugugggcuaccugcagccuagaaccuuccugcugaaguacaacgagaacggcaccaucaccgacgccguggauugugcucuggauccucugagcgagacaaagugcacccugaaguccuucaccguggaaaagggcaucuaccagaccagcaacuuccgggugcagcccaccgaauccaucgugcgguuccccaauaucaccaaucugugccccuucggcgagguguucaaugccaccagauucgccucuguguacgccuggaaccggaagcggaucagcaauugcguggccgacuacuccgugcuguacaacuccgccagcuucagcaccuucaagugcuacggcguguccccuaccaagcugaacgaccugugcuucacaaacguguacgccgacagcuucgugauccggggagaugaagugcggcagauugccccuggacagacaggcaauaucgccgacuacaacuacaagcugcccgacgacuucaccggcugugugauugccuggaacagcaacaaccuggacuccaaagucggcggcaacuacaauuaccuguaccggcuguuccggaaguccaaucugaagcccuucgagcgggacaucuccaccgagaucuaucaggccggcagcaccccuuguaacggcgugaaaggcuucaacugcuacuucccacugcaguccuacggcuuucagcccacauacggcgugggcuaucagcccuacagagugguggugcugagcuucgaacugcugcaugccccugccacagugugcggcccuaagaaaagcaccaaucucgugaagaacaaaugcgugaacuucaacuucaacggccugaccggcaccggcgugcugacagagagcaacaagaaguuccugccauuccagcaguuuggccgggauaucgccgauaccacagacgccguuagagauccccagacacuggaaauccuggacaucaccccuugcagcuucggcggagugucugugaucaccccuggcaccaacaccagcaaucagguggcagugcuguaccagggcgugaacuguaccgaagugcccguggccauucacgccgaucagcugacaccuacauggcggguguacuccaccggcagcaauguguuucagaccagagccggcugucugaucggagccgagcacgugaacaauagcuacgagugcgacauccccaucggcgcuggaaucugcgccagcuaccagacacagacaaacagcccucggagagccagaagcguggccagccagagcaucauugccuacacaaugucucugggcguggagaacagcguggccuacuccaacaacucuaucgcuauccccaccaacuucaccaucagcgugaccacagagauccugccuguguccaugaccaagaccagcguggacugcaccauguacaucugcggcgauuccaccgagugcuccaaccugcugcugcaguacggcagcuucugcacccagcugaauagagcccugacagggaucgccguggaacaggacaagaacacccaagagguguucgcccaagugaagcagaucuacaagaccccuccuaucaaggacuucggcggcuucaauuucagccagauucugcccgauccuagcaagcccagcaagcggagcuucaucgaggaccugcuguucaacaaagugacacuggccgacgccggcuucaucaagcaguauggcgauugucugggcgacauugccgccagggaucugauuugcgcccagaaguuuaacggacugacagugcugccuccucugcugaccgaugagaugaucgcccaguacacaucugcccugcuggccggcacaaucacaagcggcuggacauuuggagcaggcgccgcucugcagauccccuuugcuaugcagauggccuaccgguucaacggcaucggagugacccagaaugugcuguacgagaaccagaagcugaucgccaaccaguucaacagcgccaucggcaagauccaggacagccugagcagcacagcaagcgcccugggaaagcugcaggacguggucaaccagaaugcccaggcacugaacacccuggucaagcagcuguccuccaacuucggcgccaucagcucugugcugaacgauauccugagcagacuggacccuccugaggccgaggugcagaucgacagacugaucacaggcagacugcagagccuccagacauacgugacccagcagcugaucagagccgccgagauuagagccucugccaaucuggccgccaccaagaugucugagugugugcugggccagagcaagagaguggacuuuugcggcaagggcuaccaccugaugagcuucccucagucugccccucacggcgugguguuucugcacgugacauaugugcccgcucaagagaagaauuucaccaccgcuccagccaucugccacgacggcaaagcccacuuuccuagagaaggcguguucguguccaacggcacccauugguucgugacacagcggaacuucuacgagccccagaucaucaccaccgacaacaccuucgugucuggcaacugcgacgucgugaucggcauugugaacaauaccguguacgacccucugcagcccgagcuggacagcuucaaagaggaacuggacaaguacuuuaagaaccacacaagccccgacguggaccugggcgauaucagcggaaucaaugccagcgucgugaacauccagaaagagaucgaccggcugaacgagguggccaagaaucugaacgagagccugaucgaccugcaagaacuggggaaguacgagcaguacaucaaguggcccugguacaucuggcugggcuuuaucgccggacugauugccaucgugauggucacaaucaugcuguguugcaugaccagcugcuguagcugccugaagggcuguuguagcuguggcagcugcugcaaguucgacgaggacgauucugagcccgugcugaagggcgugaaacugcacuacacaugauga

SEQ ID NO: 59 - RNA, 3825 nt, SARS-CoV-2
auguucguguuccuggugcugcugccccuggugagcucccagugcgugaacuuuacaaacagaacacagcugcccuccgccuacacaaacagcuucaccaggggcguguacuaccccgauaaggucuuucgguccagcgugcugcacagcacccaggaucuguuccugccuuucuucagcaacgugacaugguuucacgccauccacgugagcgggacaaacggcaccaagcgguucgauaacccagugcugcccuuuaacgaugggguguacuucgccagcacagagaaguccaacaucaucaggggcuggauuuucggcaccacccucgauuccaagacacagucccugcugaucgugaacaacgccacaaacguggucauuaaggugugcgaguuccaguuuugcaacuacccauuccugggcguguacuaccacaagaacaacaaguccuggauggagagcgaguucagggucuacuccuccgccaacaacugcaccuucgaguacgugagccagcccuuccugauggaucuggagggcaagcaggggaacuucaagaaccugagcgaguucguguucaagaacauugacggcuacuuuaagaucuacaguaagcacacaccuaucaaccuggugcgggaccugccucagggcuucuccgcccucgagccacugguggaucugccaaucggcauuaacaucaccagguuccagacacugcuggcccugcacaggagcuaccugacuccaggcgauagcuccagcggguggacagccggggccgccgccuacuacgugggcuaccugcagcccagaaccuuucugcugaaguacaacgagaacgggaccaucaccgaugccguggauugcgcccuggacccccugagcgagaccaagugcacucucaaguccuucaccguggagaagggcaucuaccagaccagcaacuuccggguccagcccacagaguccaucgugagguuccccaacaucaccaaccucugccccuucggcgagguguucaacgccaccagguuugccagcguguacgccuggaacaggaagaggaucuccaacugcguggccgauuacagcgugcuguacaacuccgccuccuucagcaccuucaagugcuacggcgugagcccuaccaagcuuaacgaucugugcuuuacaaacguguacgccgauagcuuugugauccggggggacgaggugaggcagauugcccccggccagacagggaccaucgccgauuacaacuacaagcugcccgaugacuucaccgggugcgugauugccuggaacagcaacaaccucgauagcaaggucggggggaacuacaacuaccuguacaggcuguuuagaaaguccaaccucaagccuuucgagcgggauauuagcacugagaucuaccaggccgggagcacacccugcaacggggugaagggcuucaacugcuacuuuccccugcagagcuacggcuuccagccaacauacggcgugggguaccagcccuaccgggugguggugcugagcuucgagcugcugcacgccccugccaccgugugcggccccaagaaaagcacuaaccuggugaagaacaagugcgucaacuucaacuuuaacggccugaccggcacaggggugcugaccgaguccaacaagaaguuccugcccuuccagcaguucggccgggacaucgccgauaccacugacgccgugagggacccccagacccuggagauccuggacauuacacccuguagcuucggcggggucagcgugaucacacccggcaccaacacauccaaccagguggccgugcuguaccagggcgugaacugcaccgaggugcccgucgccauccacgccgaccagcugacacccacauggaggguguacagcacagggagcaacguguuccagaccagggccgggugccugaucggcgccgaguacgugaacaacuccuacgagugcgacauccccaucggggccggcauuugcgccuccuaccagacccagaccaacagcccccggcgggccaggagcguggccagccagagcaucauugccuacacaaugucucugggcgccgagaacagcguggccuacuccaacaacucuaucgcuauccccaccaacuucaccaucagcgugaccacagagauccugccuguguccaugaccaagaccagcguggacugcaccauguacaucugcggcgauuccaccgagugcuccaaccugcugcugcaguacggcagcuucugcacccagcugaauagagcccugacagggaucgccguggaacaggacaagaacacccaagagguguucgcccaagugaagcagaucuacaagaccccuccuaucaaggacuucggcggcuucaauuucagccagauucugcccgauccuagcaagcccagcaagcggagcuucaucgaggaccugcuguucaacaaagugacacuggccgacgccggcuucaucaagcaguauggcgauugucugggcgacauugccgccagggaucugauuugcgcccagaaguuuaacggacugacagugcugccuccucugcugaccgaugagaugaucgcccaguacacaucugcccugcuggccggcacaaucacaagcggcuggacauuuggagcaggcgccgcucugcagauccccuuugcuaugcagauggccuaccgguucaacggcaucggagugacccagaaugugcuguacgagaaccagaagcugaucgccaaccaguucaacagcgccaucggcaagauccaggacagccugagcagcacagcaagcgcccugggaaagcugcaggacguggucaaccagaaugcccaggcacugaacacccuggucaagcagcuguccuccaacuucggcgccaucagcucugugcugaacgauauccugagcagacuggacccuccugaggccgaggugcagaucgacagacugaucacaggcagacugcagagccuccagacauacgugacccagcagcugaucagagccgccgagauuagagccucugccaaucuggccgccaucaagaugucugagugugugcugggccagagcaagagaguggacuuuugcggcaagggcuaccaccugaugagcuucccucagucugccccucacggcgugguguuucugcacgugacauaugugcccgcucaagagaagaauuucaccaccgcuccagccaucugccacgacggcaaagcccacuuuccuagagaaggcguguucguguccaacggcacccauugguucgugacacagcggaacuucuacgagccccagaucaucaccaccgacaacaccuucgugucuggcaacugcgacgucgugaucggcauugugaacaauaccguguacgacccucugcagcccgagcuggacagcuucaaagaggaacuggacaaguacuuuaagaaccacacaagccccgacguggaccugggcgauaucagcggaaucaaugccagcuucgugaacauccagaaagagaucgaccggcugaacgagguggccaagaaucugaacgagagccugaucgaccugcaagaacuggggaaguacgagcaguacaucaaguggcccugguacaucuggcugggcuuuaucgccggacugauugccaucgugauggucacaaucaugcuguguugcaugaccagcugcuguagcugccugaagggcuguuguagcuguggcagcugcugcaaguucgacgaggacgauucugagcccgugcugaagggcgugaaacugcacuacacaugauga

SEQ ID NO: 60 - RNA, 3819 nt, SARS-CoV-2
auguucguguuccuggugcugcugccucugguguccagccagugugugaaccugagaaccagaacacagcugccuccagccuacaccaacagcuuuaccagaggcguguacuaccccgacaagguguucagauccagcgugcugcacucuacccaggaccuguuccugccuuucuucagcaacgugaccugguuccacgccauccacguguccggcaccaauggcaccaagagauucgacaaccccgugcugcccuucaacgacgggguguacuuugccagcaccgagaaguccaacaucaucagaggcuggaucuucggcaccacacuggacagcaagacccagagccugcugaucgugaacaacgccaccaacguggucaucaaagugugcgaguuccaguucugcaacgaccccuuccuggacgucuacuaccacaagaacaacaagagcuggauggaaagcggcguguacagcagcgccaacaacugcaccuucgaguacgugucccagccuuuccugauggaccuggaaggcaagcagggcaacuucaagaaccugcgcgaguucguguuuaagaacaucgacggcuacuucaagaucuacagcaagcacaccccuaucaaccucgugcgggaucugccucagggcuucucugcucuggaaccccugguggaucugcccaucggcaucaacaucacccgguuucagacacugcuggcccugcacagaagcuaccugacaccuggcgauagcagcagcggauggacagcuggugccgccgcuuacuaugugggcuaccugcagccuagaaccuuccugcugaaguacaacgagaacggcaccaucaccgacgccguggauugugcucuggauccucugagcgagacaaagugcacccugaaguccuucaccguggaaaagggcaucuaccagaccagcaacuuccgggugcagcccaccgaauccaucgugcgguuccccaauaucaccaaucugugccccuucggcgagguguucaaugccaccagauucgccucuguguacgccuggaaccggaagcggaucagcaauugcguggccgacuacuccgugcuguacaacuccgccagcuucagcaccuucaagugcuacggcguguccccuaccaagcugaacgaccugugcuucacaaacguguacgccgacagcuucgugauccggggagaugaagugcggcagauugccccuggacagacaggcaagaucgccgacuacaacuacaagcugcccgacgacuucaccggcugugugauugccuggaacagcaacaaccuggacuccaaagucggcggcaacuacaauuaccgguaccggcuguuccggaaguccaaucugaagcccuucgagcgggacaucuccaccgagaucuaucaggccggcagcaagccuuguaacggcguggaaggcuucaacugcuacuucccacugcaguccuacggcuuucagcccacaaauggcgugggcuaucagcccuacagagugguggugcugagcuucgaacugcugcaugccccugccacagugugcggcccuaagaaaagcaccaaucucgugaagaacaaaugcgugaacuucaacuucaacggccugaccggcaccggcgugcugacagagagcaacaagaaguuccugccauuccagcaguuuggccgggauaucgccgauaccacagacgccguuagagauccccagacacuggaaauccuggacaucaccccuugcagcuucggcggagugucugugaucaccccuggcaccaacaccagcaaucagguggcagugcuguaccagggcgugaacuguaccgaagugcccguggccauucacgccgaucagcugacaccuacauggcggguguacuccaccggcagcaauguguuucagaccagagccggcugucugaucggagccgagcacgugaacaauagcuacgagugcgacauccccaucggcgcuggaaucugcgccagcuaccagacacagacaaacagccggcggagagccagaagcguggccagccagagcaucauugccuacacaaugucucugggcgccgagaacagcguggccuacuccaacaacucuaucgcuauccccaccaacuucaccaucagcgugaccacagagauccugccuguguccaugaccaagaccagcguggacugcaccauguacaucugcggcgauuccaccgagugcuccaaccugcugcugcaguacggcagcuucugcacccagcugaauagagcccugacagggaucgccguggaacaggacaagaacacccaagagguguucgcccaagugaagcagaucuacaagaccccuccuaucaaggacuucggcggcuucaauuucagccagauucugcccgauccuagcaagcccagcaagcggagcuucaucgaggaccugcuguucaacaaagugacacuggccgacgccggcuucaucaagcaguauggcgauugucugggcgacauugccgccagggaucugauuugcgcccagaaguuuaacggacugacagugcugccuccucugcugaccgaugagaugaucgcccaguacacaucugcccugcuggccggcacaaucacaagcggcuggacauuuggagcaggcgccgcucugcagauccccuuugcuaugcagauggccuaccgguucaacggcaucggagugacccagaaugugcuguacgagaaccagaagcugaucgccaaccaguucaacagcgccaucggcaagauccaggacagccugagcagcacagcaagcgcccugggaaagcugcagaacguggucaaccagaaugcccaggcacugaacacccuggucaagcagcuguccuccaacuucggcgccaucagcucugugcugaacgauauccugagcagacuggacccuccugaggccgaggugcagaucgacagacugaucacaggcagacugcagagccuccagacauacgugacccagcagcugaucagagccgccgagauuagagccucugccaaucuggccgccaccaagaugucugagugugugcugggccagagcaagagaguggacuuuugcggcaagggcuaccaccugaugagcuucccucagucugccccucacggcgugguguuucugcacgugacauaugugcccgcucaagagaagaauuucaccaccgcuccagccaucugccacgacggcaaagcccacuuuccuagagaaggcguguucguguccaacggcacccauugguucgugacacagcggaacuucuacgagccccagaucaucaccaccgacaacaccuucgugucuggcaacugcgacgucgugaucggcauugugaacaauaccguguacgacccucugcagcccgagcuggacagcuucaaagaggaacuggacaaguacuuuaagaaccacacaagccccgacguggaccugggcgauaucagcggaaucaaugccagcgucgugaacauccagaaagagaucgaccggcugaacgagguggccaagaaucugaacgagagccugaucgaccugcaagaacuggggaaguacgagcaguacaucaaguggcccugguacaucuggcugggcuuuaucgccggacugauugccaucgugauggucacaaucaugcuguguugcaugaccagcugcuguagcugccugaagggcuguuguagcuguggcagcugcugcaaguucgacgaggacgauucugagcccgugcugaagggcgugaaacugcacuacacaugauga

SEQ ID NO: 61 - RNA, 3825 nt, SARS-CoV-2
auguucguguuccuggugcugcugccucugguguccauccagugugugaaccugaccaccagaacacagcugccuccagccuacaccaacagcuuuaccagaggcguguacuaccccgacaagguguucagauccagcgugcugcacucuacccaggaccuguuccugccuuucuucagcaacgugaccugguuccacgccauccacguguccggcaccaauggcaccaagagauucgacaaccccgugcugcccuucaacgacgggguguacuuugccagcaccgagaaguccaacaucaucagaggcuggaucuucggcaccacacuggacagcaagacccagagccugcugaucgugaacaacgccaccaacguggucaucaaagugugcgaguuccaguucugcaacgaccccuuccugggcgucuacuaccacaagaacaacaagagcugcauggaaagcgaguuccggguguacagcagcgccaacaacugcaccuucgaguacgugucccagccuuuccugauggaccuggaaggcaagcagggcaacuucaagaaccugcgcgaguucguguuuaagaacaucgacggcuacuucaagaucuacagcaagcacaccccuaucaaccucgugcgggaucugccucagggcuucucugcucuggaaccccugguggaucugcccaucggcaucaacaucacccgguuucagacacugcuggcccugcacagaagcuaccugacaccuggcgauagcagcagcggauggacagcuggugccgccgcuuacuaugugggcuaccugcagccuagaaccuuccugcugaaguacaacgagaacggcaccaucaccgacgccguggauugugcucuggauccucugagcgagacaaagugcacccugaaguccuucaccguggaaaagggcaucuaccagaccagcaacuuccgggugcagcccaccgaauccaucgugcgguuccccaauaucaccaaucugugccccuucggcgagguguucaaugccaccagauucgccucuguguacgccuggaaccggaagcggaucagcaauugcguggccgacuacuccgugcuguacaacuccgccagcuucagcaccuucaagugcuacggcguguccccuaccaagcugaacgaccugugcuucacaaacguguacgccgacagcuucgugauccggggagaugaagugcggcagauugccccuggacagacaggcaagaucgccgacuacaacuacaagcugcccgacgacuucaccggcugugugauugccuggaacagcaacaaccuggacuccaaagucggcggcaacuacaauuaccgcuaccggcuguuccggaaguccaaucugaagcccuucgagcgggacaucuccaccgagaucuaucaggccggcagcaccccuuguaacggcguggaaggcuucaacugcuacuucccacugcaguccuacggcuuucagcccacaaauggcgugggcuaucagcccuacagagugguggugcugagcuucgaacugcugcaugccccugccacagugugcggcccuaagaaaagcaccaaucucgugaagaacaaaugcgugaacuucaacuucaacggccugaccggcaccggcgugcugacagagagcaacaagaaguuccugccauuccagcaguuuggccgggauaucgccgauaccacagacgccguuagagauccccagacacuggaaauccuggacaucaccccuugcagcuucggcggagugucugugaucaccccuggcaccaacaccagcaaucagguggcagugcuguaccagggcgugaacuguaccgaagugcccguggccauucacgccgaucagcugacaccuacauggcggguguacuccaccggcagcaauguguuucagaccagagccggcugucugaucggagccgagcacgugaacaauagcuacgagugcgacauccccaucggcgcuggaaucugcgccagcuaccagacacagacaaacagcccucggagagccagaagcguggccagccagagcaucauugccuacacaaugucucugggcgccgagaacagcguggccuacuccaacaacucuaucgcuauccccaccaacuucaccaucagcgugaccacagagauccugccuguguccaugaccaagaccagcguggacugcaccauguacaucugcggcgauuccaccgagugcuccaaccugcugcugcaguacggcagcuucugcacccagcugaauagagcccugacagggaucgccguggaacaggacaagaacacccaagagguguucgcccaagugaagcagaucuacaagaccccuccuaucaaggacuucggcggcuucaauuucagccagauucugcccgauccuagcaagcccagcaagcggagcuucaucgaggaccugcuguucaacaaagugacacuggccgacgccggcuucaucaagcaguauggcgauugucugggcgacauugccgccagggaucugauuugcgcccagaaguuuaacggacugacagugcugccuccucugcugaccgaugagaugaucgcccaguacacaucugcccugcuggccggcacaaucacaagcggcuggacauuuggagcaggcgccgcucugcagauccccuuugcuaugcagauggccuaccgguucaacggcaucggagugacccagaaugugcuguacgagaaccagaagcugaucgccaaccaguucaacagcgccaucggcaagauccaggacagccugagcagcacagcaagcgcccugggaaagcugcaggacguggucaaccagaaugcccaggcacugaacacccuggucaagcagcuguccuccaacuucggcgccaucagcucugugcugaacgauauccugagcagacuggacccuccugaggccgaggugcagaucgacagacugaucacaggcagacugcagagccuccagacauacgugacccagcagcugaucagagccgccgagauuagagccucugccaaucuggccgccaccaagaugucugagugugugcugggccagagcaagagaguggacuuuugcggcaagggcuaccaccugaugagcuucccucagucugccccucacggcgugguguuucugcacgugacauaugugcccgcucaagagaagaauuucaccaccgcuccagccaucugccacgacggcaaagcccacuuuccuagagaaggcguguucguguccaacggcacccauugguucgugacacagcggaacuucuacgagccccagaucaucaccaccgacaacaccuucgugucuggcaacugcgacgucgugaucggcauugugaacaauaccguguacgacccucugcagcccgagcuggacagcuucaaagaggaacuggacaaguacuuuaagaaccacacaagccccgacguggaccugggcgauaucagcggaaucaaugccagcgucgugaacauccagaaagagaucgaccggcugaacgagguggccaagaaucugaacgagagccugaucgaccugcaagaacuggggaaguacgagcaguacaucaaguggcccugguacaucuggcugggcuuuaucgccggacugauugccaucgugauggucacaaucaugcuguguugcaugaccagcugcuguagcugccugaagggcuguuguagcuguggcagcugcugcaaguucgacgaggacgauucugagcccgugcugaagggcgugaaacugcacuacacaugauga

SEQ ID NO: 62 - RNA, 3816 nt, SARS-CoV-2
auguucguguuccuggugcugcugccucugguguccagccagugugugaaccugaccaccagaacacagcugccuccagccuacaccaacagcuuuaccagaggcguguacuaccccgacaagguguucagauccagcgugcugcacucuacccaggaccuguuccugccuuucuucagcaacgugaccugguuccacgugaucuccggcaccaauggcaccaagagauucgacaaccccgugcugcccuucaacgacgggguguacuuugccagcaucgagaaguccaacaucaucagaggcuggaucuucggcaccacacuggacagcaagacccagagccugcugaucgugaacaacgccaccaacguggucaucaaagugugcgaguuccaguucugcaacgaccccuuccuggaccacaagaacaacaagagcuggauggaaagcgaguuccggguguacagcagcgccaacaacugcaccuucgaguacgugucccagccuuuccugauggaccuggaaggcaagcagggcaacuucaagaaccugcgcgaguucguguuuaagaacaucgacggcuacuucaagaucuacagcaagcacaccccuaucaucgugcgggaaccugaagaucugccucagggcuucucugcucuggaaccccugguggaucugcccaucggcaucaacaucacccgguuucagacacugcuggcccugcacagaagcuaccugacaccuggcgauagcagcagcggauggacagcuggugccgccgcuuacuaugugggcuaccugcagccuagaaccuuccugcugaaguacaacgagaacggcaccaucaccgacgccguggauugugcucuggauccucugagcgagacaaagugcacccugaaguccuucaccguggaaaagggcaucuaccagaccagcaacuuccgggugcagcccaccgaauccaucgugcgguuccccaauaucaccaaucugugccccuucgacgagguguucaaugccaccagauucgccucuguguacgccuggaaccggaagcggaucagcaauugcguggccgacuacuccgugcuguacaaccuggcccccuucuucaccuucaagugcuacggcguguccccuaccaagcugaacgaccugugcuucacaaacguguacgccgacagcuucgugauccggggagaugaagugcggcagauugccccuggacagacaggcaacaucgccgacuacaacuacaagcugcccgacgacuucaccggcugugugauugccuggaacagcaacaagcuggacuccaaagucuccggcaacuacaauuaccuguaccggcuguuccggaaguccaaucugaagcccuucgagcgggacaucuccaccgagaucuaucaggccggcaacaagccuuguaacggcguggccggcuucaacugcuacuucccacugcgguccuacuccuuucggcccacauauggcgugggccaucagcccuacagagugguggugcugagcuucgaacugcugcaugccccugccacagugugcggcccuaagaaaagcaccaaucucgugaagaacaaaugcgugaacuucaacuucaacggccugaagggcaccggcgugcugacagagagcaacaagaaguuccugccauuccagcaguuuggccgggauaucgccgauaccacagacgccguuagagauccccagacacuggaaauccuggacaucaccccuugcagcuucggcggagugucugugaucaccccuggcaccaacaccagcaaucagguggcagugcuguaccagggcgugaacuguaccgaagugcccguggccauucacgccgaucagcugacaccuacauggcggguguacuccaccggcagcaauguguuucagaccagagccggcugucugaucggagccgaguacgugaacaauagcuacgagugcgacauccccaucggcgcuggaaucugcgccagcuaccagacacagacaaagagccaucggagagccagaagcguggccagccagagcaucauugccuacacaaugucucugggcgccgagaacagcguggccuacuccaacaacucuaucgcuauccccaccaacuucaccaucagcgugaccacagagauccugccuguguccaugaccaagaccagcguggacugcaccauguacaucugcggcgauuccaccgagugcuccaaccugcugcugcaguacggcagcuucugcacccagcugaagagagcccugacagggaucgccguggaacaggacaagaacacccaagagguguucgcccaagugaagcagaucuacaagaccccuccuaucaaguacuucggcggcuucaauuucagccagauucugcccgauccuagcaagcccagcaagcggagcuucaucgaggaccugcuguucaacaaagugacacuggccgacgccggcuucaucaagcaguauggcgauugucugggcgacauugccgccagggaucugauuugcgcccagaaguuuaagggacugacagugcugccuccucugcugaccgaugagaugaucgcccaguacacaucugcccugcuggccggcacaaucacaagcggcuggacauuuggagcaggcgccgcucugcagauccccuuugcuaugcagauggccuaccgguucaacggcaucggagugacccagaaugugcuguacgagaaccagaagcugaucgccaaccaguucaacagcgccaucggcaagauccaggacagccugagcagcacagcaagcgcccugggaaagcugcaggacguggucaaccacaaugcccaggcacugaacacccuggucaagcagcuguccuccaaguucggcgccaucagcucugugcugaacgauaucuucagcagacuggacccuccugaggccgaggugcagaucgacagacugaucacaggcagacugcagagccuccagacauacgugacccagcagcugaucagagccgccgagauuagagccucugccaaucuggccgccaccaagaugucugagugugugcugggccagagcaagagaguggacuuuugcggcaagggcuaccaccugaugagcuucccucagucugccccucacggcgugguguuucugcacgugacauaugugcccgcucaagagaagaauuucaccaccgcuccagccaucugccacgacggcaaagcccacuuuccuagagaaggcguguucguguccaacggcacccauugguucgugacacagcggaacuucuacgagccccagaucaucaccaccgacaacaccuucgugucuggcaacugcgacgucgugaucggcauugugaacaauaccguguacgacccucugcagcccgagcuggacagcuucaaagaggaacuggacaaguacuuuaagaaccacacaagccccgacguggaccugggcgauaucagcggaaucaaugccagcgucgugaacauccagaaagagaucgaccggcugaacgagguggccaagaaucugaacgagagccugaucgaccugcaagaacuggggaaguacgagcaguacaucaaguggcccugguacaucuggcugggcuuuaucgccggacugauugccaucgugauggucacaaucaugcuguguugcaugaccagcugcuguagcugccugaagggcuguuguagcuguggcagcugcugcaaguucgacgaggacgauucugagcccgugcugaagggcgugaaacugcacuacacaugauga

SEQ ID NO: 63 - RNA, 4157 nt, Artificial
  wild type S protein mRNA containing 5'-UTR, 3'-UTR and polyA
gaguccuccccauccucucccucugucccucugucccucugacccugcacugucccagcaccauguucguguuccuggugcugcugccucugguguccagccagugugugaaccugaccaccagaacacagcugccuccagccuacaccaacagcuuuaccagaggcguguacuaccccgacaagguguucagauccagcgugcugcacucuacccaggaccuguuccugccuuucuucagcaacgugaccugguuccacgccauccacguguccggcaccaauggcaccaagagauucgacaaccccgugcugcccuucaacgacgggguguacuuugccagcaccgagaaguccaacaucaucagaggcuggaucuucggcaccacacuggacagcaagacccagagccugcugaucgugaacaacgccaccaacguggucaucaaagugugcgaguuccaguucugcaacgaccccuuccugggcgucuacuaccacaagaacaacaagagcuggauggaaagcgaguuccggguguacagcagcgccaacaacugcaccuucgaguacgugucccagccuuuccugauggaccuggaaggcaagcagggcaacuucaagaaccugcgcgaguucguguuuaagaacaucgacggcuacuucaagaucuacagcaagcacaccccuaucaaccucgugcgggaucugccucagggcuucucugcucuggaaccccugguggaucugcccaucggcaucaacaucacccgguuucagacacugcuggcccugcacagaagcuaccugacaccuggcgauagcagcagcggauggacagcuggugccgccgcuuacuaugugggcuaccugcagccuagaaccuuccugcugaaguacaacgagaacggcaccaucaccgacgccguggauugugcucuggauccucugagcgagacaaagugcacccugaaguccuucaccguggaaaagggcaucuaccagaccagcaacuuccgggugcagcccaccgaauccaucgugcgguuccccaauaucaccaaucugugccccuucggcgagguguucaaugccaccagauucgccucuguguacgccuggaaccggaagcggaucagcaauugcguggccgacuacuccgugcuguacaacuccgccagcuucagcaccuucaagugcuacggcguguccccuaccaagcugaacgaccugugcuucacaaacguguacgccgacagcuucgugauccggggagaugaagugcggcagauugccccuggacagacaggcaagaucgccgacuacaacuacaagcugcccgacgacuucaccggcugugugauugccuggaacagcaacaaccuggacuccaaagucggcggcaacuacaauuaccuguaccggcuguuccggaaguccaaucugaagcccuucgagcgggacaucuccaccgagaucuaucaggccggcagcaccccuuguaacggcguggaaggcuucaacugcuacuucccacugcaguccuacggcuuucagcccacaaauggcgugggcuaucagcccuacagagugguggugcugagcuucgaacugcugcaugccccugccacagugugcggcccuaagaaaagcaccaaucucgugaagaacaaaugcgugaacuucaacuucaacggccugaccggcaccggcgugcugacagagagcaacaagaaguuccugccauuccagcaguuuggccgggauaucgccgauaccacagacgccguuagagauccccagacacuggaaauccuggacaucaccccuugcagcuucggcggagugucugugaucaccccuggcaccaacaccagcaaucagguggcagugcuguaccaggacgugaacuguaccgaagugcccguggccauucacgccgaucagcugacaccuacauggcggguguacuccaccggcagcaauguguuucagaccagagccggcugucugaucggagccgagcacgugaacaauagcuacgagugcgacauccccaucggcgcuggaaucugcgccagcuaccagacacagacaaacagcccucggagagccagaagcguggccagccagagcaucauugccuacacaaugucucugggcgccgagaacagcguggccuacuccaacaacucuaucgcuauccccaccaacuucaccaucagcgugaccacagagauccugccuguguccaugaccaagaccagcguggacugcaccauguacaucugcggcgauuccaccgagugcuccaaccugcugcugcaguacggcagcuucugcacccagcugaauagagcccugacagggaucgccguggaacaggacaagaacacccaagagguguucgcccaagugaagcagaucuacaagaccccuccuaucaaggacuucggcggcuucaauuucagccagauucugcccgauccuagcaagcccagcaagcggagcuucaucgaggaccugcuguucaacaaagugacacuggccgacgccggcuucaucaagcaguauggcgauugucugggcgacauugccgccagggaucugauuugcgcccagaaguuuaacggacugacagugcugccuccucugcugaccgaugagaugaucgcccaguacacaucugcccugcuggccggcacaaucacaagcggcuggacauuuggagcaggcgccgcucugcagauccccuuugcuaugcagauggccuaccgguucaacggcaucggagugacccagaaugugcuguacgagaaccagaagcugaucgccaaccaguucaacagcgccaucggcaagauccaggacagccugagcagcacagcaagcgcccugggaaagcugcaggacguggucaaccagaaugcccaggcacugaacacccuggucaagcagcuguccuccaacuucggcgccaucagcucugugcugaacgauauccugagcagacuggacccuccugaggccgaggugcagaucgacagacugaucacaggcagacugcagagccuccagacauacgugacccagcagcugaucagagccgccgagauuagagccucugccaaucuggccgccaccaagaugucugagugugugcugggccagagcaagagaguggacuuuugcggcaagggcuaccaccugaugagcuucccucagucugccccucacggcgugguguuucugcacgugacauaugugcccgcucaagagaagaauuucaccaccgcuccagccaucugccacgacggcaaagcccacuuuccuagagaaggcguguucguguccaacggcacccauugguucgugacacagcggaacuucuacgagccccagaucaucaccaccgacaacaccuucgugucuggcaacugcgacgucgugaucggcauugugaacaauaccguguacgacccucugcagcccgagcuggacagcuucaaagaggaacuggacaaguacuuuaagaaccacacaagccccgacguggaccugggcgauaucagcggaaucaaugccagcgucgugaacauccagaaagagaucgaccggcugaacgagguggccaagaaucugaacgagagccugaucgaccugcaagaacuggggaaguacgagcaguacaucaaguggcccugguacaucuggcugggcuuuaucgccggacugauugccaucgugauggucacaaucaugcuguguugcaugaccagcugcuguagcugccugaagggcuguuguagcuguggcagcugcugcaaguucgacgaggacgauucugagcccgugcugaagggcgugaaacugcacuacacaugaugacucgagguguguggaggacacccugaaccccccgcuuucaaacaaguuuucaaauuguuugaggucaggauuucucaaacugauuccuuucuuugcauaugaguauuugaaaauaaauauuuucccagaauauaaauaaaucaucacaugauuauuuuaacuaugcuagcaaaaaaaaaaaaaaaaaaaaaaaaaaaaaaaaaaaaaaaaaaaaaaaaaaaaaaaaaaaaaaaaaaaaaaaaaaaaaaaaaaaaaaaaaaaaaaaaaaaa

SEQ ID NO: 64 - RNA, 4148 nt, Artificial
  Alpha variant S protein mRNA containing 5'-UTR, 3'-UTR and polyA
gaguccuccccauccucucccucugucccucugucccucugacccugcacugucccagcaccauguucguguuccuggugcugcugccucugguguccagccagugugugaaccugaccaccagaacacagcugccuccagccuacaccaacagcuuuaccagaggcguguacuaccccgacaagguguucagauccagcgugcugcacucuacccaggaccuguuccugccuuucuucagcaacgugaccugguuccacgccaucuccggcaccaauggcaccaagagauucgacaaccccgugcugcccuucaacgacgggguguacuuugccagcaccgagaaguccaacaucaucagaggcuggaucuucggcaccacacuggacagcaagacccagagccugcugaucgugaacaacgccaccaacguggucaucaaagugugcgaguuccaguucugcaacgaccccuuccugggcgucuaccacaagaacaacaagagcuggauggaaagcgaguuccggguguacagcagcgccaacaacugcaccuucgaguacgugucccagccuuuccugauggaccuggaaggcaagcagggcaacuucaagaaccugcgcgaguucguguuuaagaacaucgacggcuacuucaagaucuacagcaagcacaccccuaucaaccucgugcgggaucugccucagggcuucucugcucuggaaccccugguggaucugcccaucggcaucaacaucacccgguuucagacacugcuggcccugcacagaagcuaccugacaccuggcgauagcagcagcggauggacagcuggugccgccgcuuacuaugugggcuaccugcagccuagaaccuuccugcugaaguacaacgagaacggcaccaucaccgacgccguggauugugcucuggauccucugagcgagacaaagugcacccugaaguccuucaccguggaaaagggcaucuaccagaccagcaacuuccgggugcagcccaccgaauccaucgugcgguuccccaauaucaccaaucugugccccuucggcgagguguucaaugccaccagauucgccucuguguacgccuggaaccggaagcggaucagcaauugcguggccgacuacuccgugcuguacaacuccgccagcuucagcaccuucaagugcuacggcguguccccuaccaagcugaacgaccugugcuucacaaacguguacgccgacagcuucgugauccggggagaugaagugcggcagauugccccuggacagacaggcaagaucgccgacuacaacuacaagcugcccgacgacuucaccggcugugugauugccuggaacagcaacaaccuggacuccaaagucggcggcaacuacaauuaccuguaccggcuguuccggaaguccaaucugaagcccuucgagcgggacaucuccaccgagaucuaucaggccggcagcaccccuuguaacggcguggaaggcuucaacugcuacuucccacugcaguccuacggcuuucagcccacauacggcgugggcuaucagcccuacagagugguggugcugagcuucgaacugcugcaugccccugccacagugugcggcccuaagaaaagcaccaaucucgugaagaacaaaugcgugaacuucaacuucaacggccugaccggcaccggcgugcugacagagagcaacaagaaguuccugccauuccagcaguuuggccgggauaucgacgauaccacagacgccguuagagauccccagacacuggaaauccuggacaucaccccuugcagcuucggcggagugucugugaucaccccuggcaccaacaccagcaaucagguggcagugcuguaccagggcgugaacuguaccgaagugcccguggccauucacgccgaucagcugacaccuacauggcggguguacuccaccggcagcaauguguuucagaccagagccggcugucugaucggagccgagcacgugaacaauagcuacgagugcgacauccccaucggcgcuggaaucugcgccagcuaccagacacagacaaacagccaccggagagccagaagcguggccagccagagcaucauugccuacacaaugucucugggcgccgagaacagcguggccuacuccaacaacucuaucgcuauccccaucaacuucaccaucagcgugaccacagagauccugccuguguccaugaccaagaccagcguggacugcaccauguacaucugcggcgauuccaccgagugcuccaaccugcugcugcaguacggcagcuucugcacccagcugaauagagcccugacagggaucgccguggaacaggacaagaacacccaagagguguucgcccaagugaagcagaucuacaagaccccuccuaucaaggacuucggcggcuucaauuucagccagauucugcccgauccuagcaagcccagcaagcggagcuucaucgaggaccugcuguucaacaaagugacacuggccgacgccggcuucaucaagcaguauggcgauugucugggcgacauugccgccagggaucugauuugcgcccagaaguuuaacggacugacagugcugccuccucugcugaccgaugagaugaucgcccaguacacaucugcccugcuggccggcacaaucacaagcggcuggacauuuggagcaggcgccgcucugcagauccccuuugcuaugcagauggccuaccgguucaacggcaucggagugacccagaaugugcuguacgagaaccagaagcugaucgccaaccaguucaacagcgccaucggcaagauccaggacagccugagcagcacagcaagcgcccugggaaagcugcaggacguggucaaccagaaugcccaggcacugaacacccuggucaagcagcuguccuccaacuucggcgccaucagcucugugcugaacgauauccuggcaagacuggacccuccugaggccgaggugcagaucgacagacugaucacaggcagacugcagagccuccagacauacgugacccagcagcugaucagagccgccgagauuagagccucugccaaucuggccgccaccaagaugucugagugugugcugggccagagcaagagaguggacuuuugcggcaagggcuaccaccugaugagcuucccucagucugccccucacggcgugguguuucugcacgugacauaugugcccgcucaagagaagaauuucaccaccgcuccagccaucugccacgacggcaaagcccacuuuccuagagaaggcguguucguguccaacggcacccauugguucgugacacagcggaacuucuacgagccccagaucaucaccacccacaacaccuucgugucuggcaacugcgacgucgugaucggcauugugaacaauaccguguacgacccucugcagcccgagcuggacagcuucaaagaggaacuggacaaguacuuuaagaaccacacaagccccgacguggaccugggcgauaucagcggaaucaaugccagcgucgugaacauccagaaagagaucgaccggcugaacgagguggccaagaaucugaacgagagccugaucgaccugcaagaacuggggaaguacgagcaguacaucaaguggcccugguacaucuggcugggcuuuaucgccggacugauugccaucgugauggucacaaucaugcuguguugcaugaccagcugcuguagcugccugaagggcuguuguagcuguggcagcugcugcaaguucgacgaggacgauucugagcccgugcugaagggcgugaaacugcacuacacaugaugacucgagguguguggaggacacccugaaccccccgcuuucaaacaaguuuucaaauuguuugaggucaggauuucucaaacugauuccuuucuuugcauaugaguauuugaaaauaaauauuuucccagaauauaaauaaaucaucacaugauuauuuuaacuaugcuagcaaaaaaaaaaaaaaaaaaaaaaaaaaaaaaaaaaaaaaaaaaaaaaaaaaaaaaaaaaaaaaaaaaaaaaaaaaaaaaaaaaaaaaaaaaaaaaaaaaaa

SEQ ID NO: 65 - RNA, 4148 nt, Artificial
  Beta variant S protein mRNA containing 5'-UTR, 3'-UTR and polyA
gaguccuccccauccucucccucugucccucugucccucugacccugcacugucccagcaccauguucguguuccuggugcugcugccucugguguccagccagugugugaacuucaccaccagaacacagcugccuccagccuacaccaacagcuuuaccagaggcguguacuaccccgacaagguguucagauccagcgugcugcacucuacccaggaccuguuccugccuuucuucagcaacgugaccugguuccacgccauccacguguccggcaccaauggcaccaagagauucgccaaccccgugcugcccuucaacgacgggguguacuuugccagcaccgagaaguccaacaucaucagaggcuggaucuucggcaccacacuggacagcaagacccagagccugcugaucgugaacaacgccaccaacguggucaucaaagugugcgaguuccaguucugcaacgaccccuuccugggcgucuacuaccacaagaacaacaagagcuggauggaaagcgaguuccggguguacagcagcgccaacaacugcaccuucgaguacgugucccagccuuuccugauggaccuggaaggcaagcagggcaacuucaagaaccugcgcgaguucguguuuaagaacaucgacggcuacuucaagaucuacagcaagcacaccccuaucaaccucgugcggggucugccucagggcuucucugcucuggaaccccugguggaucugcccaucggcaucaacaucacccgguuucagacacugcacagaagcuaccugacaccuggcgauagcagcagcggauggacagcuggugccgccgcuuacuaugugggcuaccugcagccuagaaccuuccugcugaaguacaacgagaacggcaccaucaccgacgccguggauugugcucuggauccucugagcgagacaaagugcacccugaaguccuucaccguggaaaagggcaucuaccagaccagcaacuuccgggugcagcccaccgaauccaucgugcgguuccccaauaucaccaaucugugccccuucggcgagguguucaaugccaccagauucgccucuguguacgccuggaaccggaagcggaucagcaauugcguggccgacuacuccgugcuguacaacuccgccagcuucagcaccuucaagugcuacggcguguccccuaccaagcugaacgaccugugcuucacaaacguguacgccgacagcuucgugauccggggagaugaagugcggcagauugccccuggacagacaggcaauaucgccgacuacaacuacaagcugcccgacgacuucaccggcugugugauugccuggaacagcaacaaccuggacuccaaagucggcggcaacuacaauuaccuguaccggcuguuccggaaguccaaucugaagcccuucgagcgggacaucuccaccgagaucuaucaggccggcagcaccccuuguaacggcgugaaaggcuucaacugcuacuucccacugcaguccuacggcuuucagcccacauacggcgugggcuaucagcccuacagagugguggugcugagcuucgaacugcugcaugccccugccacagugugcggcccuaagaaaagcaccaaucucgugaagaacaaaugcgugaacuucaacuucaacggccugaccggcaccggcgugcugacagagagcaacaagaaguuccugccauuccagcaguuuggccgggauaucgccgauaccacagacgccguuagagauccccagacacuggaaauccuggacaucaccccuugcagcuucggcggagugucugugaucaccccuggcaccaacaccagcaaucagguggcagugcuguaccagggcgugaacuguaccgaagugcccguggccauucacgccgaucagcugacaccuacauggcggguguacuccaccggcagcaauguguuucagaccagagccggcugucugaucggagccgagcacgugaacaauagcuacgagugcgacauccccaucggcgcuggaaucugcgccagcuaccagacacagacaaacagcccucggagagccagaagcguggccagccagagcaucauugccuacacaaugucucugggcguggagaacagcguggccuacuccaacaacucuaucgcuauccccaccaacuucaccaucagcgugaccacagagauccugccuguguccaugaccaagaccagcguggacugcaccauguacaucugcggcgauuccaccgagugcuccaaccugcugcugcaguacggcagcuucugcacccagcugaauagagcccugacagggaucgccguggaacaggacaagaacacccaagagguguucgcccaagugaagcagaucuacaagaccccuccuaucaaggacuucggcggcuucaauuucagccagauucugcccgauccuagcaagcccagcaagcggagcuucaucgaggaccugcuguucaacaaagugacacuggccgacgccggcuucaucaagcaguauggcgauugucugggcgacauugccgccagggaucugauuugcgcccagaaguuuaacggacugacagugcugccuccucugcugaccgaugagaugaucgcccaguacacaucugcccugcuggccggcacaaucacaagcggcuggacauuuggagcaggcgccgcucugcagauccccuuugcuaugcagauggccuaccgguucaacggcaucggagugacccagaaugugcuguacgagaaccagaagcugaucgccaaccaguucaacagcgccaucggcaagauccaggacagccugagcagcacagcaagcgcccugggaaagcugcaggacguggucaaccagaaugcccaggcacugaacacccuggucaagcagcuguccuccaacuucggcgccaucagcucugugcugaacgauauccugagcagacuggacccuccugaggccgaggugcagaucgacagacugaucacaggcagacugcagagccuccagacauacgugacccagcagcugaucagagccgccgagauuagagccucugccaaucuggccgccaccaagaugucugagugugugcugggccagagcaagagaguggacuuuugcggcaagggcuaccaccugaugagcuucccucagucugccccucacggcgugguguuucugcacgugacauaugugcccgcucaagagaagaauuucaccaccgcuccagccaucugccacgacggcaaagcccacuuuccuagagaaggcguguucguguccaacggcacccauugguucgugacacagcggaacuucuacgagccccagaucaucaccaccgacaacaccuucgugucuggcaacugcgacgucgugaucggcauugugaacaauaccguguacgacccucugcagcccgagcuggacagcuucaaagaggaacuggacaaguacuuuaagaaccacacaagccccgacguggaccugggcgauaucagcggaaucaaugccagcgucgugaacauccagaaagagaucgaccggcugaacgagguggccaagaaucugaacgagagccugaucgaccugcaagaacuggggaaguacgagcaguacaucaaguggcccugguacaucuggcugggcuuuaucgccggacugauugccaucgugauggucacaaucaugcuguguugcaugaccagcugcuguagcugccugaagggcuguuguagcuguggcagcugcugcaaguucgacgaggacgauucugagcccgugcugaagggcgugaaacugcacuacacaugaugacucgagguguguggaggacacccugaaccccccgcuuucaaacaaguuuucaaauuguuugaggucaggauuucucaaacugauuccuuucuuugcauaugaguauuugaaaauaaauauuuucccagaauauaaauaaaucaucacaugauuauuuuaacuaugcuagcaaaaaaaaaaaaaaaaaaaaaaaaaaaaaaaaaaaaaaaaaaaaaaaaaaaaaaaaaaaaaaaaaaaaaaaaaaaaaaaaaaaaaaaaaaaaaaaaaaaa

SEQ ID NO: 66 - RNA, 4157 nt, Artificial
  delta variant S protein mRNA containing 5'-UTR, 3'-UTR and polyA
gaguccuccccauccucucccucugucccucugucccucugacccugcacugucccagcaccauguucguguuccuggugcugcugccccuggugagcucccagugcgugaacuuuacaaacagaacacagcugcccuccgccuacacaaacagcuucaccaggggcguguacuaccccgauaaggucuuucgguccagcgugcugcacagcacccaggaucuguuccugccuuucuucagcaacgugacaugguuucacgccauccacgugagcgggacaaacggcaccaagcgguucgauaacccagugcugcccuuuaacgaugggguguacuucgccagcacagagaaguccaacaucaucaggggcuggauuuucggcaccacccucgauuccaagacacagucccugcugaucgugaacaacgccacaaacguggucauuaaggugugcgaguuccaguuuugcaacuacccauuccugggcguguacuaccacaagaacaacaaguccuggauggagagcgaguucagggucuacuccuccgccaacaacugcaccuucgaguacgugagccagcccuuccugauggaucuggagggcaagcaggggaacuucaagaaccugagcgaguucguguucaagaacauugacggcuacuuuaagaucuacaguaagcacacaccuaucaaccuggugcgggaccugccucagggcuucuccgcccucgagccacugguggaucugccaaucggcauuaacaucaccagguuccagacacugcuggcccugcacaggagcuaccugacuccaggcgauagcuccagcggguggacagccggggccgccgccuacuacgugggcuaccugcagcccagaaccuuucugcugaaguacaacgagaacgggaccaucaccgaugccguggauugcgcccuggacccccugagcgagaccaagugcacucucaaguccuucaccguggagaagggcaucuaccagaccagcaacuuccggguccagcccacagaguccaucgugagguuccccaacaucaccaaccucugccccuucggcgagguguucaacgccaccagguuugccagcguguacgccuggaacaggaagaggaucuccaacugcguggccgauuacagcgugcuguacaacuccgccuccuucagcaccuucaagugcuacggcgugagcccuaccaagcuuaacgaucugugcuuuacaaacguguacgccgauagcuuugugauccggggggacgaggugaggcagauugcccccggccagacagggaccaucgccgauuacaacuacaagcugcccgaugacuucaccgggugcgugauugccuggaacagcaacaaccucgauagcaaggucggggggaacuacaacuaccuguacaggcuguuuagaaaguccaaccucaagccuuucgagcgggauauuagcacugagaucuaccaggccgggagcacacccugcaacggggugaagggcuucaacugcuacuuuccccugcagagcuacggcuuccagccaacauacggcgugggguaccagcccuaccgggugguggugcugagcuucgagcugcugcacgccccugccaccgugugcggccccaagaaaagcacuaaccuggugaagaacaagugcgucaacuucaacuuuaacggccugaccggcacaggggugcugaccgaguccaacaagaaguuccugcccuuccagcaguucggccgggacaucgccgauaccacugacgccgugagggacccccagacccuggagauccuggacauuacacccuguagcuucggcggggucagcgugaucacacccggcaccaacacauccaaccagguggccgugcuguaccagggcgugaacugcaccgaggugcccgucgccauccacgccgaccagcugacacccacauggaggguguacagcacagggagcaacguguuccagaccagggccgggugccugaucggcgccgaguacgugaacaacuccuacgagugcgacauccccaucggggccggcauuugcgccuccuaccagacccagaccaacagcccccggcgggccaggagcguggccagccagagcaucauugccuacacaaugucucugggcgccgagaacagcguggccuacuccaacaacucuaucgcuauccccaccaacuucaccaucagcgugaccacagagauccugccuguguccaugaccaagaccagcguggacugcaccauguacaucugcggcgauuccaccgagugcuccaaccugcugcugcaguacggcagcuucugcacccagcugaauagagcccugacagggaucgccguggaacaggacaagaacacccaagagguguucgcccaagugaagcagaucuacaagaccccuccuaucaaggacuucggcggcuucaauuucagccagauucugcccgauccuagcaagcccagcaagcggagcuucaucgaggaccugcuguucaacaaagugacacuggccgacgccggcuucaucaagcaguauggcgauugucugggcgacauugccgccagggaucugauuugcgcccagaaguuuaacggacugacagugcugccuccucugcugaccgaugagaugaucgcccaguacacaucugcccugcuggccggcacaaucacaagcggcuggacauuuggagcaggcgccgcucugcagauccccuuugcuaugcagauggccuaccgguucaacggcaucggagugacccagaaugugcuguacgagaaccagaagcugaucgccaaccaguucaacagcgccaucggcaagauccaggacagccugagcagcacagcaagcgcccugggaaagcugcaggacguggucaaccagaaugcccaggcacugaacacccuggucaagcagcuguccuccaacuucggcgccaucagcucugugcugaacgauauccugagcagacuggacccuccugaggccgaggugcagaucgacagacugaucacaggcagacugcagagccuccagacauacgugacccagcagcugaucagagccgccgagauuagagccucugccaaucuggccgccaucaagaugucugagugugugcugggccagagcaagagaguggacuuuugcggcaagggcuaccaccugaugagcuucccucagucugccccucacggcgugguguuucugcacgugacauaugugcccgcucaagagaagaauuucaccaccgcuccagccaucugccacgacggcaaagcccacuuuccuagagaaggcguguucguguccaacggcacccauugguucgugacacagcggaacuucuacgagccccagaucaucaccaccgacaacaccuucgugucuggcaacugcgacgucgugaucggcauugugaacaauaccguguacgacccucugcagcccgagcuggacagcuucaaagaggaacuggacaaguacuuuaagaaccacacaagccccgacguggaccugggcgauaucagcggaaucaaugccagcuucgugaacauccagaaagagaucgaccggcugaacgagguggccaagaaucugaacgagagccugaucgaccugcaagaacuggggaaguacgagcaguacaucaaguggcccugguacaucuggcugggcuuuaucgccggacugauugccaucgugauggucacaaucaugcuguguugcaugaccagcugcuguagcugccugaagggcuguuguagcuguggcagcugcugcaaguucgacgaggacgauucugagcccgugcugaagggcgugaaacugcacuacacaugaugacucgagguguguggaggacacccugaaccccccgcuuucaaacaaguuuucaaauuguuugaggucaggauuucucaaacugauuccuuucuuugcauaugaguauuugaaaauaaauauuuucccagaauauaaauaaaucaucacaugauuauuuuaacuaugcuagcaaaaaaaaaaaaaaaaaaaaaaaaaaaaaaaaaaaaaaaaaaaaaaaaaaaaaaaaaaaaaaaaaaaaaaaaaaaaaaaaaaaaaaaaaaaaaaaaaaaa

SEQ ID NO: 67 - RNA, 4151 nt, Artificial
  delta variant S protein mRNA containing 5'-UTR, 3'-UTR and polyA
gaguccuccccauccucucccucugucccucugucccucugacccugcacugucccagcaccauguucguguuccuggugcugcugccucugguguccagccagugugugaaccugagaaccagaacacagcugccuccagccuacaccaacagcuuuaccagaggcguguacuaccccgacaagguguucagauccagcgugcugcacucuacccaggaccuguuccugccuuucuucagcaacgugaccugguuccacgccauccacguguccggcaccaauggcaccaagagauucgacaaccccgugcugcccuucaacgacgggguguacuuugccagcaccgagaaguccaacaucaucagaggcuggaucuucggcaccacacuggacagcaagacccagagccugcugaucgugaacaacgccaccaacguggucaucaaagugugcgaguuccaguucugcaacgaccccuuccuggacgucuacuaccacaagaacaacaagagcuggauggaaagcggcguguacagcagcgccaacaacugcaccuucgaguacgugucccagccuuuccugauggaccuggaaggcaagcagggcaacuucaagaaccugcgcgaguucguguuuaagaacaucgacggcuacuucaagaucuacagcaagcacaccccuaucaaccucgugcgggaucugccucagggcuucucugcucuggaaccccugguggaucugcccaucggcaucaacaucacccgguuucagacacugcuggcccugcacagaagcuaccugacaccuggcgauagcagcagcggauggacagcuggugccgccgcuuacuaugugggcuaccugcagccuagaaccuuccugcugaaguacaacgagaacggcaccaucaccgacgccguggauugugcucuggauccucugagcgagacaaagugcacccugaaguccuucaccguggaaaagggcaucuaccagaccagcaacuuccgggugcagcccaccgaauccaucgugcgguuccccaauaucaccaaucugugccccuucggcgagguguucaaugccaccagauucgccucuguguacgccuggaaccggaagcggaucagcaauugcguggccgacuacuccgugcuguacaacuccgccagcuucagcaccuucaagugcuacggcguguccccuaccaagcugaacgaccugugcuucacaaacguguacgccgacagcuucgugauccggggagaugaagugcggcagauugccccuggacagacaggcaagaucgccgacuacaacuacaagcugcccgacgacuucaccggcugugugauugccuggaacagcaacaaccuggacuccaaagucggcggcaacuacaauuaccgguaccggcuguuccggaaguccaaucugaagcccuucgagcgggacaucuccaccgagaucuaucaggccggcagcaagccuuguaacggcguggaaggcuucaacugcuacuucccacugcaguccuacggcuuucagcccacaaauggcgugggcuaucagcccuacagagugguggugcugagcuucgaacugcugcaugccccugccacagugugcggcccuaagaaaagcaccaaucucgugaagaacaaaugcgugaacuucaacuucaacggccugaccggcaccggcgugcugacagagagcaacaagaaguuccugccauuccagcaguuuggccgggauaucgccgauaccacagacgccguuagagauccccagacacuggaaauccuggacaucaccccuugcagcuucggcggagugucugugaucaccccuggcaccaacaccagcaaucagguggcagugcuguaccagggcgugaacuguaccgaagugcccguggccauucacgccgaucagcugacaccuacauggcggguguacuccaccggcagcaauguguuucagaccagagccggcugucugaucggagccgagcacgugaacaauagcuacgagugcgacauccccaucggcgcuggaaucugcgccagcuaccagacacagacaaacagccggcggagagccagaagcguggccagccagagcaucauugccuacacaaugucucugggcgccgagaacagcguggccuacuccaacaacucuaucgcuauccccaccaacuucaccaucagcgugaccacagagauccugccuguguccaugaccaagaccagcguggacugcaccauguacaucugcggcgauuccaccgagugcuccaaccugcugcugcaguacggcagcuucugcacccagcugaauagagcccugacagggaucgccguggaacaggacaagaacacccaagagguguucgcccaagugaagcagaucuacaagaccccuccuaucaaggacuucggcggcuucaauuucagccagauucugcccgauccuagcaagcccagcaagcggagcuucaucgaggaccugcuguucaacaaagugacacuggccgacgccggcuucaucaagcaguauggcgauugucugggcgacauugccgccagggaucugauuugcgcccagaaguuuaacggacugacagugcugccuccucugcugaccgaugagaugaucgcccaguacacaucugcccugcuggccggcacaaucacaagcggcuggacauuuggagcaggcgccgcucugcagauccccuuugcuaugcagauggccuaccgguucaacggcaucggagugacccagaaugugcuguacgagaaccagaagcugaucgccaaccaguucaacagcgccaucggcaagauccaggacagccugagcagcacagcaagcgcccugggaaagcugcagaacguggucaaccagaaugcccaggcacugaacacccuggucaagcagcuguccuccaacuucggcgccaucagcucugugcugaacgauauccugagcagacuggacccuccugaggccgaggugcagaucgacagacugaucacaggcagacugcagagccuccagacauacgugacccagcagcugaucagagccgccgagauuagagccucugccaaucuggccgccaccaagaugucugagugugugcugggccagagcaagagaguggacuuuugcggcaagggcuaccaccugaugagcuucccucagucugccccucacggcgugguguuucugcacgugacauaugugcccgcucaagagaagaauuucaccaccgcuccagccaucugccacgacggcaaagcccacuuuccuagagaaggcguguucguguccaacggcacccauugguucgugacacagcggaacuucuacgagccccagaucaucaccaccgacaacaccuucgugucuggcaacugcgacgucgugaucggcauugugaacaauaccguguacgacccucugcagcccgagcuggacagcuucaaagaggaacuggacaaguacuuuaagaaccacacaagccccgacguggaccugggcgauaucagcggaaucaaugccagcgucgugaacauccagaaagagaucgaccggcugaacgagguggccaagaaucugaacgagagccugaucgaccugcaagaacuggggaaguacgagcaguacaucaaguggcccugguacaucuggcugggcuuuaucgccggacugauugccaucgugauggucacaaucaugcuguguugcaugaccagcugcuguagcugccugaagggcuguuguagcuguggcagcugcugcaaguucgacgaggacgauucugagcccgugcugaagggcgugaaacugcacuacacaugaugacucgagguguguggaggacacccugaaccccccgcuuucaaacaaguuuucaaauuguuugaggucaggauuucucaaacugauuccuuucuuugcauaugaguauuugaaaauaaauauuuucccagaauauaaauaaaucaucacaugauuauuuuaacuaugcuagcaaaaaaaaaaaaaaaaaaaaaaaaaaaaaaaaaaaaaaaaaaaaaaaaaaaaaaaaaaaaaaaaaaaaaaaaaaaaaaaaaaaaaaaaaaaaaaaaaaaa

SEQ ID NO: 68 - RNA, 4157 nt, Artificial
  Epsilon variant S protein mRNA containing 5'-UTR, 3'-UTR and polyA
gaguccuccccauccucucccucugucccucugucccucugacccugcacugucccagcaccauguucguguuccuggugcugcugccucugguguccauccagugugugaaccugaccaccagaacacagcugccuccagccuacaccaacagcuuuaccagaggcguguacuaccccgacaagguguucagauccagcgugcugcacucuacccaggaccuguuccugccuuucuucagcaacgugaccugguuccacgccauccacguguccggcaccaauggcaccaagagauucgacaaccccgugcugcccuucaacgacgggguguacuuugccagcaccgagaaguccaacaucaucagaggcuggaucuucggcaccacacuggacagcaagacccagagccugcugaucgugaacaacgccaccaacguggucaucaaagugugcgaguuccaguucugcaacgaccccuuccugggcgucuacuaccacaagaacaacaagagcugcauggaaagcgaguuccggguguacagcagcgccaacaacugcaccuucgaguacgugucccagccuuuccugauggaccuggaaggcaagcagggcaacuucaagaaccugcgcgaguucguguuuaagaacaucgacggcuacuucaagaucuacagcaagcacaccccuaucaaccucgugcgggaucugccucagggcuucucugcucuggaaccccugguggaucugcccaucggcaucaacaucacccgguuucagacacugcuggcccugcacagaagcuaccugacaccuggcgauagcagcagcggauggacagcuggugccgccgcuuacuaugugggcuaccugcagccuagaaccuuccugcugaaguacaacgagaacggcaccaucaccgacgccguggauugugcucuggauccucugagcgagacaaagugcacccugaaguccuucaccguggaaaagggcaucuaccagaccagcaacuuccgggugcagcccaccgaauccaucgugcgguuccccaauaucaccaaucugugccccuucggcgagguguucaaugccaccagauucgccucuguguacgccuggaaccggaagcggaucagcaauugcguggccgacuacuccgugcuguacaacuccgccagcuucagcaccuucaagugcuacggcguguccccuaccaagcugaacgaccugugcuucacaaacguguacgccgacagcuucgugauccggggagaugaagugcggcagauugccccuggacagacaggcaagaucgccgacuacaacuacaagcugcccgacgacuucaccggcugugugauugccuggaacagcaacaaccuggacuccaaagucggcggcaacuacaauuaccgcuaccggcuguuccggaaguccaaucugaagcccuucgagcgggacaucuccaccgagaucuaucaggccggcagcaccccuuguaacggcguggaaggcuucaacugcuacuucccacugcaguccuacggcuuucagcccacaaauggcgugggcuaucagcccuacagagugguggugcugagcuucgaacugcugcaugccccugccacagugugcggcccuaagaaaagcaccaaucucgugaagaacaaaugcgugaacuucaacuucaacggccugaccggcaccggcgugcugacagagagcaacaagaaguuccugccauuccagcaguuuggccgggauaucgccgauaccacagacgccguuagagauccccagacacuggaaauccuggacaucaccccuugcagcuucggcggagugucugugaucaccccuggcaccaacaccagcaaucagguggcagugcuguaccagggcgugaacuguaccgaagugcccguggccauucacgccgaucagcugacaccuacauggcggguguacuccaccggcagcaauguguuucagaccagagccggcugucugaucggagccgagcacgugaacaauagcuacgagugcgacauccccaucggcgcuggaaucugcgccagcuaccagacacagacaaacagcccucggagagccagaagcguggccagccagagcaucauugccuacacaaugucucugggcgccgagaacagcguggccuacuccaacaacucuaucgcuauccccaccaacuucaccaucagcgugaccacagagauccugccuguguccaugaccaagaccagcguggacugcaccauguacaucugcggcgauuccaccgagugcuccaaccugcugcugcaguacggcagcuucugcacccagcugaauagagcccugacagggaucgccguggaacaggacaagaacacccaagagguguucgcccaagugaagcagaucuacaagaccccuccuaucaaggacuucggcggcuucaauuucagccagauucugcccgauccuagcaagcccagcaagcggagcuucaucgaggaccugcuguucaacaaagugacacuggccgacgccggcuucaucaagcaguauggcgauugucugggcgacauugccgccagggaucugauuugcgcccagaaguuuaacggacugacagugcugccuccucugcugaccgaugagaugaucgcccaguacacaucugcccugcuggccggcacaaucacaagcggcuggacauuuggagcaggcgccgcucugcagauccccuuugcuaugcagauggccuaccgguucaacggcaucggagugacccagaaugugcuguacgagaaccagaagcugaucgccaaccaguucaacagcgccaucggcaagauccaggacagccugagcagcacagcaagcgcccugggaaagcugcaggacguggucaaccagaaugcccaggcacugaacacccuggucaagcagcuguccuccaacuucggcgccaucagcucugugcugaacgauauccugagcagacuggacccuccugaggccgaggugcagaucgacagacugaucacaggcagacugcagagccuccagacauacgugacccagcagcugaucagagccgccgagauuagagccucugccaaucuggccgccaccaagaugucugagugugugcugggccagagcaagagaguggacuuuugcggcaagggcuaccaccugaugagcuucccucagucugccccucacggcgugguguuucugcacgugacauaugugcccgcucaagagaagaauuucaccaccgcuccagccaucugccacgacggcaaagcccacuuuccuagagaaggcguguucguguccaacggcacccauugguucgugacacagcggaacuucuacgagccccagaucaucaccaccgacaacaccuucgugucuggcaacugcgacgucgugaucggcauugugaacaauaccguguacgacccucugcagcccgagcuggacagcuucaaagaggaacuggacaaguacuuuaagaaccacacaagccccgacguggaccugggcgauaucagcggaaucaaugccagcgucgugaacauccagaaagagaucgaccggcugaacgagguggccaagaaucugaacgagagccugaucgaccugcaagaacuggggaaguacgagcaguacaucaaguggcccugguacaucuggcugggcuuuaucgccggacugauugccaucgugauggucacaaucaugcuguguugcaugaccagcugcuguagcugccugaagggcuguuguagcuguggcagcugcugcaaguucgacgaggacgauucugagcccgugcugaagggcgugaaacugcacuacacaugaugacucgagguguguggaggacacccugaaccccccgcuuucaaacaaguuuucaaauuguuugaggucaggauuucucaaacugauuccuuucuuugcauaugaguauuugaaaauaaauauuuucccagaauauaaauaaaucaucacaugauuauuuuaacuaugcuagcaaaaaaaaaaaaaaaaaaaaaaaaaaaaaaaaaaaaaaaaaaaaaaaaaaaaaaaaaaaaaaaaaaaaaaaaaaaaaaaaaaaaaaaaaaaaaaaaaaaa

SEQ ID NO: 69 - RNA, 4148 nt, Artificial
  Omicron variant S protein mRNA containing 5'-UTR, 3'-UTR and polyA
gaguccuccccauccucucccucugucccucugucccucugacccugcacugucccagcaccauguucguguuccuggugcugcugccucugguguccagccagugugugaaccugaccaccagaacacagcugccuccagccuacaccaacagcuuuaccagaggcguguacuaccccgacaagguguucagauccagcgugcugcacucuacccaggaccuguuccugccuuucuucagcaacgugaccugguuccacgugaucuccggcaccaauggcaccaagagauucgacaaccccgugcugcccuucaacgacgggguguacuuugccagcaucgagaaguccaacaucaucagaggcuggaucuucggcaccacacuggacagcaagacccagagccugcugaucgugaacaacgccaccaacguggucaucaaagugugcgaguuccaguucugcaacgaccccuuccuggaccacaagaacaacaagagcuggauggaaagcgaguuccggguguacagcagcgccaacaacugcaccuucgaguacgugucccagccuuuccugauggaccuggaaggcaagcagggcaacuucaagaaccugcgcgaguucguguuuaagaacaucgacggcuacuucaagaucuacagcaagcacaccccuaucaucgugcgggaaccugaagaucugccucagggcuucucugcucuggaaccccugguggaucugcccaucggcaucaacaucacccgguuucagacacugcuggcccugcacagaagcuaccugacaccuggcgauagcagcagcggauggacagcuggugccgccgcuuacuaugugggcuaccugcagccuagaaccuuccugcugaaguacaacgagaacggcaccaucaccgacgccguggauugugcucuggauccucugagcgagacaaagugcacccugaaguccuucaccguggaaaagggcaucuaccagaccagcaacuuccgggugcagcccaccgaauccaucgugcgguuccccaauaucaccaaucugugccccuucgacgagguguucaaugccaccagauucgccucuguguacgccuggaaccggaagcggaucagcaauugcguggccgacuacuccgugcuguacaaccuggcccccuucuucaccuucaagugcuacggcguguccccuaccaagcugaacgaccugugcuucacaaacguguacgccgacagcuucgugauccggggagaugaagugcggcagauugccccuggacagacaggcaacaucgccgacuacaacuacaagcugcccgacgacuucaccggcugugugauugccuggaacagcaacaagcuggacuccaaagucuccggcaacuacaauuaccuguaccggcuguuccggaaguccaaucugaagcccuucgagcgggacaucuccaccgagaucuaucaggccggcaacaagccuuguaacggcguggccggcuucaacugcuacuucccacugcgguccuacuccuuucggcccacauauggcgugggccaucagcccuacagagugguggugcugagcuucgaacugcugcaugccccugccacagugugcggcccuaagaaaagcaccaaucucgugaagaacaaaugcgugaacuucaacuucaacggccugaagggcaccggcgugcugacagagagcaacaagaaguuccugccauuccagcaguuuggccgggauaucgccgauaccacagacgccguuagagauccccagacacuggaaauccuggacaucaccccuugcagcuucggcggagugucugugaucaccccuggcaccaacaccagcaaucagguggcagugcuguaccagggcgugaacuguaccgaagugcccguggccauucacgccgaucagcugacaccuacauggcggguguacuccaccggcagcaauguguuucagaccagagccggcugucugaucggagccgaguacgugaacaauagcuacgagugcgacauccccaucggcgcuggaaucugcgccagcuaccagacacagacaaagagccaucggagagccagaagcguggccagccagagcaucauugccuacacaaugucucugggcgccgagaacagcguggccuacuccaacaacucuaucgcuauccccaccaacuucaccaucagcgugaccacagagauccugccuguguccaugaccaagaccagcguggacugcaccauguacaucugcggcgauuccaccgagugcuccaaccugcugcugcaguacggcagcuucugcacccagcugaagagagcccugacagggaucgccguggaacaggacaagaacacccaagagguguucgcccaagugaagcagaucuacaagaccccuccuaucaaguacuucggcggcuucaauuucagccagauucugcccgauccuagcaagcccagcaagcggagcuucaucgaggaccugcuguucaacaaagugacacuggccgacgccggcuucaucaagcaguauggcgauugucugggcgacauugccgccagggaucugauuugcgcccagaaguuuaagggacugacagugcugccuccucugcugaccgaugagaugaucgcccaguacacaucugcccugcuggccggcacaaucacaagcggcuggacauuuggagcaggcgccgcucugcagauccccuuugcuaugcagauggccuaccgguucaacggcaucggagugacccagaaugugcuguacgagaaccagaagcugaucgccaaccaguucaacagcgccaucggcaagauccaggacagccugagcagcacagcaagcgcccugggaaagcugcaggacguggucaaccacaaugcccaggcacugaacacccuggucaagcagcuguccuccaaguucggcgccaucagcucugugcugaacgauaucuucagcagacuggacccuccugaggccgaggugcagaucgacagacugaucacaggcagacugcagagccuccagacauacgugacccagcagcugaucagagccgccgagauuagagccucugccaaucuggccgccaccaagaugucugagugugugcugggccagagcaagagaguggacuuuugcggcaagggcuaccaccugaugagcuucccucagucugccccucacggcgugguguuucugcacgugacauaugugcccgcucaagagaagaauuucaccaccgcuccagccaucugccacgacggcaaagcccacuuuccuagagaaggcguguucguguccaacggcacccauugguucgugacacagcggaacuucuacgagccccagaucaucaccaccgacaacaccuucgugucuggcaacugcgacgucgugaucggcauugugaacaauaccguguacgacccucugcagcccgagcuggacagcuucaaagaggaacuggacaaguacuuuaagaaccacacaagccccgacguggaccugggcgauaucagcggaaucaaugccagcgucgugaacauccagaaagagaucgaccggcugaacgagguggccaagaaucugaacgagagccugaucgaccugcaagaacuggggaaguacgagcaguacaucaaguggcccugguacaucuggcugggcuuuaucgccggacugauugccaucgugauggucacaaucaugcuguguugcaugaccagcugcuguagcugccugaagggcuguuguagcuguggcagcugcugcaaguucgacgaggacgauucugagcccgugcugaagggcgugaaacugcacuacacaugaugacucgagguguguggaggacacccugaaccccccgcuuucaaacaaguuuucaaauuguuugaggucaggauuucucaaacugauuccuuucuuugcauaugaguauuugaaaauaaauauuuucccagaauauaaauaaaucaucacaugauuauuuuaacuaugcuagcaaaaaaaaaaaaaaaaaaaaaaaaaaaaaaaaaaaaaaaaaaaaaaaaaaaaaaaaaaaaaaaaaaaaaaaaaaaaaaaaaaaaaaaaaaaaaaaaaaaa

SEQ ID NO: 70 - RNA, 4157 nt, Artificial
  SARS-CoV2 S protein mRNA containing 5'-UTR, 3'-UTR and polyA
gagugcuccccauccaacuaaacugucccucuguccgaacuaaacugcacugucccagcaccauguucguguuccuggugcugcugccucugguguccagccagugugugaaccugaccaccagaacacagcugccuccagccuacaccaacagcuuuaccagaggcguguacuaccccgacaagguguucagauccagcgugcugcacucuacccaggaccuguuccugccuuucuucagcaacgugaccugguuccacgccauccacguguccggcaccaauggcaccaagagauucgacaaccccgugcugcccuucaacgacgggguguacuuugccagcaccgagaaguccaacaucaucagaggcuggaucuucggcaccacacuggacagcaagacccagagccugcugaucgugaacaacgccaccaacguggucaucaaagugugcgaguuccaguucugcaacgaccccuuccugggcgucuacuaccacaagaacaacaagagcuggauggaaagcgaguuccggguguacagcagcgccaacaacugcaccuucgaguacgugucccagccuuuccugauggaccuggaaggcaagcagggcaacuucaagaaccugcgcgaguucguguuuaagaacaucgacggcuacuucaagaucuacagcaagcacaccccuaucaaccucgugcgggaucugccucagggcuucucugcucuggaaccccugguggaucugcccaucggcaucaacaucacccgguuucagacacugcuggcccugcacagaagcuaccugacaccuggcgauagcagcagcggauggacagcuggugccgccgcuuacuaugugggcuaccugcagccuagaaccuuccugcugaaguacaacgagaacggcaccaucaccgacgccguggauugugcucuggauccucugagcgagacaaagugcacccugaaguccuucaccguggaaaagggcaucuaccagaccagcaacuuccgggugcagcccaccgaauccaucgugcgguuccccaauaucaccaaucugugccccuucggcgagguguucaaugccaccagauucgccucuguguacgccuggaaccggaagcggaucagcaauugcguggccgacuacuccgugcuguacaacuccgccagcuucagcaccuucaagugcuacggcguguccccuaccaagcugaacgaccugugcuucacaaacguguacgccgacagcuucgugauccggggagaugaagugcggcagauugccccuggacagacaggcaagaucgccgacuacaacuacaagcugcccgacgacuucaccggcugugugauugccuggaacagcaacaaccuggacuccaaagucggcggcaacuacaauuaccuguaccggcuguuccggaaguccaaucugaagcccuucgagcgggacaucuccaccgagaucuaucaggccggcagcaccccuuguaacggcguggaaggcuucaacugcuacuucccacugcaguccuacggcuuucagcccacaaauggcgugggcuaucagcccuacagagugguggugcugagcuucgaacugcugcaugccccugccacagugugcggcccuaagaaaagcaccaaucucgugaagaacaaaugcgugaacuucaacuucaacggccugaccggcaccggcgugcugacagagagcaacaagaaguuccugccauuccagcaguuuggccgggauaucgccgauaccacagacgccguuagagauccccagacacuggaaauccuggacaucaccccuugcagcuucggcggagugucugugaucaccccuggcaccaacaccagcaaucagguggcagugcuguaccaggacgugaacuguaccgaagugcccguggccauucacgccgaucagcugacaccuacauggcggguguacuccaccggcagcaauguguuucagaccagagccggcugucugaucggagccgagcacgugaacaauagcuacgagugcgacauccccaucggcgcuggaaucugcgccagcuaccagacacagacaaacagcccucggagagccagaagcguggccagccagagcaucauugccuacacaaugucucugggcgccgagaacagcguggccuacuccaacaacucuaucgcuauccccaccaacuucaccaucagcgugaccacagagauccugccuguguccaugaccaagaccagcguggacugcaccauguacaucugcggcgauuccaccgagugcuccaaccugcugcugcaguacggcagcuucugcacccagcugaauagagcccugacagggaucgccguggaacaggacaagaacacccaagagguguucgcccaagugaagcagaucuacaagaccccuccuaucaaggacuucggcggcuucaauuucagccagauucugcccgauccuagcaagcccagcaagcggagcuucaucgaggaccugcuguucaacaaagugacacuggccgacgccggcuucaucaagcaguauggcgauugucugggcgacauugccgccagggaucugauuugcgcccagaaguuuaacggacugacagugcugccuccucugcugaccgaugagaugaucgcccaguacacaucugcccugcuggccggcacaaucacaagcggcuggacauuuggagcaggcgccgcucugcagauccccuuugcuaugcagauggccuaccgguucaacggcaucggagugacccagaaugugcuguacgagaaccagaagcugaucgccaaccaguucaacagcgccaucggcaagauccaggacagccugagcagcacagcaagcgcccugggaaagcugcaggacguggucaaccagaaugcccaggcacugaacacccuggucaagcagcuguccuccaacuucggcgccaucagcucugugcugaacgauauccugagcagacuggacccuccugaggccgaggugcagaucgacagacugaucacaggcagacugcagagccuccagacauacgugacccagcagcugaucagagccgccgagauuagagccucugccaaucuggccgccaccaagaugucugagugugugcugggccagagcaagagaguggacuuuugcggcaagggcuaccaccugaugagcuucccucagucugccccucacggcgugguguuucugcacgugacauaugugcccgcucaagagaagaauuucaccaccgcuccagccaucugccacgacggcaaagcccacuuuccuagagaaggcguguucguguccaacggcacccauugguucgugacacagcggaacuucuacgagccccagaucaucaccaccgacaacaccuucgugucuggcaacugcgacgucgugaucggcauugugaacaauaccguguacgacccucugcagcccgagcuggacagcuucaaagaggaacuggacaaguacuuuaagaaccacacaagccccgacguggaccugggcgauaucagcggaaucaaugccagcgucgugaacauccagaaagagaucgaccggcugaacgagguggccaagaaucugaacgagagccugaucgaccugcaagaacuggggaaguacgagcaguacaucaaguggcccugguacaucuggcugggcuuuaucgccggacugauugccaucgugauggucacaaucaugcuguguugcaugaccagcugcuguagcugccugaagggcuguuguagcuguggcagcugcugcaaguucgacgaggacgauucugagcccgugcugaagggcgugaaacugcacuacacaugaugacucgagguguguggaggacacccugaaccccccgcuuucaaacaaguuuucaaauuguuugaggucaggauuucucaaacugauuccuuucuuugcauaugaguauuugaaaauaaauauuuucccagaauauaaauaaaucaucacaugauuauuuuaacuaugcuagcaaaaaaaaaaaaaaaaaaaaaaaaaaaaaaaaaaaaaaaaaaaaaaaaaaaaaaaaaaaaaaaaaaaaaaaaaaaaaaaaaaaaaaaaaaaaaaaaaaaa

SEQ ID NO: 71 - RNA, 4148 nt, Artificial
  Alpha variant S protein mRNA containing 5'-UTR, 3'-UTR and polyA
gagugcuccccauccaacuaaacugucccucuguccgaacuaaacugcacugucccagcaccauguucguguuccuggugcugcugccucugguguccagccagugugugaaccugaccaccagaacacagcugccuccagccuacaccaacagcuuuaccagaggcguguacuaccccgacaagguguucagauccagcgugcugcacucuacccaggaccuguuccugccuuucuucagcaacgugaccugguuccacgccaucuccggcaccaauggcaccaagagauucgacaaccccgugcugcccuucaacgacgggguguacuuugccagcaccgagaaguccaacaucaucagaggcuggaucuucggcaccacacuggacagcaagacccagagccugcugaucgugaacaacgccaccaacguggucaucaaagugugcgaguuccaguucugcaacgaccccuuccugggcgucuaccacaagaacaacaagagcuggauggaaagcgaguuccggguguacagcagcgccaacaacugcaccuucgaguacgugucccagccuuuccugauggaccuggaaggcaagcagggcaacuucaagaaccugcgcgaguucguguuuaagaacaucgacggcuacuucaagaucuacagcaagcacaccccuaucaaccucgugcgggaucugccucagggcuucucugcucuggaaccccugguggaucugcccaucggcaucaacaucacccgguuucagacacugcuggcccugcacagaagcuaccugacaccuggcgauagcagcagcggauggacagcuggugccgccgcuuacuaugugggcuaccugcagccuagaaccuuccugcugaaguacaacgagaacggcaccaucaccgacgccguggauugugcucuggauccucugagcgagacaaagugcacccugaaguccuucaccguggaaaagggcaucuaccagaccagcaacuuccgggugcagcccaccgaauccaucgugcgguuccccaauaucaccaaucugugccccuucggcgagguguucaaugccaccagauucgccucuguguacgccuggaaccggaagcggaucagcaauugcguggccgacuacuccgugcuguacaacuccgccagcuucagcaccuucaagugcuacggcguguccccuaccaagcugaacgaccugugcuucacaaacguguacgccgacagcuucgugauccggggagaugaagugcggcagauugccccuggacagacaggcaagaucgccgacuacaacuacaagcugcccgacgacuucaccggcugugugauugccuggaacagcaacaaccuggacuccaaagucggcggcaacuacaauuaccuguaccggcuguuccggaaguccaaucugaagcccuucgagcgggacaucuccaccgagaucuaucaggccggcagcaccccuuguaacggcguggaaggcuucaacugcuacuucccacugcaguccuacggcuuucagcccacauacggcgugggcuaucagcccuacagagugguggugcugagcuucgaacugcugcaugccccugccacagugugcggcccuaagaaaagcaccaaucucgugaagaacaaaugcgugaacuucaacuucaacggccugaccggcaccggcgugcugacagagagcaacaagaaguuccugccauuccagcaguuuggccgggauaucgacgauaccacagacgccguuagagauccccagacacuggaaauccuggacaucaccccuugcagcuucggcggagugucugugaucaccccuggcaccaacaccagcaaucagguggcagugcuguaccagggcgugaacuguaccgaagugcccguggccauucacgccgaucagcugacaccuacauggcggguguacuccaccggcagcaauguguuucagaccagagccggcugucugaucggagccgagcacgugaacaauagcuacgagugcgacauccccaucggcgcuggaaucugcgccagcuaccagacacagacaaacagccaccggagagccagaagcguggccagccagagcaucauugccuacacaaugucucugggcgccgagaacagcguggccuacuccaacaacucuaucgcuauccccaucaacuucaccaucagcgugaccacagagauccugccuguguccaugaccaagaccagcguggacugcaccauguacaucugcggcgauuccaccgagugcuccaaccugcugcugcaguacggcagcuucugcacccagcugaauagagcccugacagggaucgccguggaacaggacaagaacacccaagagguguucgcccaagugaagcagaucuacaagaccccuccuaucaaggacuucggcggcuucaauuucagccagauucugcccgauccuagcaagcccagcaagcggagcuucaucgaggaccugcuguucaacaaagugacacuggccgacgccggcuucaucaagcaguauggcgauugucugggcgacauugccgccagggaucugauuugcgcccagaaguuuaacggacugacagugcugccuccucugcugaccgaugagaugaucgcccaguacacaucugcccugcuggccggcacaaucacaagcggcuggacauuuggagcaggcgccgcucugcagauccccuuugcuaugcagauggccuaccgguucaacggcaucggagugacccagaaugugcuguacgagaaccagaagcugaucgccaaccaguucaacagcgccaucggcaagauccaggacagccugagcagcacagcaagcgcccugggaaagcugcaggacguggucaaccagaaugcccaggcacugaacacccuggucaagcagcuguccuccaacuucggcgccaucagcucugugcugaacgauauccuggcaagacuggacccuccugaggccgaggugcagaucgacagacugaucacaggcagacugcagagccuccagacauacgugacccagcagcugaucagagccgccgagauuagagccucugccaaucuggccgccaccaagaugucugagugugugcugggccagagcaagagaguggacuuuugcggcaagggcuaccaccugaugagcuucccucagucugccccucacggcgugguguuucugcacgugacauaugugcccgcucaagagaagaauuucaccaccgcuccagccaucugccacgacggcaaagcccacuuuccuagagaaggcguguucguguccaacggcacccauugguucgugacacagcggaacuucuacgagccccagaucaucaccacccacaacaccuucgugucuggcaacugcgacgucgugaucggcauugugaacaauaccguguacgacccucugcagcccgagcuggacagcuucaaagaggaacuggacaaguacuuuaagaaccacacaagccccgacguggaccugggcgauaucagcggaaucaaugccagcgucgugaacauccagaaagagaucgaccggcugaacgagguggccaagaaucugaacgagagccugaucgaccugcaagaacuggggaaguacgagcaguacaucaaguggcccugguacaucuggcugggcuuuaucgccggacugauugccaucgugauggucacaaucaugcuguguugcaugaccagcugcuguagcugccugaagggcuguuguagcuguggcagcugcugcaaguucgacgaggacgauucugagcccgugcugaagggcgugaaacugcacuacacaugaugacucgagguguguggaggacacccugaaccccccgcuuucaaacaaguuuucaaauuguuugaggucaggauuucucaaacugauuccuuucuuugcauaugaguauuugaaaauaaauauuuucccagaauauaaauaaaucaucacaugauuauuuuaacuaugcuagcaaaaaaaaaaaaaaaaaaaaaaaaaaaaaaaaaaaaaaaaaaaaaaaaaaaaaaaaaaaaaaaaaaaaaaaaaaaaaaaaaaaaaaaaaaaaaaaaaaaa

SEQ ID NO: 72 - RNA, 4148 nt, Artificial
  beta variant S protein mRNA containing 5'-UTR, 3'-UTR and polyA
gagugcuccccauccaacuaaacugucccucuguccgaacuaaacugcacugucccagcaccauguucguguuccuggugcugcugccucugguguccagccagugugugaacuucaccaccagaacacagcugccuccagccuacaccaacagcuuuaccagaggcguguacuaccccgacaagguguucagauccagcgugcugcacucuacccaggaccuguuccugccuuucuucagcaacgugaccugguuccacgccauccacguguccggcaccaauggcaccaagagauucgccaaccccgugcugcccuucaacgacgggguguacuuugccagcaccgagaaguccaacaucaucagaggcuggaucuucggcaccacacuggacagcaagacccagagccugcugaucgugaacaacgccaccaacguggucaucaaagugugcgaguuccaguucugcaacgaccccuuccugggcgucuacuaccacaagaacaacaagagcuggauggaaagcgaguuccggguguacagcagcgccaacaacugcaccuucgaguacgugucccagccuuuccugauggaccuggaaggcaagcagggcaacuucaagaaccugcgcgaguucguguuuaagaacaucgacggcuacuucaagaucuacagcaagcacaccccuaucaaccucgugcggggucugccucagggcuucucugcucuggaaccccugguggaucugcccaucggcaucaacaucacccgguuucagacacugcacagaagcuaccugacaccuggcgauagcagcagcggauggacagcuggugccgccgcuuacuaugugggcuaccugcagccuagaaccuuccugcugaaguacaacgagaacggcaccaucaccgacgccguggauugugcucuggauccucugagcgagacaaagugcacccugaaguccuucaccguggaaaagggcaucuaccagaccagcaacuuccgggugcagcccaccgaauccaucgugcgguuccccaauaucaccaaucugugccccuucggcgagguguucaaugccaccagauucgccucuguguacgccuggaaccggaagcggaucagcaauugcguggccgacuacuccgugcuguacaacuccgccagcuucagcaccuucaagugcuacggcguguccccuaccaagcugaacgaccugugcuucacaaacguguacgccgacagcuucgugauccggggagaugaagugcggcagauugccccuggacagacaggcaauaucgccgacuacaacuacaagcugcccgacgacuucaccggcugugugauugccuggaacagcaacaaccuggacuccaaagucggcggcaacuacaauuaccuguaccggcuguuccggaaguccaaucugaagcccuucgagcgggacaucuccaccgagaucuaucaggccggcagcaccccuuguaacggcgugaaaggcuucaacugcuacuucccacugcaguccuacggcuuucagcccacauacggcgugggcuaucagcccuacagagugguggugcugagcuucgaacugcugcaugccccugccacagugugcggcccuaagaaaagcaccaaucucgugaagaacaaaugcgugaacuucaacuucaacggccugaccggcaccggcgugcugacagagagcaacaagaaguuccugccauuccagcaguuuggccgggauaucgccgauaccacagacgccguuagagauccccagacacuggaaauccuggacaucaccccuugcagcuucggcggagugucugugaucaccccuggcaccaacaccagcaaucagguggcagugcuguaccagggcgugaacuguaccgaagugcccguggccauucacgccgaucagcugacaccuacauggcggguguacuccaccggcagcaauguguuucagaccagagccggcugucugaucggagccgagcacgugaacaauagcuacgagugcgacauccccaucggcgcuggaaucugcgccagcuaccagacacagacaaacagcccucggagagccagaagcguggccagccagagcaucauugccuacacaaugucucugggcguggagaacagcguggccuacuccaacaacucuaucgcuauccccaccaacuucaccaucagcgugaccacagagauccugccuguguccaugaccaagaccagcguggacugcaccauguacaucugcggcgauuccaccgagugcuccaaccugcugcugcaguacggcagcuucugcacccagcugaauagagcccugacagggaucgccguggaacaggacaagaacacccaagagguguucgcccaagugaagcagaucuacaagaccccuccuaucaaggacuucggcggcuucaauuucagccagauucugcccgauccuagcaagcccagcaagcggagcuucaucgaggaccugcuguucaacaaagugacacuggccgacgccggcuucaucaagcaguauggcgauugucugggcgacauugccgccagggaucugauuugcgcccagaaguuuaacggacugacagugcugccuccucugcugaccgaugagaugaucgcccaguacacaucugcccugcuggccggcacaaucacaagcggcuggacauuuggagcaggcgccgcucugcagauccccuuugcuaugcagauggccuaccgguucaacggcaucggagugacccagaaugugcuguacgagaaccagaagcugaucgccaaccaguucaacagcgccaucggcaagauccaggacagccugagcagcacagcaagcgcccugggaaagcugcaggacguggucaaccagaaugcccaggcacugaacacccuggucaagcagcuguccuccaacuucggcgccaucagcucugugcugaacgauauccugagcagacuggacccuccugaggccgaggugcagaucgacagacugaucacaggcagacugcagagccuccagacauacgugacccagcagcugaucagagccgccgagauuagagccucugccaaucuggccgccaccaagaugucugagugugugcugggccagagcaagagaguggacuuuugcggcaagggcuaccaccugaugagcuucccucagucugccccucacggcgugguguuucugcacgugacauaugugcccgcucaagagaagaauuucaccaccgcuccagccaucugccacgacggcaaagcccacuuuccuagagaaggcguguucguguccaacggcacccauugguucgugacacagcggaacuucuacgagccccagaucaucaccaccgacaacaccuucgugucuggcaacugcgacgucgugaucggcauugugaacaauaccguguacgacccucugcagcccgagcuggacagcuucaaagaggaacuggacaaguacuuuaagaaccacacaagccccgacguggaccugggcgauaucagcggaaucaaugccagcgucgugaacauccagaaagagaucgaccggcugaacgagguggccaagaaucugaacgagagccugaucgaccugcaagaacuggggaaguacgagcaguacaucaaguggcccugguacaucuggcugggcuuuaucgccggacugauugccaucgugauggucacaaucaugcuguguugcaugaccagcugcuguagcugccugaagggcuguuguagcuguggcagcugcugcaaguucgacgaggacgauucugagcccgugcugaagggcgugaaacugcacuacacaugaugacucgagguguguggaggacacccugaaccccccgcuuucaaacaaguuuucaaauuguuugaggucaggauuucucaaacugauuccuuucuuugcauaugaguauuugaaaauaaauauuuucccagaauauaaauaaaucaucacaugauuauuuuaacuaugcuagcaaaaaaaaaaaaaaaaaaaaaaaaaaaaaaaaaaaaaaaaaaaaaaaaaaaaaaaaaaaaaaaaaaaaaaaaaaaaaaaaaaaaaaaaaaaaaaaaaaaa

SEQ ID NO: 73 - RNA, 4157 nt, Artificial
  Gamma S protein mRNA containing 5'-UTR, 3'-UTR and polyA
gagugcuccccauccaacuaaacugucccucuguccgaacuaaacugcacugucccagcaccauguucguguuccuggugcugcugccccuggugagcucccagugcgugaacuuuacaaacagaacacagcugcccuccgccuacacaaacagcuucaccaggggcguguacuaccccgauaaggucuuucgguccagcgugcugcacagcacccaggaucuguuccugccuuucuucagcaacgugacaugguuucacgccauccacgugagcgggacaaacggcaccaagcgguucgauaacccagugcugcccuuuaacgaugggguguacuucgccagcacagagaaguccaacaucaucaggggcuggauuuucggcaccacccucgauuccaagacacagucccugcugaucgugaacaacgccacaaacguggucauuaaggugugcgaguuccaguuuugcaacuacccauuccugggcguguacuaccacaagaacaacaaguccuggauggagagcgaguucagggucuacuccuccgccaacaacugcaccuucgaguacgugagccagcccuuccugauggaucuggagggcaagcaggggaacuucaagaaccugagcgaguucguguucaagaacauugacggcuacuuuaagaucuacaguaagcacacaccuaucaaccuggugcgggaccugccucagggcuucuccgcccucgagccacugguggaucugccaaucggcauuaacaucaccagguuccagacacugcuggcccugcacaggagcuaccugacuccaggcgauagcuccagcggguggacagccggggccgccgccuacuacgugggcuaccugcagcccagaaccuuucugcugaaguacaacgagaacgggaccaucaccgaugccguggauugcgcccuggacccccugagcgagaccaagugcacucucaaguccuucaccguggagaagggcaucuaccagaccagcaacuuccggguccagcccacagaguccaucgugagguuccccaacaucaccaaccucugccccuucggcgagguguucaacgccaccagguuugccagcguguacgccuggaacaggaagaggaucuccaacugcguggccgauuacagcgugcuguacaacuccgccuccuucagcaccuucaagugcuacggcgugagcccuaccaagcuuaacgaucugugcuuuacaaacguguacgccgauagcuuugugauccggggggacgaggugaggcagauugcccccggccagacagggaccaucgccgauuacaacuacaagcugcccgaugacuucaccgggugcgugauugccuggaacagcaacaaccucgauagcaaggucggggggaacuacaacuaccuguacaggcuguuuagaaaguccaaccucaagccuuucgagcgggauauuagcacugagaucuaccaggccgggagcacacccugcaacggggugaagggcuucaacugcuacuuuccccugcagagcuacggcuuccagccaacauacggcgugggguaccagcccuaccgggugguggugcugagcuucgagcugcugcacgccccugccaccgugugcggccccaagaaaagcacuaaccuggugaagaacaagugcgucaacuucaacuuuaacggccugaccggcacaggggugcugaccgaguccaacaagaaguuccugcccuuccagcaguucggccgggacaucgccgauaccacugacgccgugagggacccccagacccuggagauccuggacauuacacccuguagcuucggcggggucagcgugaucacacccggcaccaacacauccaaccagguggccgugcuguaccagggcgugaacugcaccgaggugcccgucgccauccacgccgaccagcugacacccacauggaggguguacagcacagggagcaacguguuccagaccagggccgggugccugaucggcgccgaguacgugaacaacuccuacgagugcgacauccccaucggggccggcauuugcgccuccuaccagacccagaccaacagcccccggcgggccaggagcguggccagccagagcaucauugccuacacaaugucucugggcgccgagaacagcguggccuacuccaacaacucuaucgcuauccccaccaacuucaccaucagcgugaccacagagauccugccuguguccaugaccaagaccagcguggacugcaccauguacaucugcggcgauuccaccgagugcuccaaccugcugcugcaguacggcagcuucugcacccagcugaauagagcccugacagggaucgccguggaacaggacaagaacacccaagagguguucgcccaagugaagcagaucuacaagaccccuccuaucaaggacuucggcggcuucaauuucagccagauucugcccgauccuagcaagcccagcaagcggagcuucaucgaggaccugcuguucaacaaagugacacuggccgacgccggcuucaucaagcaguauggcgauugucugggcgacauugccgccagggaucugauuugcgcccagaaguuuaacggacugacagugcugccuccucugcugaccgaugagaugaucgcccaguacacaucugcccugcuggccggcacaaucacaagcggcuggacauuuggagcaggcgccgcucugcagauccccuuugcuaugcagauggccuaccgguucaacggcaucggagugacccagaaugugcuguacgagaaccagaagcugaucgccaaccaguucaacagcgccaucggcaagauccaggacagccugagcagcacagcaagcgcccugggaaagcugcaggacguggucaaccagaaugcccaggcacugaacacccuggucaagcagcuguccuccaacuucggcgccaucagcucugugcugaacgauauccugagcagacuggacccuccugaggccgaggugcagaucgacagacugaucacaggcagacugcagagccuccagacauacgugacccagcagcugaucagagccgccgagauuagagccucugccaaucuggccgccaucaagaugucugagugugugcugggccagagcaagagaguggacuuuugcggcaagggcuaccaccugaugagcuucccucagucugccccucacggcgugguguuucugcacgugacauaugugcccgcucaagagaagaauuucaccaccgcuccagccaucugccacgacggcaaagcccacuuuccuagagaaggcguguucguguccaacggcacccauugguucgugacacagcggaacuucuacgagccccagaucaucaccaccgacaacaccuucgugucuggcaacugcgacgucgugaucggcauugugaacaauaccguguacgacccucugcagcccgagcuggacagcuucaaagaggaacuggacaaguacuuuaagaaccacacaagccccgacguggaccugggcgauaucagcggaaucaaugccagcuucgugaacauccagaaagagaucgaccggcugaacgagguggccaagaaucugaacgagagccugaucgaccugcaagaacuggggaaguacgagcaguacaucaaguggcccugguacaucuggcugggcuuuaucgccggacugauugccaucgugauggucacaaucaugcuguguugcaugaccagcugcuguagcugccugaagggcuguuguagcuguggcagcugcugcaaguucgacgaggacgauucugagcccgugcugaagggcgugaaacugcacuacacaugaugacucgagguguguggaggacacccugaaccccccgcuuucaaacaaguuuucaaauuguuugaggucaggauuucucaaacugauuccuuucuuugcauaugaguauuugaaaauaaauauuuucccagaauauaaauaaaucaucacaugauuauuuuaacuaugcuagcaaaaaaaaaaaaaaaaaaaaaaaaaaaaaaaaaaaaaaaaaaaaaaaaaaaaaaaaaaaaaaaaaaaaaaaaaaaaaaaaaaaaaaaaaaaaaaaaaaaa

SEQ ID NO: 74 - RNA, 4151 nt, Artificial
  Delta variant S protein mRNA containing 5'-UTR, 3'-UTR and polyA
gagugcuccccauccaacuaaacugucccucuguccgaacuaaacugcacugucccagcaccauguucguguuccuggugcugcugccucugguguccagccagugugugaaccugagaaccagaacacagcugccuccagccuacaccaacagcuuuaccagaggcguguacuaccccgacaagguguucagauccagcgugcugcacucuacccaggaccuguuccugccuuucuucagcaacgugaccugguuccacgccauccacguguccggcaccaauggcaccaagagauucgacaaccccgugcugcccuucaacgacgggguguacuuugccagcaccgagaaguccaacaucaucagaggcuggaucuucggcaccacacuggacagcaagacccagagccugcugaucgugaacaacgccaccaacguggucaucaaagugugcgaguuccaguucugcaacgaccccuuccuggacgucuacuaccacaagaacaacaagagcuggauggaaagcggcguguacagcagcgccaacaacugcaccuucgaguacgugucccagccuuuccugauggaccuggaaggcaagcagggcaacuucaagaaccugcgcgaguucguguuuaagaacaucgacggcuacuucaagaucuacagcaagcacaccccuaucaaccucgugcgggaucugccucagggcuucucugcucuggaaccccugguggaucugcccaucggcaucaacaucacccgguuucagacacugcuggcccugcacagaagcuaccugacaccuggcgauagcagcagcggauggacagcuggugccgccgcuuacuaugugggcuaccugcagccuagaaccuuccugcugaaguacaacgagaacggcaccaucaccgacgccguggauugugcucuggauccucugagcgagacaaagugcacccugaaguccuucaccguggaaaagggcaucuaccagaccagcaacuuccgggugcagcccaccgaauccaucgugcgguuccccaauaucaccaaucugugccccuucggcgagguguucaaugccaccagauucgccucuguguacgccuggaaccggaagcggaucagcaauugcguggccgacuacuccgugcuguacaacuccgccagcuucagcaccuucaagugcuacggcguguccccuaccaagcugaacgaccugugcuucacaaacguguacgccgacagcuucgugauccggggagaugaagugcggcagauugccccuggacagacaggcaagaucgccgacuacaacuacaagcugcccgacgacuucaccggcugugugauugccuggaacagcaacaaccuggacuccaaagucggcggcaacuacaauuaccgguaccggcuguuccggaaguccaaucugaagcccuucgagcgggacaucuccaccgagaucuaucaggccggcagcaagccuuguaacggcguggaaggcuucaacugcuacuucccacugcaguccuacggcuuucagcccacaaauggcgugggcuaucagcccuacagagugguggugcugagcuucgaacugcugcaugccccugccacagugugcggcccuaagaaaagcaccaaucucgugaagaacaaaugcgugaacuucaacuucaacggccugaccggcaccggcgugcugacagagagcaacaagaaguuccugccauuccagcaguuuggccgggauaucgccgauaccacagacgccguuagagauccccagacacuggaaauccuggacaucaccccuugcagcuucggcggagugucugugaucaccccuggcaccaacaccagcaaucagguggcagugcuguaccagggcgugaacuguaccgaagugcccguggccauucacgccgaucagcugacaccuacauggcggguguacuccaccggcagcaauguguuucagaccagagccggcugucugaucggagccgagcacgugaacaauagcuacgagugcgacauccccaucggcgcuggaaucugcgccagcuaccagacacagacaaacagccggcggagagccagaagcguggccagccagagcaucauugccuacacaaugucucugggcgccgagaacagcguggccuacuccaacaacucuaucgcuauccccaccaacuucaccaucagcgugaccacagagauccugccuguguccaugaccaagaccagcguggacugcaccauguacaucugcggcgauuccaccgagugcuccaaccugcugcugcaguacggcagcuucugcacccagcugaauagagcccugacagggaucgccguggaacaggacaagaacacccaagagguguucgcccaagugaagcagaucuacaagaccccuccuaucaaggacuucggcggcuucaauuucagccagauucugcccgauccuagcaagcccagcaagcggagcuucaucgaggaccugcuguucaacaaagugacacuggccgacgccggcuucaucaagcaguauggcgauugucugggcgacauugccgccagggaucugauuugcgcccagaaguuuaacggacugacagugcugccuccucugcugaccgaugagaugaucgcccaguacacaucugcccugcuggccggcacaaucacaagcggcuggacauuuggagcaggcgccgcucugcagauccccuuugcuaugcagauggccuaccgguucaacggcaucggagugacccagaaugugcuguacgagaaccagaagcugaucgccaaccaguucaacagcgccaucggcaagauccaggacagccugagcagcacagcaagcgcccugggaaagcugcagaacguggucaaccagaaugcccaggcacugaacacccuggucaagcagcuguccuccaacuucggcgccaucagcucugugcugaacgauauccugagcagacuggacccuccugaggccgaggugcagaucgacagacugaucacaggcagacugcagagccuccagacauacgugacccagcagcugaucagagccgccgagauuagagccucugccaaucuggccgccaccaagaugucugagugugugcugggccagagcaagagaguggacuuuugcggcaagggcuaccaccugaugagcuucccucagucugccccucacggcgugguguuucugcacgugacauaugugcccgcucaagagaagaauuucaccaccgcuccagccaucugccacgacggcaaagcccacuuuccuagagaaggcguguucguguccaacggcacccauugguucgugacacagcggaacuucuacgagccccagaucaucaccaccgacaacaccuucgugucuggcaacugcgacgucgugaucggcauugugaacaauaccguguacgacccucugcagcccgagcuggacagcuucaaagaggaacuggacaaguacuuuaagaaccacacaagccccgacguggaccugggcgauaucagcggaaucaaugccagcgucgugaacauccagaaagagaucgaccggcugaacgagguggccaagaaucugaacgagagccugaucgaccugcaagaacuggggaaguacgagcaguacaucaaguggcccugguacaucuggcugggcuuuaucgccggacugauugccaucgugauggucacaaucaugcuguguugcaugaccagcugcuguagcugccugaagggcuguuguagcuguggcagcugcugcaaguucgacgaggacgauucugagcccgugcugaagggcgugaaacugcacuacacaugaugacucgagguguguggaggacacccugaaccccccgcuuucaaacaaguuuucaaauuguuugaggucaggauuucucaaacugauuccuuucuuugcauaugaguauuugaaaauaaauauuuucccagaauauaaauaaaucaucacaugauuauuuuaacuaugcuagcaaaaaaaaaaaaaaaaaaaaaaaaaaaaaaaaaaaaaaaaaaaaaaaaaaaaaaaaaaaaaaaaaaaaaaaaaaaaaaaaaaaaaaaaaaaaaaaaaaaa

SEQ ID NO: 75 - RNA, 4157 nt, Artificial
  Epsilon variant S protein mRNA containing 5'-UTR, 3'-UTR and polyA
gagugcuccccauccaacuaaacugucccucuguccgaacuaaacugcacugucccagcaccauguucguguuccuggugcugcugccucugguguccauccagugugugaaccugaccaccagaacacagcugccuccagccuacaccaacagcuuuaccagaggcguguacuaccccgacaagguguucagauccagcgugcugcacucuacccaggaccuguuccugccuuucuucagcaacgugaccugguuccacgccauccacguguccggcaccaauggcaccaagagauucgacaaccccgugcugcccuucaacgacgggguguacuuugccagcaccgagaaguccaacaucaucagaggcuggaucuucggcaccacacuggacagcaagacccagagccugcugaucgugaacaacgccaccaacguggucaucaaagugugcgaguuccaguucugcaacgaccccuuccugggcgucuacuaccacaagaacaacaagagcugcauggaaagcgaguuccggguguacagcagcgccaacaacugcaccuucgaguacgugucccagccuuuccugauggaccuggaaggcaagcagggcaacuucaagaaccugcgcgaguucguguuuaagaacaucgacggcuacuucaagaucuacagcaagcacaccccuaucaaccucgugcgggaucugccucagggcuucucugcucuggaaccccugguggaucugcccaucggcaucaacaucacccgguuucagacacugcuggcccugcacagaagcuaccugacaccuggcgauagcagcagcggauggacagcuggugccgccgcuuacuaugugggcuaccugcagccuagaaccuuccugcugaaguacaacgagaacggcaccaucaccgacgccguggauugugcucuggauccucugagcgagacaaagugcacccugaaguccuucaccguggaaaagggcaucuaccagaccagcaacuuccgggugcagcccaccgaauccaucgugcgguuccccaauaucaccaaucugugccccuucggcgagguguucaaugccaccagauucgccucuguguacgccuggaaccggaagcggaucagcaauugcguggccgacuacuccgugcuguacaacuccgccagcuucagcaccuucaagugcuacggcguguccccuaccaagcugaacgaccugugcuucacaaacguguacgccgacagcuucgugauccggggagaugaagugcggcagauugccccuggacagacaggcaagaucgccgacuacaacuacaagcugcccgacgacuucaccggcugugugauugccuggaacagcaacaaccuggacuccaaagucggcggcaacuacaauuaccgcuaccggcuguuccggaaguccaaucugaagcccuucgagcgggacaucuccaccgagaucuaucaggccggcagcaccccuuguaacggcguggaaggcuucaacugcuacuucccacugcaguccuacggcuuucagcccacaaauggcgugggcuaucagcccuacagagugguggugcugagcuucgaacugcugcaugccccugccacagugugcggcccuaagaaaagcaccaaucucgugaagaacaaaugcgugaacuucaacuucaacggccugaccggcaccggcgugcugacagagagcaacaagaaguuccugccauuccagcaguuuggccgggauaucgccgauaccacagacgccguuagagauccccagacacuggaaauccuggacaucaccccuugcagcuucggcggagugucugugaucaccccuggcaccaacaccagcaaucagguggcagugcuguaccagggcgugaacuguaccgaagugcccguggccauucacgccgaucagcugacaccuacauggcggguguacuccaccggcagcaauguguuucagaccagagccggcugucugaucggagccgagcacgugaacaauagcuacgagugcgacauccccaucggcgcuggaaucugcgccagcuaccagacacagacaaacagcccucggagagccagaagcguggccagccagagcaucauugccuacacaaugucucugggcgccgagaacagcguggccuacuccaacaacucuaucgcuauccccaccaacuucaccaucagcgugaccacagagauccugccuguguccaugaccaagaccagcguggacugcaccauguacaucugcggcgauuccaccgagugcuccaaccugcugcugcaguacggcagcuucugcacccagcugaauagagcccugacagggaucgccguggaacaggacaagaacacccaagagguguucgcccaagugaagcagaucuacaagaccccuccuaucaaggacuucggcggcuucaauuucagccagauucugcccgauccuagcaagcccagcaagcggagcuucaucgaggaccugcuguucaacaaagugacacuggccgacgccggcuucaucaagcaguauggcgauugucugggcgacauugccgccagggaucugauuugcgcccagaaguuuaacggacugacagugcugccuccucugcugaccgaugagaugaucgcccaguacacaucugcccugcuggccggcacaaucacaagcggcuggacauuuggagcaggcgccgcucugcagauccccuuugcuaugcagauggccuaccgguucaacggcaucggagugacccagaaugugcuguacgagaaccagaagcugaucgccaaccaguucaacagcgccaucggcaagauccaggacagccugagcagcacagcaagcgcccugggaaagcugcaggacguggucaaccagaaugcccaggcacugaacacccuggucaagcagcuguccuccaacuucggcgccaucagcucugugcugaacgauauccugagcagacuggacccuccugaggccgaggugcagaucgacagacugaucacaggcagacugcagagccuccagacauacgugacccagcagcugaucagagccgccgagauuagagccucugccaaucuggccgccaccaagaugucugagugugugcugggccagagcaagagaguggacuuuugcggcaagggcuaccaccugaugagcuucccucagucugccccucacggcgugguguuucugcacgugacauaugugcccgcucaagagaagaauuucaccaccgcuccagccaucugccacgacggcaaagcccacuuuccuagagaaggcguguucguguccaacggcacccauugguucgugacacagcggaacuucuacgagccccagaucaucaccaccgacaacaccuucgugucuggcaacugcgacgucgugaucggcauugugaacaauaccguguacgacccucugcagcccgagcuggacagcuucaaagaggaacuggacaaguacuuuaagaaccacacaagccccgacguggaccugggcgauaucagcggaaucaaugccagcgucgugaacauccagaaagagaucgaccggcugaacgagguggccaagaaucugaacgagagccugaucgaccugcaagaacuggggaaguacgagcaguacaucaaguggcccugguacaucuggcugggcuuuaucgccggacugauugccaucgugauggucacaaucaugcuguguugcaugaccagcugcuguagcugccugaagggcuguuguagcuguggcagcugcugcaaguucgacgaggacgauucugagcccgugcugaagggcgugaaacugcacuacacaugaugacucgagguguguggaggacacccugaaccccccgcuuucaaacaaguuuucaaauuguuugaggucaggauuucucaaacugauuccuuucuuugcauaugaguauuugaaaauaaauauuuucccagaauauaaauaaaucaucacaugauuauuuuaacuaugcuagcaaaaaaaaaaaaaaaaaaaaaaaaaaaaaaaaaaaaaaaaaaaaaaaaaaaaaaaaaaaaaaaaaaaaaaaaaaaaaaaaaaaaaaaaaaaaaaaaaaaa

SEQ ID NO: 76 - RNA, 4148 nt, Artificial
  Omicron variant S protein mRNA containing 5'-UTR, 3'-UTR and polyA
gagugcuccccauccaacuaaacugucccucuguccgaacuaaacugcacugucccagcaccauguucguguuccuggugcugcugccucugguguccagccagugugugaaccugaccaccagaacacagcugccuccagccuacaccaacagcuuuaccagaggcguguacuaccccgacaagguguucagauccagcgugcugcacucuacccaggaccuguuccugccuuucuucagcaacgugaccugguuccacgugaucuccggcaccaauggcaccaagagauucgacaaccccgugcugcccuucaacgacgggguguacuuugccagcaucgagaaguccaacaucaucagaggcuggaucuucggcaccacacuggacagcaagacccagagccugcugaucgugaacaacgccaccaacguggucaucaaagugugcgaguuccaguucugcaacgaccccuuccuggaccacaagaacaacaagagcuggauggaaagcgaguuccggguguacagcagcgccaacaacugcaccuucgaguacgugucccagccuuuccugauggaccuggaaggcaagcagggcaacuucaagaaccugcgcgaguucguguuuaagaacaucgacggcuacuucaagaucuacagcaagcacaccccuaucaucgugcgggaaccugaagaucugccucagggcuucucugcucuggaaccccugguggaucugcccaucggcaucaacaucacccgguuucagacacugcuggcccugcacagaagcuaccugacaccuggcgauagcagcagcggauggacagcuggugccgccgcuuacuaugugggcuaccugcagccuagaaccuuccugcugaaguacaacgagaacggcaccaucaccgacgccguggauugugcucuggauccucugagcgagacaaagugcacccugaaguccuucaccguggaaaagggcaucuaccagaccagcaacuuccgggugcagcccaccgaauccaucgugcgguuccccaauaucaccaaucugugccccuucgacgagguguucaaugccaccagauucgccucuguguacgccuggaaccggaagcggaucagcaauugcguggccgacuacuccgugcuguacaaccuggcccccuucuucaccuucaagugcuacggcguguccccuaccaagcugaacgaccugugcuucacaaacguguacgccgacagcuucgugauccggggagaugaagugcggcagauugccccuggacagacaggcaacaucgccgacuacaacuacaagcugcccgacgacuucaccggcugugugauugccuggaacagcaacaagcuggacuccaaagucuccggcaacuacaauuaccuguaccggcuguuccggaaguccaaucugaagcccuucgagcgggacaucuccaccgagaucuaucaggccggcaacaagccuuguaacggcguggccggcuucaacugcuacuucccacugcgguccuacuccuuucggcccacauauggcgugggccaucagcccuacagagugguggugcugagcuucgaacugcugcaugccccugccacagugugcggcccuaagaaaagcaccaaucucgugaagaacaaaugcgugaacuucaacuucaacggccugaagggcaccggcgugcugacagagagcaacaagaaguuccugccauuccagcaguuuggccgggauaucgccgauaccacagacgccguuagagauccccagacacuggaaauccuggacaucaccccuugcagcuucggcggagugucugugaucaccccuggcaccaacaccagcaaucagguggcagugcuguaccagggcgugaacuguaccgaagugcccguggccauucacgccgaucagcugacaccuacauggcggguguacuccaccggcagcaauguguuucagaccagagccggcugucugaucggagccgaguacgugaacaauagcuacgagugcgacauccccaucggcgcuggaaucugcgccagcuaccagacacagacaaagagccaucggagagccagaagcguggccagccagagcaucauugccuacacaaugucucugggcgccgagaacagcguggccuacuccaacaacucuaucgcuauccccaccaacuucaccaucagcgugaccacagagauccugccuguguccaugaccaagaccagcguggacugcaccauguacaucugcggcgauuccaccgagugcuccaaccugcugcugcaguacggcagcuucugcacccagcugaagagagcccugacagggaucgccguggaacaggacaagaacacccaagagguguucgcccaagugaagcagaucuacaagaccccuccuaucaaguacuucggcggcuucaauuucagccagauucugcccgauccuagcaagcccagcaagcggagcuucaucgaggaccugcuguucaacaaagugacacuggccgacgccggcuucaucaagcaguauggcgauugucugggcgacauugccgccagggaucugauuugcgcccagaaguuuaagggacugacagugcugccuccucugcugaccgaugagaugaucgcccaguacacaucugcccugcuggccggcacaaucacaagcggcuggacauuuggagcaggcgccgcucugcagauccccuuugcuaugcagauggccuaccgguucaacggcaucggagugacccagaaugugcuguacgagaaccagaagcugaucgccaaccaguucaacagcgccaucggcaagauccaggacagccugagcagcacagcaagcgcccugggaaagcugcaggacguggucaaccacaaugcccaggcacugaacacccuggucaagcagcuguccuccaaguucggcgccaucagcucugugcugaacgauaucuucagcagacuggacccuccugaggccgaggugcagaucgacagacugaucacaggcagacugcagagccuccagacauacgugacccagcagcugaucagagccgccgagauuagagccucugccaaucuggccgccaccaagaugucugagugugugcugggccagagcaagagaguggacuuuugcggcaagggcuaccaccugaugagcuucccucagucugccccucacggcgugguguuucugcacgugacauaugugcccgcucaagagaagaauuucaccaccgcuccagccaucugccacgacggcaaagcccacuuuccuagagaaggcguguucguguccaacggcacccauugguucgugacacagcggaacuucuacgagccccagaucaucaccaccgacaacaccuucgugucuggcaacugcgacgucgugaucggcauugugaacaauaccguguacgacccucugcagcccgagcuggacagcuucaaagaggaacuggacaaguacuuuaagaaccacacaagccccgacguggaccugggcgauaucagcggaaucaaugccagcgucgugaacauccagaaagagaucgaccggcugaacgagguggccaagaaucugaacgagagccugaucgaccugcaagaacuggggaaguacgagcaguacaucaaguggcccugguacaucuggcugggcuuuaucgccggacugauugccaucgugauggucacaaucaugcuguguugcaugaccagcugcuguagcugccugaagggcuguuguagcuguggcagcugcugcaaguucgacgaggacgauucugagcccgugcugaagggcgugaaacugcacuacacaugaugacucgagguguguggaggacacccugaaccccccgcuuucaaacaaguuuucaaauuguuugaggucaggauuucucaaacugauuccuuucuuugcauaugaguauuugaaaauaaauauuuucccagaauauaaauaaaucaucacaugauuauuuuaacuaugcuagcaaaaaaaaaaaaaaaaaaaaaaaaaaaaaaaaaaaaaaaaaaaaaaaaaaaaaaaaaaaaaaaaaaaaaaaaaaaaaaaaaaaaaaaaaaaaaaaaaaaa

SEQ ID NO: 77 - DNA, 57 bp, Artificial
  primer
ccctctgtccctctgaccctgcactgtcccagcaccatgttcgtgttcctggtgctg

SEQ ID NO: 78 - DNA, 71 bp, Artificial
  primer
atataagctttaatacgactcactataagtcctccccatcctctccctctgtccctctgtccctctgaccc

SEQ ID NO: 79 - DNA, 59 bp, Artificial
  primer
cctctccctctgtccctctcctgcactgtcccagcaccatgttcgtgttcctggtgctg

SEQ ID NO: 80 - DNA, 70 bp, Artificial
  primer
atataagctttaatacgactcactataagtcctcccccgtccctctgaatcctctccctctgtccctctc

SEQ ID NO: 81 - DNA, 65 bp, Artificial
  primer
ccctctttccctctgtccctcttacccttcactttcccagcaccatgttcgtgttcctggtgctg

SEQ ID NO: 82 - DNA, 65 bp, Artificial
  primer
atataagctttaatacgactcactataagtcctccccatcctctccctctttccctctgtccctc

SEQ ID NO: 83 - DNA, 57 bp, Artificial; identical to SEQ ID NO: 77
  primer

SEQ ID NO: 84 - DNA, 71 bp, Artificial
  primer
atataagctttaatacgactcactataagtcctccccattttttttttctgtccctctgtccctctgaccc

SEQ ID NO: 85 - DNA, 57 bp, Artificial; identical to SEQ ID NO: 77
  primer

SEQ ID NO: 86 - DNA, 71 bp, Artificial
  primer
atataagctttaatacgactcactataagtcctccccatccaactaaactgtccctctgtccctctgaccc

SEQ ID NO: 87 - DNA, 57 bp, Artificial
  primer
ccctctgtcccaactaaactgcactgtcccagcaccatgttcgtgttcctggtgctg

SEQ ID NO: 88 - DNA, 74 bp, Artificial
  primer
atataagctttaatacgactcactataagtcctccccatccaactaaactgtccctctgtcccaactaaactgc

SEQ ID NO: 89 - DNA, 63 bp, Artificial
  primer
ctctgtccctctgtcccaactaaactgcactgtcccagcaccatgttcgtgttcctggtgctg

SEQ ID NO: 90 - DNA, 67 bp, Artificial
  primer
atataagctttaatacgactcactataagtcctccccataactaaactctgtccctctgtcccaact

SEQ ID NO: 91 - DNA, 61 bp, Artificial
  primer
ctgtccctctgtcccaactaaactgcactgtcccagcaccatgttcgtgttcctggtgctg

SEQ ID NO: 92 - DNA, 71 bp, Artificial
  primer
atataagctttaatacgactcactataagtcctccccataactaaaaactgtccctctgtcccaactaaac

SEQ ID NO: 93 - DNA, 61 bp, Artificial
  primer
ctgtccctctatcccaactaaactgcactgttccagcaccatgttcgtgttcctggtgctg

SEQ ID NO: 94 - DNA, 73 bp, Artificial
  primer
atataagctttaatacgactcactataagtcctccccatccaactaaactgtccctctatcccaactaaactg

SEQ ID NO: 95 - DNA, 74 bp, Artificial
  primer
atataagctttaatacgactcactatagagtcctccccatccaactaaactgtccctctatcccaactaaactg

SEQ ID NO: 96 - DNA, 61 bp, Artificial
  primer
ctgtccctctgtccgaactaaactgcactgtcccagcaccatgttcgtgttcctggtgctg

SEQ ID NO: 97 - DNA, 71 bp, Artificial
  primer
atataagctttaatacgactcactataagtgctccccatccaactaaactgtccctctgtccgaactaaac

SEQ ID NO: 98 - DNA, 61 bp, Artificial
  primer
ctgtccttctgtcccaactaaactgcactgtcccagcaccatgttcgtgttcctggtgctg

SEQ ID NO: 99 - DNA, 73 bp, Artificial
  primer
atataagctttaatacgactcactataagtcctacccatccaactaaactgtccttctgtcccaactaaactg

SEQ ID NO: 100 - DNA, 19 bp, Artificial
  primer
gccacgcaattgctgatcc

SEQ ID NO: 101 - RNA, 100 nt, Artificial
  polyA RNA
aaaaaaaaaaaaaaaaaaaaaaaaaaaaaaaaaaaaaaaaaaaaaaaaaaaaaaaaaaaaaaaaaaaaaaaaaaaaaaaaaaaaaaaaaaaaaaaaaaaa

SEQ ID NO: 102 - RNA, 181 nt, Artificial
  3'-UTR with restriction site
cucgagccacacccccauucccccacuccagauaaagcuucaguuauaucucacgugucuggaguucuuugccaagagggagaggcugaaauccccagccgccucaccugcagcucagcuccauccccucaccuguucccaccgcauuuucuccuggcguucgccugcuaguguggcuagc

SEQ ID NO: 103 - RNA, 198 nt, Artificial
  3'-UTR with restriction site
cucgagccacacccccauucccccacuccagauaaagcuucaguuauaucucacgugucuggaguucuuugccaagagggagaggcugaaauccccagccgccucaccugcagcucagcuccauccuccacccccccaucuccccucaccuguucccaccgcauuuucuccuggcguucgccugcuaguguggcuagc

SEQ ID NO: 104 - RNA, 188 nt, Artificial
  3'-UTR with restriction site
cucgagccacacccccauucccccacuccagauaaagcuucaguuauaucucacgugucuggaguucuuugccaagagggagaggcugaaauccccagccgccucaccugcagcucagcuccauccuugguuuccucaccuguucccaccgcauuuucuccuggcguucgccugcuaguguggcuagc

SEQ ID NO: 105 - RNA, 162 nt, Artificial
  3'-UTR with restriction site
cucgaggugugacccugaaccccccgcuuucaaacaaguuuucaaauuguuugaggucaggauuucucaaacugauuccuuucuuugcauaugaguauuugaaaauaaauauuuucccagaauauaaauaaaucaucacaugauuauuuuaacuaugcuagc

SEQ ID NO: 106 - RNA, 179 nt, Artificial
  3'-UTR with restriction site
cucgagguguguccacccccccaucuccacccugaaccccccgcuuucaaacaaguuuucaaauuguuugaggucaggauuucucaaacugauuccuuucuuugcauaugaguauuugaaaauaaauauuuucccagaauauaaauaaaucaucacaugauuauuuuaacuaugcuagc

SEQ ID NO: 107 - RNA, 169 nt, Artificial
  3'-UTR with restriction site
cucgagguguguugguuuacccugaaccccccgcuuucaaacaaguuuucaaauuguuugaggucaggauuucucaaacugauuccuuucuuugcauaugaguauuugaaaauaaauauuuucccagaauauaaauaaaucaucacaugauuauuuuaacuaugcuagc

SEQ ID NO: 108 - RNA, 170 nt, Artificial
  3'-UTR with restriction site
cucgagguguguggaggacacccugaaccccccgcuuucaaacaaguuuucaaauuguuugaggucaggauuucucaaacugauuccuuucuuugcauaugaguauuugaaaauaaauauuuucccagaauauaaauaaaucaucacaugauuauuuuaacuaugcuagc

SEQ ID NO: 109 - DNA, 181 bp, Artificial
  a sequence encoding 3'-UTR with restriction site
ctcgagccacacccccattcccccactccagataaagcttcagttatatctcacgtgtctggagttctttgccaagagggagaggctgaaatccccagccgcctcacctgcagctcagctccatcccctcacctgttcccaccgcattttctcctggcgttcgcctgctagtgtggctagc

SEQ ID NO: 110 - DNA, 198 bp, Artificial
  a sequence encoding 3'-UTR with restriction site
ctcgagccacacccccattcccccactccagataaagcttcagttatatctcacgtgtctggagttctttgccaagagggagaggctgaaatccccagccgcctcacctgcagctcagctccatcctccacccccccatctcccctcacctgttcccaccgcattttctcctggcgttcgcctgctagtgtggctagc

SEQ ID NO: 111 - DNA, 188 bp, Artificial
  a sequence encoding 3'-UTR with restriction site
ctcgagccacacccccattcccccactccagataaagcttcagttatatctcacgtgtctggagttctttgccaagagggagaggctgaaatccccagccgcctcacctgcagctcagctccatccttggtttcctcacctgttcccaccgcattttctcctggcgttcgcctgctagtgtggctagc

SEQ ID NO: 112 - DNA, 162 bp, Artificial
  a sequence encoding 3'-UTR with restriction site
ctcgaggtgtgaccctgaaccccccgctttcaaacaagttttcaaattgtttgaggtcaggatttctcaaactgattcctttctttgcatatgagtatttgaaaataaatattttcccagaatataaataaatcatcacatgattattttaactatgctagc

SEQ ID NO: 113 - DNA, 179 bp, Artificial
  a sequence encoding 3'-UTR with restriction site
ctcgaggtgtgtccacccccccatctccaccctgaaccccccgctttcaaacaagttttcaaattgtttgaggtcaggatttctcaaactgattcctttctttgcatatgagtatttgaaaataaatattttcccagaatataaataaatcatcacatgattattttaactatgctagc

SEQ ID NO: 114 - DNA, 169 bp, Artificial
  a sequence encoding 3'-UTR with restriction site
ctcgaggtgtgttggtttaccctgaaccccccgctttcaaacaagttttcaaattgtttgaggtcaggatttctcaaactgattcctttctttgcatatgagtatttgaaaataaatattttcccagaatataaataaatcatcacatgattattttaactatgctagc

SEQ ID NO: 115 - DNA, 170 bp, Artificial
  a sequence encoding 3'-UTR with restriction site
ctcgaggtgtgtggaggacaccctgaaccccccgctttcaaacaagttttcaaattgtttgaggtcaggatttctcaaactgattcctttctttgcatatgagtatttgaaaataaatattttcccagaatataaataaatcatcacatgattattttaactatgctagc